European Patent Specification EP 3 379 945 B1, published September 30, 2026. Title: POLYPEPTIDES CAPABLE OF PRODUCING GLUCANS HAVING ALPHA-1,2 BRANCHES AND USE OF THE SAME. Applicant: E. I. du Pont de Nemours and Company DiCosimo, Robert Zhang, Zhenghong Prasad, Jahnavi Cheng, Qiong. The sequence listing filed with the application follows.

SEQUENCE LISTING (34 sequences)

SEQ ID NO: 1 - protein, 2771 aa, Leuconostoc mesenteroides
MTAGIFSAVIFGVSTTNVSADSTNNTGVTVSQATDKVADTTATTDKVADTTATTDKVADTAATTDKVADTTATTDKVADTAATTDKVADTTATTDKVADTAAATDKAADTAATTDKVADTAAATDKVADTVAATDKVADTTATTDKAADTAATTDKVTDTTAATDKAADTTATTDKVADTTATTSEKSKSIKQIDGKTYFIGNDGQPKKNFTAIVDGQVLYFDKDTGALTSNSSQYTDGLANIGNEHNAAYSLSSDSFTQVDGYLTANSWYRPKDILKNGTTWTAATANDFRPLLMSWWPDKDTQVSYLKYMQSAGLLSDDVALSNNDSMNSLTDTAMTVQKKIEEKIGLLGSTDWLKADMNQMVDSQSNWNISSESKGTDHLQGGALLYVNSDLTPNANSDYRLLNRTPTNQKGQITTNGNQGGYEMLLANDVDNSNPIVQAEQLNWLYYMMNIGSIAQNDPTANFDGYRVDAVDNVNADLLQIAGDYFKAAYGTNQSDANANNHISILEDWDNNDPAYVKAQGNNQLTMDFPMHLALKYSLNMPSSARSGLEPAISTSLVNRAADATENEAQPNYSFIRAHDSEVQTVIAQIIKDKINPSSDGLTVSTDEIAKAFEIYNADELKADKEYTAYNIPSSYALMLTNKDTIPRVYYGDLFTDDGQYMSAKSPYYDALTSLLQSRVKYVSGGQSMNMTYLHNNQGLLTSVRYGKDAMTANDTGTSETRTQGIGLIVGNKTDLNLNNDEQIVLNMGAAHKNQAYRALMLSTKDGLKIYNNDDEAPVSYTDDQGRLIFKSDVVYGVSDAQVSGYLAAWVPVGANDSQDARTESSTTASTDGNTYHSNSALDSQLIYEGFSNFQAMPTQADEYTNIKIAENAQLFKSLGITSFELAPQYRSSTDNSFLDSVIQNGYAFTDRYDIGYNTPTKYGTVDQLLDALRALHAQGIQAINDWVPDQIYNLPGEEIVTASRTNGSGKVNESSVINNTLYDSRTVGGGEYQAIYGGAFLDKLKQDYPELFETKQISTGEAMNPDVKITEWSAKYFNGSNIQGRGAWYVLKDWSTNQYFNVSSGSEFLPKQLLGEKTSTGFTNVDNGKTEFYSTSGYQAKNTFIQDNDNWYYFDNDGYMVVGGQEINGKKYYFLPNGVELQDAYLSDGTSEYYYSSDGRQISNQYYQGSDNNWRYFFADGHMAVGLATITTENGTTNQQYFDANGVQLKGVAIKDTDGNVHYFDGKTGNMVINSWGKISDGSWLYLNDSGVAVTGPQNINGQNLYFNEDGIQVKGEAITDNSGNIHYYDRSTGNMVVNSWGETNNGSWLYLNDKGDAVTGEQVIDGQKLYFSSNGIQLKNTFKKLSDGSWLYLNDKGLPVTGAQVIDGQNLYFDQDGKQVKGDVATDGQGNTHYYDGNTGNMVTNSWAELPDGSWMYLDNDGNPLTGQQKIDGQSLYFNDAGKQIKNALVKLDDGSTIYLDDKGVSSTGIQRIDDKIYYFDPDGKQVVCRFEELPDGSWMYLDDDGVAATGAQKINGQELYFDNSGKQVKNDKVINDDGTINYYTGMSGEKLKNDFGELPDGSWMYLDNQGNAVIGAQKINGQNLYFKTDGRQVKGEANVDSSGEMHFYDPDSGELITNRFEQVASGVWAYFDAKGVAVTGEQRIGKQNLFFDPTGYQVKGDKRTIDGVLYTFDKESGERKGLDSISVLPTNGQYTTDKAQNWYYQVDGENVKGLYTNNDGQLRYFDLTTGVQTKGNFVTIGNDTYYFTKEQGDGQIVSEVVSGHYGTVQLSDNSSAWVYRGANDQILKGLQNINGRLQYFDLTTGAQLKGGAANYDGNLYYFESSDGNLVSKIQQSYSTGNYVTDGDKVTYADEQNNQVTGLALIDDQLQYFDPSDGRQVKNEQVIVDGVTYYFDKNGNGQYLFTNTATMSTNEFAKHSAAYSNDSSSFKNTIDGFLTADTWYRPKDILENGQTWVVSSTNDVRPLITVWWLNKDVQVNYSNFMKQNGLLDTSSQFNLQSDQYDLNVAAQKVQVAIEKRISKEKSTDWLKDLLFEAHEDTPSFVKQQFIWNKDSEYQGQGDAWFQGGYLKYGNNELTPTTNSDYRESGNTLDFLLANDVDNSNPAVQAENLNWLHYLMNFGTITANDDDANFDSIRIDAVDFIDNDAIQRTYDYMRDAYKVDASEDNANKHISLVEAGLDAGTSTIKSDALVESNFREAATLSLANQSGENSSLTNMLQDIDGGQIIADHANNATENESTPNYSIIHAHDKGIQEKVGAAITDVTGADWTNFTDDQLKEGLAAYYQDQRSTNKKYNIYNLPSIYALMLTNKDTVPRVYYGDMYQDDGQYMEKQSIYYDAIVSLMNTRKSYVSGGQTMDVDEHGLLKSVRFGKDAMTASDLGTNETRTEGVGVLVGNDSSLKLNDSDTVTLEMGAAHKNQKYRAALLTTSDGIVTYDADNDAPTIWTDDRGTLTFSNKEIAGQDYTSVQGFANSQVSGYLAVWVPVGASDDQDVRTAALTDANLDDKVLHSNAALDSNLIYEGFSNFQPKATTNDELTNVVIAKNANLFEKWGITSFEMAPQYRSSGDHTFLDSTIDNGYAFTDRYDLGFETPTKYGTDKDLRTAIKALHQSNMQVMADVVDNQVYNLSGQEVVSASRAGVYGNDVSTGFGTQLYAVNSVGGGKYQAQYGGEYLNELKQQYPDLFEAKTYDYWVKNYSNDGSDPYYTLSQNTRKDMPSSEVIKQWSAKYMNGTNVLGNGMGYVLKDWNTGEYFKIGEKNADFITN

SEQ ID NO: 2 - protein, 2821 aa, Leuconostoc mesenteroides
MTAGIFSAVIFGVSTTNVSADSTNNTGVTVSQAPDKVADTTATTDKVADTTATTDKAADTTATTDKVADTAAATDKVADTTATTDKVADTTATTDKVADTAAATDKVADTTATTDKVADTTATTDKVADTTATTDKVADTAAATDKAADTTATTDKAADTTATTDKVADTAATTDKAADTTATTDKVADTAATTDKAADTAATTDKVTDTTVATNKAVDTTATTDKVDDTTATTSEKSKSIKQIDGKTYFIGDDGQPKKNFTAIVDGQVLYFDKDTGALTSNSSQYTDGLVNIGNEHNAAYSLSSDSFTQVDGYLTANSWYRPKDILKNGTTWTAATANDFRPLLMSWWPDKDTQVSYLKYMQSAGLLSDDVALSNNDSMNSLTDTAMTVQKNIEEKIGLLGSTDWLKADMNQMVDSQSNWNISSESKGTDHLQGGALLYVNSDLTPNANSDYRLLNRTPTNQKGQITTNGNQGGYEMLLANDVDNSNPIVQAEQLNWLYYMMNIGSIAQNDPTANFDGYRVDAVDNVNADLLQIAGDYFKAAYGTNQSDANANNHISILEDWDNNDPAYVKAQGNNQLTMDFPMHLALKYSLNMPSSARSGLEPAISTSLVNRAADATENEAQPNYSFIRAHDSEVQTVIAQIIKDKINPSSDGLTVSTDEIAKAFEIYNADELKADKEYTAYNIPSSYALMLTNKDTIPRVYYGDLFTDDGQYMSAKSPYYDALTSLLQSRVKYVSGGQSMNMTYLHNNQGLLTSVRYGKDAMTANDTGTSETRTQGIGLIVGNKTDLNLNNDEQIVLNMGAAHKNQAYRALMLSTKDGLKIYNSDDEAPVSYTDDQGRLIFKSDVVYGVSDAQVSGYLAAWVPVGANDSQDARTESSTTASTDGNTYHSNSALDSQVIYEGFSNFQAMPTQADEYTNIKIAENAQLFKSLGITSFELAPQYRSSTDNSFLDSVIQNGYAFTDRYDIGYNTPTKYGTVDQLLDALRALHAQGIQAINDWVPDQIYNLPGEEIVTASRTNGSGKVNESSVINNTLYDSRTVGGGEYQAIYGGAFLDKLKQDYPELFETKQISTGEAMNPDVKITEWSAKYFNGSNIQGRGAWYVLKDWSTNQYFNVSSGSEFLPKQLLGEKTSTGFTNVDNGKTEFYSTSGYQAKNTFIQDNDNWYYFDNDGYMVVGGQEINGKKYYFLPNGVELQDAYLSDGTSEYYYSSDGRQISNQYYQGSDNNWRYFFADGHMAVGLATITTENGTTNQQYFDANGMQLKGVAIKDTDGNVHYFDGKTGNMVINSWGKISDGSWLYLNDSGVAVTGPQNINGQNLYFNEDGIQVKGEAITDNSGNIHYYDRSTGNMVVNSWGETNNGSWLYLNDKGDAVTGEQVIDGQKLYFSSNGIQLKNTFKKLSDGSWLYLNDKGLPVTGAQVIDGQNLYFDQDGKQVKGDVATDGQGNTHYYDGNTGNMVTNSWAELADGSWMYLDNDGNPLTGPQKIDGQSLYFNDAGKQIKNALVKLDDGSTIYLDDKGVSSTGIQRIDDKIYYFDPDGKQVVCRFEELPDGSWMYLDDDGVAATGAQKINGQELYFDNNGKQVKNDKVINDDGTINYYTGMSGEKLKNDFGELPDGSWMYLDNQGNAVIGAQKINGQNLYFKTDGRQVKGEANVDSSGEMHFYDPDSGELITNRFEQVASGVWAYFDANGVAVTGEQRIGKQNLFFDPTGYQVKGDKRTIDGVLYTFDKESGERKGLDSISVLPTNGQYTTDKAQNWYYQVDGENVKGLYTNNDGQLRYFDLTTGVQTKGNFVTIGNDTYYFTKEQGDGQIVSEVVSGHYGTVQLSDNSSAWVYRGANDQILKGLQNINGRLQYFDLTTGAQLKGGAANYDGNLYYFESSDGNLVSKIQQSYSTGNYVTDGDKVTYVDEQNNQVTGLALIDDQLQYFNPSDGSQVKNEQVIVDGVTYYFDKNGNGQYLFTNTATMSTNEFAKHSAAYSNDSSSFKNTIDGFLTADTWYRPKDILENGQTWVVSSTNDVRPLITVWWPNKDVQVNYLNFMKKNGLLDTSSQFNLQFDQYDLNVAAQKVQVAIEKRISKEKSTDWLKDLLFEAHEDTPSFVKQQFIWNKDSEYQGQGDAWFQGGYLKYDNSELTPTTNSDYRESGNTLDFLLANDVDNSNPAVQAENLNWLHYLMNFGTITANDDDANFDSIRIDAVDFIDNDAIQRTYDYMRDAYKVDASEDNANKHISLVEAGLDAGTSTIKNNALVESNFREAATLSLANQSGKNSSLTNMLQDIDGGQIIADHANNATENEATPNYSIIHAHDKGIQEKVGAAITDVTGADWTNFTDDQLKEGLAAYYQDQRSTNKKYNIYNLPSIYALMLTNKDTVPRVYYGDMYQDDGQYMEKQSIYYDAIVSLMNTRKSYVSGGQTMDVDEHGLLKSVRFGKDAMTASELGTNETRTEGVGVLVGNDSSLKLNDSDTVTLEMGAAHKNQEYRAALLTTSDGIVTYDADNDAPTIWTDDRGTLTFSNKEIAGQDYTSVQGFANPQVSGYLAVWVPVGASDDQDARTAASTDKNTDDKVLHSNAALDSNLIYEGFSNFQPKATTNDELTNVVIAKNANLFEKWGITSFEMAPQYRSSGDHTFLDSTIDNGYVFTDRYDLGFETPTKYGTDKDLRTAIKALHQSNMQVMADVVDNQVYNLSGQEVVSASRAGVYGNDVSTGFGTQLYAVNSVGGGKYQAQYGGEYLNELKQQYPDLFEAKTYDYWVKNYSNDGSDPYYTLSQNTRKDMPSSEVIKQWSAKYMNGTNVLGNGMGYVLKDWNTGEYFKIGEKNADFITN

SEQ ID NO: 3 - protein, 2844 aa, Leuconostoc carnosum
MRDKNVICDRKKLYKSGKLLVTAGIFSTVVFGMAVSDVSANDTDNTVLTSNSGFLDKVVDTTSTDKAATPDKVVDTTSTDKAVTPDKVADTTSTDKAVTPDKVADTTSTDKAATPDKVVDTTSTDKAATPDKVVDTTSTDKAATPDKVVDTTSTDKAATPDKVVDTTSTDKAATPDKVADTTSTDKAATPDKVVDTTSTDKAATPDKVVDTTSTDKAATPDKVVDTTSTDKAATPDKVVDTTSTDKAADRTISISGKTVKNIEEIGGKTYFVGDDGKVKKNFTVIVDGQVMYFDKESGALTSNHKQYKEGLSDITNEHNAAYSLENDNFTQIDSYLTANSWYRPKDILKSGTTWTASTDKDSRPLLMSWWPDQQTELSYLKYMQSAGFLAEDVNLSENNSIDDLTAAAMDVQKNVEAKISLSGNTDWLKEDMNQFVDSQSNWNISSESKGTDHLQGGALLYGNSDMTPDANSDYRLLNRTPKNQTGQISATNDQGGYEMLLANDVDNSNPIVQAEQLNWLHYMMNIGSITKNDSTANFDGYRVDAVDNVNADLLQIAGDYFKAAYGTDKSDANANNHISILEDWDNSDPDYVKKHGNEQLTMDFPMHLALKYALNMPIDMRSGLEPAIKTSLVNRSQDATENEAQPNYSFIRAHDSEVQTVIAQIIKDKINPKSDGLTVTPDEIAKAFEIYNADELKADKAYTAFNIPSSYALLLTNKDTVPRVYYGDLFTDDGQYMSDHSPYYDAITTLLASRIKYAAGGQSMGMTYLHDNQEVLTSVRYGKGALTADDLGNVDTRTQGIGLVISNKTDLSLKSDESVVLNMGVAHKNQAYRPAMLTTKSGLKIYDTDDGAPIVYTNNLGQLIFNADTVYGVSDPQVSGYLAAWVPVGATEDQDARTKGSHDGTTDGNVYHSNAALDSQVIYEGFSNFQAMPTTTDEYTNVKIAQNAQWFKKLGLTSFELAPQYRSSTDSSFLDSVIQNGYAFTDRYDVGYNTPTKYGTVDQLLDALRALHSQDIQAINDWVPDQIYNLPGEQIVTASRTNGSGKYDDDSVISNTLYDSRTIGGGEYQAMYGGAFLDQLKQAYPGLFETKQLSTGVAMDPDVKIKEWSAKYFNGSNIQGRGAWYVLKDWATNKYFSVSSNNTFLPKQLLGEKASTGFITNDGKTEFYSTSGYQAKNTFIEDNGNWYYFDNDGYSVVGKQVIDNKHYYFLPNGVELQDAYLSDGDKQYYYKKTGRQIVNQYYRDEQGDWRYFFADGHMALGLTDIVSNDGTHATQYFDNNGVQVKGTSERDKDGNIHYFDGTSGNLVVSSWGQLSDGSWLYLNDKGIAVTGAQQIDGQSLYFNEDGKEVKGDAVTDNQGNIRYFDGESGHMVVNSWGKLPDGSWMYLNDKGIAVTGQQKINNEVLYFNADGKQIKSAFKELVDGSWLYLNDKGIAVTGAQQIDGQSLYFNEDGKEVKGDAVTDNQGNIRYFDGESGHMVVNSWGKLPDGSWMYLNDKGIAVTGQQKINNEILYFDADGKQLKNTLKTLSDGSRIYLDGKGVSATGVQKINGKVSYFDVNGKQVSNHIQELPDGSWMYLDNDGLALIGNQDVDGKQLYFDVDGKQIKNDKVKNSDGTINYYTGTVGEKLKHDFGQLSDGSWMYLDENGNAVTGEQNINGQHLYFKDDGQQVKGDVFEDDLGRMRYYSANSGEMVVNQFEQISDGAWAYFGDDGVAVTGEQHINGQDLFFDATGQQVKGESRTINGIPYTFEKESGEKRSVNIAPLLAMGNYVTNNGTDWQYEVQGNPVKGLYSTSDNKLRYFDLTTGVQIKGNFVTIGHNTYYFNPANGDGELLPDVSDGHYGTIQVKDANTNEKTVWVYRNQSNTILKGIQNIHGNIQYFDLSTGEQIKGGIANYDGNDYYFESAKGNLTSKIKQVYTDGQYVTKDGKSIYEDAQQQSVSGLVSINGQLQYFNPQDGVQVKNQQIIVDGVTYYFDENGNGQYLFTNTTVMPMDDFTKHNTVYSDNDNNFKNNVDGFLTADTWYRPKEILKAGTTWTTTSESDMRPLITTWWPNKNVQVNYLNFMKQNNLLHTNVEYSLLSDQYDLNIAAQAVQTAIEKRIAQENSTDWLQNLLFTAQDDQPSFVKQQFIWNKDSEYQGKGDAWFQGGYLKYGNNKLTPNTNSNYRKTDNAFEFLLANDIDNSNPVVQAENLNWLEYLMNFGTITGKDDDANFDSIRVDAVDFISNDTIQRTYDYLRDAYQVDQSEAKANQHISLVEAGLDAGTSTVKNDALIESNLREAATLSLANASGKNSALTNMLQDVDGGTLIADHTHNSTENEATPNYSIIHAHDKGIQEKVGAAISDATGADWTNFTDTQLKSGLDLYYKDQRATDKKYNIYNLPSIYALMLTNKDTVPRVYYGDMYQDNGQYMAEKSIYYNALESLMSARKSYVSGGQTMDVDSHGLLKSVRFGKGAMTADTVGNEETRTEGIGVLVGNDASLKLNDSDTVTLDMGAAHKNQKYRAAILTTNNGLSTFDSDKDAPIAWTNDKGILTFSNKNVSGQDNTNVHGVANPQVSGYLAVWVPVGAKDDQNAGTSASTVVNTDGKVLHSNASLDSNLIFEGFSNFQPRATTNDELTNVVIAKNADLFQKWGITSFEMAPQYRSSQDHTFLDSTIDNGYAFTDRYDLGFNTPTKYGTDSDLRLAIKSLHKAGMQVMADVVDNQVYNLPDQEVVSASRAGVYGNDVATGFDTQLYAVNSVGGGKYQAQYGGQYLSELKNKYPDLFEAKAYDYWTKNYANDGSNPYYTLSQQTRDDIPSDEKIKQWSAKYMNGTNVLGHGMGYVLKDWNTGQYFKINKDGDSNLPV

SEQ ID NO: 4 - protein, 1672 aa, Fructobacillus tropaeoli
MRKKLYKSGKMWVAASVAISFSALSISVGNNGAKADDSQQSSTQIQSTQVTTALPAGGQYSTTNGGQSWNYLVNGVAIKGMYQDGQGQLRYFNFIDGTQVKGEFLSINGTYYYFDQNSGEGHLVPTQSNGHYTEIGNTGAWGYQNSNGELVKGIQNIDGQLRYFDENTGNQVKGGSATIGNKSYYFEPSQGTLTTTIDQVSDAQNANIRGLATVNGQLNYFDPTTGEQAKHKQVATNGATYYFNDSGVGTYLFTNVQNTPANDVSQHNAVNSTDTKDYTNTVDGFLTADTWYRPKYILDNGENWRASNEGEYRPFIMNWWPNKNVEVNYLKLMQNNNLLSSTVQYDLFTDQAILNQAAYQAQIAIEKRIKSEGSTDWLNTLLFGGDDSHPSFVKQQFIWNSDSESPWQGDAWFQGGYLKYGNSVMTPTSNSNYRQAGNAFDFLLANDVDNQNPIVQAEDLNWLYYLMNFGSITTNGLDNDSNFDSIRLDAVDFIHNDAIQRTYDYLRQAFNLTKNEATANQHLSLVEAGVDAGTTTYNSDGLIESNIRPLATDSLTNAPGKNASLSNLIKDVDSGEVIADHANFSTDDGIPNYSIIHAHDKGIQENVGAAITAATGADWTNFTTEQLEQGLDLYYQDQRSTNKKYNIYNLPSIYALMLTNKGTVPRVYYGDMYQDNGQYMQQKSLYYDAISSLMTARKQYVAGGQTMSVDENGLLKSVRFGKNAMTAQDTGDAETRTEGVGVIIGNDPSVKVADGQTVTLDMGAAHKNQAYRPLILTTSDGIQTYDSDENAPVVYTDDNGILTFSNQDINGQANTKIVGTLNPQVSGYLAVWVPVGASADQDARTAPSTQSTNDGKVLHTGAALDSNLIFEGFSNFQPMPTTHDEMTNVVISQNASQFAKWGITSFEMAPQYRSSEDHSFLDSTIDNGYAFSDRYDLGFGTPTKYGTDEDLRNAIKALHQNGMQVMADVVMNQLYSLNGKEVVSASRAGVYGNDVDLPFGTQLYVVNTTGGGEYQKKYGGAFLNIIKEKYPTLFDSESYDYYLKNYSDNGHGPAYMTTATATREAIPSDQPLKEWSAKYMNGTNILGLGMGYVLKDWNNGAYFKLSGTDTTLPQSLVALTGWNQNDDGTWSYYSTDTDDRVTGKQVIDGRTLLFDNQGNQIKGGWGENPDGTWSYYNADTGDRVIGEQVIDGRTLFFDNQGVQVKGGWGENYDGTWSYYNADTGDRVTGKQVIDGRTLLFDNRGVQVKGGWGENSDGTWSYYNADTGDRVTGNQLIGGRNLLFDNQGNQIKGGWDENPDGTWSYYNADTGDRVTGVQVIDGKQLLFDSNGIQVKNSWQKNANGTWSYYDANDGHLVPANSSNDGTSSSTQDSGNKSNQNPSSSSNAVNKTTGWIKNSDGTWSYLSAKSGQKVTGSQTIDGKQLLFDDHGVQIKGGWGKNADGTWSYYDANSGELTSTSDMSNVNPQQTTTTTNEQSTTNQPTDITKNSDGVYVYKNDSNKKAQGYLNDGSSWKWFNDGQLYTGFQNYMGAYYYFINGIRQQNQWENIWGLKYYVGDDGRTVEGIHAIDGHAYDFGTDGTFNVKGSASGYLNDGKSWMWYEGGNPYTGFRYYMDTYYWFENGVRQDNAWHQAWGLTYYTGADGRAVQGVQNINGKLYYFGNDGTFFMRTNQEV

SEQ ID NO: 5 - protein, 1632 aa, Lactobacillus kunkeei
MNNNNSEQKLRFKMYKSGKHWVVAGLTTAVVSVAIYSGSSIINGGVTVKADVQSTTQATTSVSDNSKDSSNSISNNNSNDDNQIATLPQDGTYSTGDNGQTWKYVEQNKNIQGLYKDSDNQLRYFNEYDGTQAKGDIVNVNNNNYYFDSGSGQGHKIDNYSGGNYVESNVNNENGWIYKATDNTEVKGIATIDGNVQYFDQSTGLQLKGGAVQVGGADYYFDPNKGNLVGKVDQVVNSNNYSDNKLLDSNKNVVKGLTVNNGTLQYYDPSTGDQVKNKQVIANGVTYYFDASGNGTYLFTNTGNSAVNDFSQRNAANSVNPSDYKNVVDGFFTADTWYRPKQIIDNGTTWRNSNSNDLRPMITAWWPNKDVQVNYLKLMQDNGLLDKSDTYTLQSDQQVLNQAAQSAQVNIEKKISQTGSTDWLNDLLFASHGNNPSFVKQQYVWNSDSESPWQGDAWFQGGYLKYGNSVMTPNTNSNYRDSNNLFDFLLANDVDNSNPAVQAEDLNWLYYLTNFGTITANDSNANFDSIRIDAVDFISNDIIQRSYDYLRQKFNLTQSDANADSHISLVEGGVDAGTTSYSNDGLVEAPFRLGAYPLLHKQGGDVFKDLINEEDSGIDISNHNGETNTTNTIGGLTLSGGKPNYSIVHAHDKDVQEKVGQAIVDTTGIKDWTDFTPSQLAQGLETFYNDQRQTDKKYNDYNVPSAYAIMLTNKGTVPRIYYGDMYQDDGQFMQKKSLYYDDIANLMTARKKYVSGGQYMVDNDGILTSVRFGKGANTVNDSGTSDTRNQGIGLIVGSDPKKVLNDGDTIVLHMGAAHKNQKYRALMLTTENGVQNYSSDDNAPVAETDDNGDLVFSNKDINGQDNTAIKQVANPEVNGYLAAWVPFGASDDQDARTSPSTSQNNDGNVLHENDALDSNLIFEGFSNFQPTPTNHDEYANVVIAKNASLFKDWGVTSFEMAPQYRSSQDHTFVDSTIDNGYAFSDRYDLGFGTPTKYGTDEDLRNAIKSLHANGMQVMADVVYNQLYNLPGEEVVSATRAGVTGNDNALPFGTQLYVVNTVGGGDYQKKYGGAFLNQLQEQYPSLFQSQKYKYYYKNYANNGAGPGYLTVTDGERSAIPSDQPITAWSAKYMNGTNILGRGMGYVLKDWNTGAYFKISGDDSTLPTSLTYRSGWVENPDSTWSYYSKDSIAKLTGAQIVNDQRVFFDNNGIQVKGGWVENPDGTYSYYDKNSGELLVGSQLVDGRHVFFDNVGVQVKGGWVANTDGSYSYYNANDGTMLTGAQFIDGQNVYFDADGKQVKGNWVQNNDGSWAYYDANLGHLVKDAKHVDSQPSTQQVNNKQSEEKSNSPLVEAQNNKDSASVESQNHQNSVSVESKNENKNQSNDVRNPSEKTDTKTSNEKSKEVSKEDAAYDNAKKSLVEAKKLVDKKPNKTNINKYKKALKSYENAQKKMNKSVISSYKKAAKELNAAKKNLSKKNNKVNMKKYSIALNKYRNAKKSYVVIKKKDLDKSKSALNTAKKALAKKKTKQSQKKYNDALKKYYDAEKTYLNLTGNYTKKYYYDFDKVGKKVKVIKSTSVYNSLKPNSKKVVKKIKKGSVIKVKKLILSNKKSYFDLGYNRFVIASKSSIKKAK

SEQ ID NO: 6 - protein, 1318 aa, Lactobacillus kunkeei
MKSKDNNSKIHFKMYKSGKQWVIAGLTTAVAAVSIYGGTTIFNDSVVAKADTAVKSSQSSNADTTQSSSAVVDSSSANSSSPSSTEVSVNVKNTSNADTQGIQALPDGGNYTSEDNGQTWKYSYQNNDVKGLYQENNNIRYFSENDGSQVKGNILNVNNKNYYFDSNNGDGHLIKDYSGGNYVEQSQDKWTYKTSDNNLVKGIATIDGQIKYYDPTTGIQLKGGAFEIGGAAYYVDPAQGNVVGRVNSIINSGNYVNKNNNTTFVDDNNNTVKGLNVVRGNLQYFNSTTGYQAKSEQVVANGATYYFDKDGNGTFLFNNTGSFSVTDFAKHNVANSNQPSDFTNTVDGFLTAETWYRPKQILDNGTKWRNSNKDDLRPLITVWWPNKDVQVNYLKLMQDNGLLDNSVKYTVFSDQQTLNEAAQSAQVNIEKRITQQKASSWLYDLLFKGDSSHPSFMNQQYIWNMGSESQWQGDAWFQGGYLKYGNSPLTPTTNSKYRKTDNQFDFLLANDVDNSNPAVQAEDINWLYYLTHFGTITGKNDKANFDSIRLDAVDFVSNEIIERSNDYLRDLYKLTKSDANADKHISLVEAGVDAGTSSTNGDSLVEAPFRLSAYGLLHNSGKVDALQDLVKEVDSGVLISDHSKNSKDGGVPNYSIVHAHDKDVQERVGQAIVDSTGIKDWTNFTPAQLAKGLSVYYADQRKTVKKYNDYNMPSAYAIMLTNKGTVPRIYYGDMYQDDGQFMQKKSFYYDDIVKLMTARLKYVAGGQTMSVDSNGFLKSVRFGKGAKTVNSKGTKETRHEGIGLIVGNDAKKVLSNGQKVTLNMGAAHKNQKYRALMLTTNKGVQTFASDKNAPVVKTDGNGVLTFTNKDIKGQANTSVRGVLNPKVSGYLAVWVPVGAKDNQDARTQPSKKNRNDGKVLHSNDALDSNLIYEGFSNFQPQPKKRSQYANVVIAKNAKLFKKWGITSFEMAPQYRSSNDKTFVDSTINNGYAFSDRYDLGFGKPTKYGTDKDLRKAIESLHDQGMQVMADAVLNQLYNLPGKQVVSAQRAGVTGNIADLPFGKQLYVVNTIGGGKYQKKYGGKFLKALKAKYPNIFKGKTYKYNYKNYSPTGEGYLTLNTGKTVSIPSNQPITEWSAKYMNGTNILGRGMGYVLKDWNTGTYFKLNGLKTVLPSELTDKSNWVNEVSTSSKDVYNKSVSNLKDAKKKLAAKKSKENTQLYNNALNSYYKAEKEYLSSAKLYNKKYYYDFDKLPSKVKVAKVTYSYKSTDFSKDNRIKKLKKGTVLNVKGLVLNGKVTRINIGNGKFVTASKDFIKAIR

SEQ ID NO: 7 - protein, 1139 aa, Lactobacillus kunkeei
MKAEHNNLKLHFKMYKSGKQWVIAGLTTVVASIAIFSGNQLFSGNVVAKADGVTTTQVSQNSNSSNGISTLPKDGKYVSSDNGKTWKYVSQNNAAKGLYSDGSNIFYFNESDGTQVKGNIISVGKNTYYFDSKTGQGTKISDYTGGKYTNPSTDNKAAWTYQDKSNNTVKGVATIGDSVQYYDEKDGFQLKGGSINLGNTNYYVDSNQGNVTSKVNRVVSSNDGTLKGLNVVNGNLQYLDYKTGKQVKNKQVAVNGVTYYFDDNGNGSYLFTNLGKSVRTNFDKYNAVNGVNKSNFTNTVDGFLTADSWYRPKQVLANGKKWRKSTSKDFRPLVTVAWPNKDVQVNYLALMQMNGLLSNKEKYTVFSDQQTLNAAAQKAQVNIEKRISKKKSTKWLDKLLFQGTTTEPSFIKRQYVWSSASEYPGQGDAQWFQGGYLKYGNNRLTPKTNSKYRQIGNAFDFLLANDVDNSNPSVQAEDINWLHYLTHFGSITAKDPKANFDSIRIDAVDFISNDIVQRSNDYLRDLYKLTKNDSNADKHISLVEGSLEAATSYSHSDSLIESPYRNDIDGLLGNSGNSADLSKLIKEYDSGIIISDHSGTTNNSSIPTYSIVHAHDKGVQERVGQAIMDNSGITDWANFTPKQLRDGLKLYYDDQRKTVKKYNDYNVPSAYAIMLTNNNTVPRIYYGDMYQDDGQFMQKKSLYYDDIVSLMLARTKYVAGGQSMSMDSNGFLTSVRYGKGANNVNSQGTSETRNEGIGVIVGNDTNKVLNDGQTVTLNMGAAHKNQQYRPVLLTTKDGIKTYSSDKNAPVVETDSNGVLTFSNKDVNGQSDTSVRGTLNPQVSGYLAVWVPVGAKNGQDARTKPSKKARNDGKVLHLNDALASNLIFEGFSNFQPMPKNKSQYTNVVIAKNAKTFKKWGITSFEMAPQYRSTNDKSFVDSTIKNGYAFSDRYDLGFGKPTKYGTDKDLRKAIKSLHAQGMQVMADVVYNQLYNLPGKEVVSTSRASAYGNNVDVPFGNQLYVVNTIGGGKYQTKFGGKYLKELKKKYPSLFKAKTYKYYYKDNQKDGSVKLALTSSKRSSIPANKPIKEWSAKYMNGTNVLGLGMGYVLKDWNNGKYFKINGTKTSLPSSIYYKSTKNK

SEQ ID NO: 8 - protein, 1463 aa, Lactobacillus kunkeei
MNINSNERKVRFKMYKSGKQWIVAGLTTAVISIAVYGGSSIANGGIEAKADAQNAATSSIVNTNNSTNSSNANSIASLPQNGTYSTNDNGQTWKYVSQNKDIQGLYKDNNDQLRYFNEYDGTQAKGDIVNVNNDNYYFDKDSGQGHKIDSYTGGSYSESKVNNQDGWIYKSSDNNDVKGVATVDGNIQYFDQNTGLQLKGGSAQIGGVDYYFDPNKGNLVGKVDQVVNSNDYSDNKLLDSNKNVVKGLVVNNGQLQFFDTSNGNQAKNKQVIANGITYYFDTNGNGQYLFTNTGKSAVDDFTQRNAANSVNPSDYKNVVDGFFTADTWYRPKQILDNGTTWRNSNSNELRPMITAWWPNKDVQVNYLKLMQNNGLLDKSNSYSIQSDQQTLNQAAQKAQVNIEKKISQTGNTDWLNDLLFKGNGDNPSFVKQQYIWSSDSESPWQGDAWFQGGYLKYGNSVMTPNTNSNYRDSNNLFDFLLANDVDNSNPAVQAEDLNWLYYLTNFGTITANDSNANFDSIRIDAVDFISNDIIQRSYDYLRQKFNLMQSDANADSHISLVEGGVDAGTTSYSNDGLVEAPFRLDAYPLLHKQDGDVFKNLIDEEDSGIDISNHNGETNTNNTIGGITLSGGKPNYSIVHAHDKDVQEKVGQAIIDTTGIKDWTDFTPSQLAQGLETFYNDQRQTVKKYNDYNVPSAYAIMLTNKGTVPRIYYGDMYQDDGQFMQKKSLYYDDIANLMTARKKYVSGGQSMVDNNGILTSVRFGKGANTVSDSGTEDTRNQGIGLIVGSDPKKVLNDGDTVVLHMGAAHKNQKYRALMLTTENGIQNYNSDDNAPVAETDDNGDLVFSNKDINGQANTAIKQVANPEVNGYLAAWVPVGASDDQDSRTAPSTSQNNDGNVLHENDALDSNLIFEGFSNFQPTPTNHDEYANVVIAKNASLFKDWGVTSFEMAPQYRSSQDHTFVDSTIDNGYAFSDRYDLGFGTPTKYGTDEDLRNAIKSLHDNGMQVMADVVYNQLYNLPGQEVVSATRAGVTGNTNALPFGTQLYVVNTIGGGDYQKKYGGAFLNELQEQYPSLFKSQKYKYYYKNYANNGAGPGYLTVNDAERSDIPYNQPITEWSAKYMNGTNILGRGMGYVLKDWNTGDYFKLSGSDSTLPSSLTYKSGWVENPDSTWSYYEKNNIDKLTGSQVINEERVFFDNNGIQVKGGWVKNSNGTYSYYDKNSGNILTGDQLIDGEHFFFDNNGVQVKGKWIKNSDGSKSYYDSHLGKLIKTDKKVSSNARKKKSKEELLYENALKVLRKDKKRLDKNKTKANIRKYNKSLKKYRKAKKKLLAITKNRVANARKAIKIAKKVLSKRKNINNEKRYYKALKEYYVAEKSYLKITGNYNKKYYYEFDKLTPKVKVVKNIYSYKSRHFTKKNRVKKIKKGTLVRVKSIVRSGKVARINIGNGHFITSSKDFIKMFK

SEQ ID NO: 9 - protein, 2841 aa, Leuconostoc mesenteroides
MRDKRIICDRKKLYKSGKLLVTAGIFSAVIFGVSTTNVSADSTNNTGVTVSQAPDKVADTTATTDKVADTTATTDKAADTTATTDKVADTAAATDKVADTTATTDKVADTTATTDKVADTAAATDKVADTTATTDKVADTTATTDKVADTTATTDKVADTAAATDKAADTTATTDKAADTTATTDKVADTAATTDKAADTTATTDKVADTAATTDKAADTAATTDKVTDTTVATNKAVDTTATTDKVDDTTATTSEKSKSIKQIDGKTYFIGDDGQPKKNFTAIVDGQVLYFDKDTGALTSNSSQYTDGLVNIGNEHNAAYSLSSDSFTQVDGYLTANSWYRPKDILKNGTTWTAATANDFRPLLMSWWPDKDTQVSYLKYMQSAGLLSDDVALSNNDSMNSLTDTAMTVQKNIEEKIGLLGSTDWLKADMNQMVDSQSNWNISSESKGTDHLQGGALLYVNSDLTPNANSDYRLLNRTPTNQKGQITTNGNQGGYEMLLANDVDNSNPIVQAEQLNWLYYMMNIGSIAQNDPTANFDGYRVDAVDNVNADLLQIAGDYFKAAYGTNQSDANANNHISILEDWDNNDPAYVKAQGNNQLTMDFPMHLALKYSLNMPSSARSGLEPAISTSLVNRAADATENEAQPNYSFIRAHDSEVQTVIAQIIKDKINPSSDGLTVSTDEIAKAFEIYNADELKADKEYTAYNIPSSYALMLTNKDTIPRVYYGDLFTDDGQYMSAKSPYYDALTSLLQSRVKYVSGGQSMNMTYLHNNQGLLTSVRYGKDAMTANDTGTSETRTQGIGLIVGNKTDLNLNNDEQIVLNMGAAHKNQAYRALMLSTKDGLKIYNSDDEAPVSYTDDQGRLIFKSDVVYGVSDAQVSGYLAAWVPVGANDSQDARTESSTTASTDGNTYHSNSALDSQVIYEGFSNFQAMPTQADEYTNIKIAENAQLFKSLGITSFELAPQYRSSTDNSFLDSVIQNGYAFTDRYDIGYNTPTKYGTVDQLLDALRALHAQGIQAINDWVPDQIYNLPGEEIVTASRTNGSGKVNESSVINNTLYDSRTVGGGEYQAIYGGAFLDKLKQDYPELFETKQISTGEAMNPDVKITEWSAKYFNGSNIQGRGAWYVLKDWSTNQYFNVSSGSEFLPKQLLGEKTSTGFTNVDNGKTEFYSTSGYQAKNTFIQDNDNWYYFDNDGYMVVGGQEINGKKYYFLPNGVELQDAYLSDGTSEYYYSSDGRQISNQYYQGSDNNWRYFFADGHMAVGLATITTENGTTNQQYFDANGMQLKGVAIKDTDGNVHYFDGKTGNMVINSWGKISDGSWLYLNDSGVAVTGPQNINGQNLYFNEDGIQVKGEAITDNSGNIHYYDRSTGNMVVNSWGETNNGSWLYLNDKGDAVTGEQVIDGQKLYFSSNGIQLKNTFKKLSDGSWLYLNDKGLPVTGAQVIDGQNLYFDQDGKQVKGDVATDGQGNTHYYDGNTGNMVTNSWAELADGSWMYLDNDGNPLTGPQKIDGQSLYFNDAGKQIKNALVKLDDGSTIYLDDKGVSSTGIQRIDDKIYYFDPDGKQVVCRFEELPDGSWMYLDDDGVAATGAQKINGQELYFDNNGKQVKNDKVINDDGTINYYTGMSGEKLKNDFGELPDGSWMYLDNQGNAVIGAQKINGQNLYFKTDGRQVKGEANVDSSGEMHFYDPDSGELITNRFEQVASGVWAYFDANGVAVTGEQRIGKQNLFFDPTGYQVKGDKRTIDGVLYTFDKESGERKGLDSISVLPTNGQYTTDKAQNWYYQVDGENVKGLYTNNDGQLRYFDLTTGVQTKGNFVTIGNDTYYFTKEQGDGQIVSEVVSGHYGTVQLSDNSSAWVYRGANDQILKGLQNINGRLQYFDLTTGAQLKGGAANYDGNLYYFESSDGNLVSKIQQSYSTGNYVTDGDKVTYVDEQNNQVTGLALIDDQLQYFNPSDGSQVKNEQVIVDGVTYYFDKNGNGQYLFTNTATMSTNEFAKHSAAYSNDSSSFKNTIDGFLTADTWYRPKDILENGQTWVVSSTNDVRPLITVWWPNKDVQVNYLNFMKKNGLLDTSSQFNLQFDQYDLNVAAQKVQVAIEKRISKEKSTDWLKDLLFEAHEDTPSFVKQQFIWNKDSEYQGQGDAWFQGGYLKYDNSELTPTTNSDYRESGNTLDFLLANDVDNSNPAVQAENLNWLHYLMNFGTITANDDDANFDSIRIDAVDFIDNDAIQRTYDYMRDAYKVDASEDNANKHISLVEAGLDAGTSTIKNNALVESNFREAATLSLANQSGKNSSLTNMLQDIDGGQIIADHANNATENEATPNYSIIHAHDKGIQEKVGAAITDVTGADWTNFTDDQLKEGLAAYYQDQRSTNKKYNIYNLPSIYALMLTNKDTVPRVYYGDMYQDDGQYMEKQSIYYDAIVSLMNTRKSYVSGGQTMDVDEHGLLKSVRFGKDAMTASELGTNETRTEGVGVLVGNDSSLKLNDSDTVTLEMGAAHKNQEYRAALLTTSDGIVTYDADNDAPTIWTDDRGTLTFSNKEIAGQDYTSVQGFANPQVSGYLAVWVPVGASDDQDARTAASTDKNTDDKVLHSNAALDSNLIYEGFSNFQPKATTNDELTNVVIAKNANLFEKWGITSFEMAPQYRSSGDHTFLDSTIDNGYVFTDRYDLGFETPTKYGTDKDLRTAIKALHQSNMQVMADVVDNQVYNLSGQEVVSASRAGVYGNDVSTGFGTQLYAVNSVGGGKYQAQYGGEYLNELKQQYPDLFEAKTYDYWVKNYSNDGSDPYYTLSQNTRKDMPSSEVIKQWSAKYMNGTNVLGNGMGYVLKDWNTGEYFKIGEKNADFITN

SEQ ID NO: 10 - protein, 2580 aa, Lactobacillus kunkeei
MNNYQDRKLHYKMYKSGKNWVVAGIVSATMSIVLFQNINDVTAKASQNQITYSGSYASTDSGSAKSAYSASSYINGSSSLSVPSTDNSNKSSLASSTNSSVVTSSLSSNVMNQSSNSHASSISSDVSNQSQSSKSASTSSNSSEKSDSASQSNNSVQSYESVSLSVSLASNASQNLKSHTKNIDGKTYFYDLNNNEVKSALIDDNNTYYYFGPNGYLTTFDDSKFSDGSINSSDQLSIYTPDGKSITNVDGFLTADSWYRPKQIQVSDTQWRNSTNADFRPLLSVWWPNKTVEINYLNYMSKNGLVNGHFDNNSSANDINQAAATVRLSIENKIKADNGDLSAIRSLFTTFINSQDEWNIDSEDYNSGDGLQGGSLLFGNNSETKDANSNYRLLNRNPTQQDGKIDYTHTQDPGFEFLLANDVDNSNPVVQAETLNWLHYLMNFGSIVNKDSSANFDGVRVDAVDNMDADVLNIISQYFRDAYKINANDVNSNNHLSILEDWSGNDPYYQKDHGTNQMTLDSDYLSSLRSILMYNPSVRSDMSTIINAGIVDRADDNTTNKAIPNYEIVRAHDAGVQDIISQIIIDNIDPHASASNPTWEQMREAFKIYDADENSTVKKYTQYNIPASYALTLTNKDTTPRVYYGDLYTDDGQFMEQKTPYYDAIAEMLKSRVKYVAGGQHMEAVKVNNGEDTILTSVRYGKDALNADDLGDSLTRTSGIAVVESNNPTLSLSDKDKVVIHMGAAHKNQEYRQLLTASNSGIDSFDSDSSKGYVVVRTDDNGDLTLDGNIIKGYANPQVSGYLSMWVPLGASDNQDIRTAPSSESSTDGQSIHSNEASDSNVILEAFSNFQNFPQTTDQYENVVIQKNAEDFKNLGFTYLELPPQYKSTKDGSFIDSVVQNGYSFNDRYDLGFDTPTKYGTAEQLIDAIKSLHAQGIKVLADIVPDQIYSLPNQQIVNATRTNPYGDANFNSNLINVLYDAFSKGSGTDYQYKYGGEFLEQLKKLYPDLFTTKQISTGQPIDASKKLKIWTAEYLNGSNIQGRGSGYVLSSTPNSNYYTVVDDGNTNIKSSNLPKGLLGDNVEYGLKLIDGKMKYVSTGGFIAKNTFIQDDNHNWYYVDNNGDFVTSPQVINGNKYFFLSNGVNLRDFISVNSDGTMNYYQSNGILANNPGYYYSNNINQMVHVNNNGVLDTGIVNVNGYVQYFDDNGYQVKGDIVNFNGRKMYFDDGSGNLVYNRFVSYNGNWYYAGSNGLLVNGLQNINNQSLYFDDNGKQVKGGMISLDNHKMYFDANSGNLYKNSFVLLDGDVYYANNDGYIVNGYQNIGGRNLYFDSDGKQVKDQFVNINGNKVYFNGTDGSEVKDDFIIHDDKEYYADNQGHLLTGYNFVNGQNMYFNEDGSQVKNSIVSLDGKLMYFDENSGNQVKNGFILHNGNVYYSNKDGILVTGYQNIDGQDLFFNADGTQIKGGTAEIDGVNYYFENGEGHLVGKVDQVINSNRFSDNKLLDANNNVVKGLIFNNGQLQYFDSLTGDQAKNKQIIADGNTYYFDNSGNGTYLFTNIGESETNDFSQRNAANSVNLSDYKNVVDGFFTADTWYRPKQILDNGTTWRNSNSNDFRPMITVWWPNKNVQVNYLKLMQNNNLLDKSTNYTLQSNQQMLNQAAQNAQVNIEKKIAQTGNTDWLNDLLFKGNGDTPSFVKQQYIWNILSESPGQDDALLQNGYFKYVNSELTPNTNSSYRISNNLCDFLLANDVDNSNPAVQAEDLNWLYYLTNFGTITANDPNANFDSIRIDAYAFINNDIVQRSNDYMKQKYKLTESSNNANSHLSIVEAGVDAGTTSTNNDELVESPFRTISYGLIHKDRNPQDMNNFIKEVDTGVVIADHENNSQEIGQPNYSIVHAHDKDIQDKVGEAIVDATGIKDWTNFTPSELSAGLKLYYDDQRSSEKKYNDYNIPSAYAIMLTNKGTVPRIYYGDMYQDDGQFMQKQSVYYDDIVSLLTARKKYVSGGQSMSVDHNNFLESVRFGKGAGSESDSGNAETRNEGIGLIVGNDQNKKLNDGDTVVLHMGAAHRNQKYRALMLTTNDGIKNYDSDENAPIAETDSNGDLVFSNKDINGQANTSVRGVLNPEVAGYVAAWVPLGASDDQDSRTLSSNKSYNDGKVLHSGDDLDSNVIFEAFSNFQPEPTNENEYENVVIPQKASLFKDWGITSFELPPQYRSSNDHTFVDATINNGYAFSDRYDLGFGQPTKYGTDVDLRNTIKSLHDNGMQVMADVVYNQLYNLPGQEVVSAVRAGFTGNTVSLPFGNQLYVVNTVGGGDYQKKYGGAFLQKLYQEYPSLFDSEKYQYNSKNYVTDLLVMTDGERSAIPSDQPITEWSAKYMNGTNILGRGMGYVLKDWNTGTYFKLNGNNSVLPDVLTYRNSFDDNTGTQSSSSAQSSASNHETQISSSAQSSASNHEAQSSSSAQSSVSSHEVQSSSSAQSSASSHEVQSSSSAQSSASSHEVQSSSSAQSSASSYEAQSSSSAQSSASSHEVQSSSSAQSSVSSHETQSSSSAQSSASSHEVQSSSSAQSSASSNEAQSSSSAQ

SEQ ID NO: 11 - protein, 1463 aa, Lactobacillus kunkeei
MNINSNERKVRFKMYKSGKQWIVAGLTTAVISIAVYGGSSIANGGIEAKADAQNAATSSIVNTNNSTNSSNANSIASLPQNGTYSTNDNGQTWKYVSQNKDIQGLYKDNNDQLRYFNEYDGTQAKGDIVNVNNDNYYFDKDSGQGHKIDSYTGGSYSESKVNNQDGWIYKSSDNNDVKGVATVDGNIQYFDQNTGLQLKGGSAQIGGVDYYFDPNKGNLVGKVDQVVNSNDYSDNKLLDSNKNVVKGLVVNNGQLQFFDTSNGNQAKNKQVIANGITYYFDTNGNGQYLFTNTGKSAVDDFTQRNAANSVNPSDYKNVVDGFFTADTWYRPKQILDNGTTWRNSNSNELRPMITAWWPNKDVQVNYLKLMQNNGLLDKSNSYSIQSDQQTLNQAAQKAQVNIEKKISQTGNTDWLNDLLFKGNGDNPSFVKQQYIWSSDSESPWQGDAWFQGGYLKYGNSVMTPNTNSNYRDSNNLFDFLLANDVDNSNPAVQAEDLNWLYYLTNFGTITANDSNANFDSIRIDAVDFISNDIIQRSYDYLRQKFNLMQSDANADSHISLVEGGVDAGTTSYSNDGLVEAPFRLDAYPLLHKQDGDVFKNLIDEEDSGIDISNHNGETNTNNTIGGITLSGGKPNYSIVHAHDKDVQEKVGQAIIDTTGIKDWTDFTPSQLAQGLETFYNDQRQTVKKYNDYNVPSAYAIMLTNKGTVPRIYYGDMYQDDGQFMQKKSLYYDDIANLMTARKKYVSGGQSMVDNNGILTSVRFGKGANTVSDSGTEDTRNQGIGLIVGSAPKKVLNDGDTVVLHMGAAHKNQKYRALMLTTENGIQNYNSDDNAPVAETDDNGDLVFSNKDINGQANTAIKQVANPEVNGYLAAWVPVGASDDQDSRTAPSTSQNNDGNVLHENDALDSNLIFEGFSNFQPTPTNHDEYANVVIAKNASLFKDWGVTSFEMAPQYRSSQDHTFVDSTIDNGYAFSDRYDLGFGTPTKYGTDEDLRNAIKSLHDNGMQVMADVVYNQLYNLPGQEVVSATRAGVTGNTNALPFGTQLYVVNTIGGGDYQKKYGGAFLNELQEQYPSLFKSQKYKYYYKNYANNGAGPGYLTVNDAERSDIPYNQPITEWSAKYMNGTNILGRGMGYVLKDWNTGDYFKLSGSDSTLPSSLTYKSGWVENPDSTWSYYEKNNIDKLTGSQVINEERVFFDNNGIQVKGGWVKNSNGTYSYYDKNSGNILTGDQLIDGEHFFFDNNGVQVKGKWIKNSDGSKSYYDSHLGKLIKTDKKVSSNARKKKSKEELLYENALKVLRKDKKRLDKNKTKANIRKYNKSLKKYRKAKKKLLAITKNRVANARKAIKIAKKVLSKRKNINNEKRYYKALKEYYVAEKSYLKITGNYNKKYYYEFDKLTPKVKVVKNIYSYKSRHFTKKNRVKKIKKGTLVRVKSIVRSGKVARINIGNGHFITSSKDFIKMFK

SEQ ID NO: 12 - protein, 2824 aa, Leuconostoc carnosum JB16
MTAGIFSTVVFGMAVSDVSANDTDNTVLTSNSGFLDKVVDTTSTDKAATPDKVVDTTSTDKAVTPDKVADTTSTDKAVTPDKVADTTSTDKAATPDKVVDTTSTDKAATPDKVVDTTSTDKAATPDKVVDTTSTDKAATPDKVVDTTSTDKAATPDKVADTTSTDKAATPDKVVDTTSTDKAATPDKVVDTTSTDKAATPDKVVDTTSTDKAATPDKVVDTTSTDKAADRTISISGKTVKNIEEIGGKTYFVGDDGKVKKNFTVIVDGQVMYFDKESGALTSNHKQYKEGLSDITNEHNAAYSLENDNFTQIDSYLTANSWYRPKDILKSGTTWTASTDKDSRPLLMSWWPDQQTELSYLKYMQSAGFLAEDVNLSENNSIDDLTAAAMDVQKNVEAKISLSGNTDWLKEDMNQFVDSQSNWNISSESKGTDHLQGGALLYGNSDMTPDANSDYRLLNRTPKNQTGQISATNDQGGYEMLLANDVDNSNPIVQAEQLNWLHYMMNIGSITKNDSTANFDGYRVDAVDNVNADLLQIAGDYFKAAYGTDKSDANANNHISILEDWDNSDPDYVKKHGNEQLTMDFPMHLALKYALNMPIDMRSGLEPAIKTSLVNRSQDATENEAQPNYSFIRAHDSEVQTVIAQIIKDKINPKSDGLTVTPDEIAKAFEIYNADELKADKAYTAFNIPSSYALLLTNKDTVPRVYYGDLFTDDGQYMSDHSPYYDAITTLLASRIKYAAGGQSMGMTYLHDNQEVLTSVRYGKGALTADDLGNVDTRTQGIGLVISNKTDLSLKSDESVVLNMGVAHKNQAYRPAMLTTKSGLKIYDTDDGAPIVYTNNLGQLIFNADTVYGVSDPQVSGYLAAWVPVGATEDQDARTKGSHDGTTDGNVYHSNAALDSQVIYEGFSNFQAMPTTTDEYTNVKIAQNAQWFKKLGLTSFELAPQYRSSTDSSFLDSVIQNGYAFTDRYDVGYNTPTKYGTVDQLLDALRALHSQDIQAINDWVPDQIYNLPGEQIVTASRTNGSGKYDDDSVISNTLYDSRTIGGGEYQAMYGGAFLDQLKQAYPGLFETKQLSTGVAMDPDVKIKEWSAKYFNGSNIQGRGAWYVLKDWATNKYFSVSSNNTFLPKQLLGEKASTGFITNDGKTEFYSTSGYQAKNTFIEDNGNWYYFDNDGYSVVGKQVIDNKHYYFLPNGVELQDAYLSDGDKQYYYKKTGRQIVNQYYRDEQGDWRYFFADGHMALGLTDIVSNDGTHATQYFDNNGVQVKGTSERDKDGNIHYFDGTSGNLVVSSWGQLSDGSWLYLNDKGIAVTGAQQIDGQSLYFNEDGKEVKGDAVTDNQGNIRYFDGESGHMVVNSWGKLPDGSWMYLNDKGIAVTGQQKINNEVLYFNADGKQIKSAFKELVDGSWLYLNDKGIAVTGAQQIDGQSLYFNEDGKEVKGDAVTDNQGNIRYFDGESGHMVVNSWGKLPDGSWMYLNDKGIAVTGQQKINNEILYFDADGKQLKNTLKTLSDGSRIYLDGKGVSATGVQKINGKVSYFDVNGKQVSNHIQELPDGSWMYLDNDGLALIGNQDVDGKQLYFDVDGKQIKNDKVKNSDGTINYYTGTVGEKLKHDFGQLSDGSWMYLDENGNAVTGEQNINGQHLYFKDDGQQVKGDVFEDDLGRMRYYSANSGEMVVNQFEQISDGAWAYFGDDGVAVTGEQHINGQDLFFDATGQQVKGESRTINGIPYTFEKESGEKRSVNIAPLLAMGNYVTNNGTDWQYEVQGNPVKGLYSTSDNKLRYFDLTTGVQIKGNFVTIGHNTYYFNPANGDGELLPDVSDGHYGTIQVKDANTNEKTVWVYRNQSNTILKGIQNIHGNIQYFDLSTGEQIKGGIANYDGNDYYFESAKGNLTSKIKQVYTDGQYVTKDGKSIYEDAQQQSVSGLVSINGQLQYFNPQDGVQVKNQQIIVDGVTYYFDENGNGQYLFTNTTVMPMDDFTKHNTVYSDNDNNFKNNVDGFLTADTWYRPKEILKAGTTWTTTSESDMRPLITTWWPNKNVQVNYLNFMKQNNLLHTNVEYSLLSDQYDLNIAAQAVQTAIEKRIAQENSTDWLQNLLFTAQDDQPSFVKQQFIWNKDSEYQGKGDAWFQGGYLKYGNNKLTPNTNSNYRKTDNAFEFLLANDIDNSNPVVQAENLNWLEYLMNFGTITGKDDDANFDSIRVDAVDFISNDTIQRTYDYLRDAYQVDQSEAKANQHISLVEAGLDAGTSTVKNDALIESNLREAATLSLANASGKNSALTNMLQDVDGGTLIADHTHNSTENEATPNYSIIHAHDKGIQEKVGAAISDATGADWTNFTDTQLKSGLDLYYKDQRATDKKYNIYNLPSIYALMLTNKDTVPRVYYGDMYQDNGQYMAEKSIYYNALESLMSARKSYVSGGQTMDVDSHGLLKSVRFGKGAMTADTVGNEETRTEGIGVLVGNDASLKLNDSDTVTLDMGAAHKNQKYRAAILTTNNGLSTFDSDKDAPIAWTNDKGILTFSNKNVSGQDNTNVHGVANPQVSGYLAVWVPVGAKDDQNAGTSASTVVNTDGKVLHSNASLDSNLIFEGFSNFQPRATTNDELTNVVIAKNADLFQKWGITSFEMAPQYRSSQDHTFLDSTIDNGYAFTDRYDLGFNTPTKYGTDSDLRLAIKSLHKAGMQVMADVVDNQVYNLPDQEVVSASRAGVYGNDVATGFDTQLYAVNSVGGGKYQAQYGGQYLSELKNKYPDLFEAKAYDYWTKNYANDGSNPYYTLSQQTRDDIPSDEKIKQWSAKYMNGTNVLGHGMGYVLKDWNTGQYFKINKDGDSNLPV

SEQ ID NO: 13 - protein, 2771 aa, Leuconostoc mesenteroides; identical to SEQ ID NO: 1

SEQ ID NO: 14 - DNA, 8316 bp, Leuconostoc mesenteroides
gtgacagccggtattttttctgctgtgatatttggcgtttccacaactaacgtaagcgctgatagcactaacaacactggtgttacggtgtcacaagcaacagataaagtagcagacacgacggctacaacggacaaagtagcggacacaacagctacaacagataaagtggccgacacagcagctacaacggacaaagtagcggacacaacagctacaacagataaagtggccgacacagcagctacaacggacaaagtagcggacacaacagctacaacagataaagtggccgacacagcagctgcaacagataaagcagccgatacagcggctacaacggataaagtggccgacacagcagctgcaacggataaagtagcggacacagtagctgcaacggacaaagtagcggacacaacagctacaacagataaagcagccgatacagcggctacaacggataaagtaaccgacacaacagctgcaacggataaagcagcggacacgacggctacaacagataaagtggccgacacaacagccacaacatcagaaaaatcaaaaagtattaaacaaattgatggtaaaacttatttcattggtaatgatggtcagcctaagaaaaattttacagccattgttgacggtcaagtattatatttcgacaaagatactggtgctttgacatcaaatagtagtcaatataccgatggtttagccaatataggaaatgagcataatgcggcttattcattgtcttcggatagttttacacaagttgatggctatctaacggctaacagttggtaccgacctaaagatatattaaaaaatggtacaacttggacggctgcaacagcaaacgattttcgaccattgttaatgtcttggtggccagataaagatacccaagtttcatacttaaaatatatgcaatctgcgggattattatcagatgacgttgcattatcaaacaatgatagtatgaacagtttgacggatacggctatgactgttcaaaaaaaaattgaagaaaaaattggcttattgggcagtactgactggcttaaggccgatatgaaccaaatggttgattcacaatcgaattggaacattagtagtgagtctaaaggaacagatcatttgcaaggtggtgcgctcctatacgttaatagtgatttaacaccaaatgccaattctgattatcgtttattaaatcgaacgccaactaaccaaaaaggtcaaattacaacaaatggtaatcaaggtggctatgagatgctgttggccaacgatgttgataattctaacccaattgttcaagctgaacaattaaattggttatactacatgatgaatatcggtagcatcgcccaaaatgatccaacagcaaattttgacggttacagagttgatgctgttgataacgtgaatgctgacttgttgcaaattgctggagattattttaaagcagcatatggaacaaatcaaagtgacgctaatgcaaacaatcacatttccatcttagaagactgggacaataatgatccagcgtatgtaaaagcacaggggaacaaccaattaaccatggattttccaatgcatttggcattgaagtattcattgaatatgccaagtagtgctcgtagcggtttggaaccagcaatttcaacaagcctagtaaatcgtgcagcagacgccacagaaaatgaagcccaaccgaactattcatttattcgtgcacatgatagtgaagtacaaacggttattgctcaaattattaaagataaaattaatcctagttccgatggattgactgtctcaacagatgaaattgccaaagcattcgaaatatataatgctgacgaattaaaggctgataaagagtataccgcatataatataccctcatcatatgcattgatgttaactaacaaagatacaattcctcgtgtgtattatggtgatttgtttacggatgatggacaatatatgtctgcaaaatcaccatattatgatgcacttacttcattgcttcaatcgcgagtaaaatatgtttcaggtggtcaatctatgaatatgacttaccttcataataatcaaggccttttgacgtcagtccgctatggaaaagacgccatgacagctaacgacactggtacaagtgaaacgcgcacacaaggtattggattaattgtcggcaacaaaactgatttaaacctgaataatgatgagcaaattgtacttaacatgggggccgcacacaaaaatcaagcttaccgtgcattaatgttaagtactaaagatggcttgaaaatttataataatgatgacgaggcaccggtatcgtatacagatgaccaaggccgtttgatttttaaatctgatgtggtttatggtgtgagtgatgctcaggtttctggttatttagcagcttgggtgccagtcggtgcaaacgatagccaagatgctagaacagaaagtagtacaacagcgtcaacagatggtaatacctatcattcaaatagtgccttagattctcaacttatatatgaaggcttttcaaacttccaagccatgccaacacaggccgatgagtataccaatatcaagattgccgaaaatgcacaattattcaagagccttgggataacaagctttgaattggcacctcaataccgttcaagtacggataacagtttcttagattcagttattcaaaatggctatgccttcacggatcgctacgacattggttataatacgcctacaaagtacggtacagttgaccaactattagatgctttaagagcattgcatgctcaaggcattcaggctatcaatgattgggtcccagaccaaatttataatttgcctggggaagaaatagtgacagccagtcgaacaaacggttcgggaaaggtgaatgaaagttcagttattaataatacgctatatgattctcgtactgttggtggcggagagtatcaagcaatatatggaggtgctttcttagataagttaaaacaagattatcctgagttatttgaaacaaaacaaatttcaacaggtgaagcaatgaaccctgatgtcaaaatcacagaatggtcagctaagtattttaatggctcaaacattcaaggacgtggtgcatggtatgttctcaaggattggtcaacaaatcaatactttaatgtttcaagtggtagtgaatttttacctaagcaactgttaggcgaaaaaacaagtacagggtttaccaacgtggacaatggcaagactgagttttattctacgagtggctaccaagcaaagaatacatttattcaagataatgacaattggtattattttgataatgatggctatatggttgttggcggtcaagaaattaatggtaaaaaatattatttcctaccaaatggtgtagagttacaagatgcttatttgtctgatgggactagtgagtattactacagtagtgatggtcgtcaaatttctaatcaatattatcaaggatcagacaacaactggcgttatttctttgcagatggtcatatggctgtagggttagcaacaattactacagaaaatggtacaacaaatcaacaatatttcgatgcaaatggtgtgcaacttaagggcgtagctataaaggatactgatggcaatgtgcactattttgatggcaagacaggaaacatggttataaattcctggggtaaaataagcgatggttcatggttatacttaaatgatagcggtgtagcggtcacaggaccgcaaaatattaacggccaaaatctttacttcaacgaagacggtattcaagtaaagggtgaagccattactgataatagtggaaacatacattattatgatcgcagcacaggaaatatggttgtgaactcatggggtgaaacgaataatggttcatggctatacttgaacgacaagggtgatgccgttacaggagaacaagttattgacggtcaaaaactatatttcagtagtaatggaatccaacttaaaaatacattcaagaagctatccgatggttcatggctatatttgaacgataaaggtcttccagtgacaggagcacaggtcattgatggacaaaacttgtatttcgaccaagatgggaagcaagtcaagggtgacgttgctacagatggacaaggtaacactcattattatgatggcaacacaggaaatatggttactaattcatgggcagagttaccggacggttcatggatgtatctagacaatgatggcaatcctttaacaggacagcaaaagattgatggccagtcactctactttaatgatgctggtaagcaaatcaaaaacgcattggttaaactagatgatgggtcaacaatttacctcgatgataaaggtgtttcatcaactggtattcaaagaattgatgataagatatattattttgatcctgatggtaaacaagtagtatgtcgttttgaagaattaccagatggttcatggatgtatctagatgatgacggtgttgctgctacgggcgctcaaaaaattaatggccaggaattatatttcgacaatagcgggaaacaagtcaagaacgacaaagtaattaatgacgatggaacaataaactattacacaggtatgagcggtgaaaaactaaaaaatgattttggtgaattaccagacggttcatggatgtacttggataatcaaggtaatgctgtaataggtgcccaaaaaattaatggccagaatctttacttcaagacagacggacgacaggttaagggtgaagcaaatgttgattcatcaggtgaaatgcacttctatgatcctgattctggcgagctaattacaaatagatttgaacaagttgctagtggtgtatgggcttactttgatgccaaaggtgttgctgtaactggtgagcaacgcattggtaagcaaaatttattttttgatccaactggttatcaagttaaaggcgacaaacgaacaattgacggcgttctctatacctttgataaagaaagtggtgagagaaagggtttagattctatatcggtattacccaccaatggacaatacacaaccgataaggcccaaaattggtattaccaagtcgatggtgaaaatgtaaaagggctatatacaaataatgatggtcaattacgttacttcgatttgacaactggcgtgcagactaaaggtaattttgtgacaattggcaatgatacctactatttcaccaaggaacaaggggatggacagatagtttctgaggttgtgtcaggacactatggtactgtccagttgagtgacaattcgtctgcatgggtttatcgcggtgcaaatgatcaaattttgaaaggcctacagaatataaacggtcgtctgcaatattttgatctaaccaccggtgcgcaattaaaaggcggtgctgcaaactatgatggcaacctttattattttgaatcatcagatggtaacctagtcagtaaaattcagcaatcttattctactgggaattatgtgaccgatggtgataaagtaacatatgctgatgagcaaaacaaccaagtcacgggattagcgttgattgatgatcaactacaatacttcgatccaagtgacggtcgtcaagtcaagaatgagcaggttatcgttgatggcgtcacatactactttgataaaaatggtaatggacaatacttgtttacaaatactgcaacgatgtcaactaatgaatttgccaaacatagtgctgcttatagcaatgatagttctagcttcaagaatacgatagatggtttcttgacggccgatacctggtatcgccctaaagatatcttggaaaacggacaaacgtgggtagtttcttcaacaaatgacgtgcgaccactgataacagtttggtggctaaataaagatgttcaagttaattattcaaattttatgaagcaaaatggtttgctagatacaagtagtcaatttaatctacaatctgatcaatatgacttgaatgtcgccgcgcaaaaagttcaagtggctattgaaaaacgcatttcgaaagaaaagagtacagattggttgaaagatcttttgtttgaagctcatgaagatacgccttcatttgtgaaacaacaatttatttggaataaagattctgaatatcaaggtcaaggggatgcgtggttccaaggtggttatctgaaatatggtaacaatgaattaaccccaacaacgaactcagattatcgtgaatccggtaatacattagacttcttgcttgctaatgatgtcgacaattctaacccagcggttcaagctgaaaatttgaattggttacattatttaatgaactttggcacgattacagctaatgatgatgatgctaattttgacagtattcgtattgatgccgttgactttattgataatgatgccattcagagaacctacgattacatgcgtgatgcttataaagttgatgcaagtgaagacaacgctaataagcatatttcactagtggaagctggattagatgctggtacctctacaattaagagtgatgctttagttgaatctaactttagagaggcagctacactatcgctagcaaatcaatcaggggaaaatagttccttgactaatatgttgcaagacattgatggtggccagattatagctgatcacgccaacaatgcaacagaaaatgaatcaacgccaaattattcaattattcatgctcatgataaggggattcaagaaaaggttggtgcagcaattaccgacgttactggtgcagactggacgaatttcaccgatgaccaattaaaagaaggattagcagcttattatcaagatcaacgttcaacgaataaaaagtataacatctataacttacctagtatctatgctttaatgttgaccaataaggacacagttcctcgtgtttattacggtgatatgtatcaagatgatggccagtatatggaaaagcaaagtatttattatgatgccattgtttccttgatgaacactagaaagagttatgtgagtggtgggcaaactatggatgtagatgaacatggtttgttgaagagtgttcgttttggtaaagacgcaatgacagctagtgaccttggtacgaatgaaacacgcactgaaggtgttggtgtgctggtcggcaatgattcttcactaaaactaaatgattcagatacagttactttagagatgggggcggctcataaaaaccaaaagtaccgagctgcattgttgacaactagtgatggtattgttacgtatgatgctgataatgatgcaccaacaatctggacagatgaccgtggtacattgacgttctcaaataaggagattgctggtcaagattatactagtgtgcaaggattcgctaattcacaagtatcaggttacttagcagtttgggtgcccgtaggagctagtgacgatcaagatgtccgaacagcagcattaacagatgcaaatcttgatgacaaagtactgcattctaatgctgcattagattcgaacttgatttacgaaggcttttctaactttcaacctaaagcaaccaccaatgatgaattgactaacgtagtaattgctaaaaatgctaatttatttgaaaagtggggaatcacaagttttgagatggcaccacaatatcgttcaagtggggaccacacgttcttagattcaacgattgataatggttatgcatttactgaccgatacgatttgggatttgaaacaccaactaagtacggtactgataaggatttgcgtactgcaattaaagcattgcaccaatcaaatatgcaggttatggctgatgtagttgataaccaagtttataatttatctggacaggaggtcgtatcagcttcacgtgccggtgtttacggcaatgatgtgtcaactggatttgggacacaactctatgcggttaatagtgttggtggtggtaaatatcaagcccaatacggtggtgaatatttgaatgaattgaagcaacaatacccagatttgttcgaagctaagacgtatgactattgggttaaaaattattcaaatgacggatcggatccgtattacacactgtcgcaaaacacacgaaaagatatgccaagtagtgaggtcattaaacaatggtcagctaaatatatgaatggtactaatgtattaggaaacggtatgggatatgttttgaaagattggaatacaggtgagtatttcaaaattggagaaaagaatgctgattttataacaaattaa

SEQ ID NO: 15 - DNA, 8466 bp, Leuconostoc mesenteroides
gtgacagccggtattttttctgctgtgatatttggcgtttccacaactaacgtaagcgctgatagcactaacaacactggtgttacggtgtcacaagcaccagataaagtagcggacacaacagctacaacagataaagtagcagacacgacggctacaacggataaagcagcggacacaacagctacaacagataaagtggccgacacagcagctgcaacggacaaagtagcggacacaacagctacaacggacaaagtagcggacacaacagctacaacagataaagtggccgacacagcagctgcaacggacaaagtagcggacacaacagctacaacagataaagtagcggacacaacagctacaacggacaaagtagcggacacaacagctacaacagataaagtagcggacacagcagctgcaacggataaagcagcggacacgacggctacaacagataaagcagcggacacgacggctacaacagataaagtggccgacacagcagctacaacagataaagcagcggacacgacggctacaacagataaagtggccgacacagcagctacaacagataaagcagccgatacagcggctacaacggataaagtaaccgacacaacagttgcaacgaataaagcagtggacacaacagctacaacagataaagtggacgacacaacagccacaacgtcagaaaaatcaaaaagtattaaacaaattgatggtaaaacttatttcattggtgatgatggtcagcctaagaaaaattttacagccattgttgacggtcaagtattatatttcgacaaagatactggtgctttgacatcaaatagtagtcaatataccgatggtttagtcaatataggaaatgagcataatgcggcttattcattgtcttcggatagttttacacaagttgatggctatctaacggctaacagttggtaccgacctaaagatatattaaaaaatggtacaacttggacggctgcaacagcaaacgattttcgaccattgttaatgtcttggtggccagataaagatacccaagtttcatacttaaaatatatgcaatctgcgggattattatcagatgacgttgcattatcaaacaatgatagtatgaacagtttgacggatacggctatgactgttcaaaaaaacattgaagaaaaaattggcctattgggcagtactgactggcttaaggccgatatgaaccaaatggttgattcacaatcgaattggaacattagtagtgagtctaaaggaacagatcatttgcaaggtggtgcgctcctatacgttaatagtgatttaacaccaaatgccaattctgattatcgtttattaaatcgaacgccaactaaccaaaaaggtcaaattacaacaaatggtaatcaaggtggctatgagatgctgttggccaacgatgttgataattctaacccaattgttcaagctgaacaattgaattggttatactacatgatgaatatcggtagcatcgcccaaaatgatccaacagcaaattttgacggttacagagttgatgctgttgataacgtgaatgctgacttgttgcaaattgctggagattattttaaagcagcatatggaacaaatcaaagtgacgctaatgcaaacaatcacatttccatcttagaagactgggacaataatgatccagcgtatgtaaaagcacaggggaacaaccaattaaccatggattttccaatgcatttggcattgaagtattcattgaatatgccaagtagtgctcgtagcggtttggaaccagcaatttcaacaagcctagtaaatcgtgcagcagacgccacagaaaatgaagcccaaccgaactattcatttattcgtgcacatgatagtgaagtacaaacggttattgctcaaattattaaagataaaattaatcctagttccgatggattgactgtctcaacagatgaaattgccaaagcattcgaaatatataatgctgacgaattaaaggctgataaagagtataccgcatataatataccctcatcatatgcattgatgttaactaacaaagatacaattcctcgtgtgtattatggtgatttgtttacggatgatggacaatatatgtctgcaaaatcaccatattatgatgcacttacttcattgcttcaatcgcgagtaaaatatgtttcaggtggtcaatctatgaatatgacttaccttcataataatcaaggccttttgacgtcagtccgctatggaaaagacgccatgacagctaacgacactggtacaagtgaaacgcgcacacaaggtattggattaattgtcggcaacaaaactgatttaaacctgaataatgatgagcaaattgtgcttaacatgggcgccgcacacaaaaatcaagcttaccgtgcattaatgttaagtactaaagatggcttgaaaatttataatagtgatgacgaggcaccggtatcgtatacagatgatcaaggccgtttgatttttaaatctgatgtggtttatggtgtgagtgatgctcaggtttctggttatttagcagcttgggtgccagtcggtgcaaacgatagccaagatgctagaacagaaagtagtacaacagcgtcaacagatggtaatacctatcattcaaatagtgccttagattctcaagttatatatgaaggtttttcaaacttccaagccatgccaacacaggccgatgagtataccaatatcaagattgccgaaaatgcacaattattcaagagccttgggataacaagctttgaattggcacctcaataccgttcaagtacggataacagtttcttagattcagttattcaaaatggctatgccttcacggatcgctacgacattggttataatacgcctacaaagtacggtacagttgaccaactattagatgctttaagagcattgcatgcccaaggcattcaggctatcaatgattgggtcccagaccaaatttataatttgcctggcgaagaaatagtgacagccagtcgaacaaacggttcgggaaaggtgaatgaaagttcagttattaataatacgctatatgattctcgtactgttggtggcggagagtatcaagcaatatatggaggtgctttcttagataagttaaaacaagattatcctgagttatttgaaacaaaacaaatttcaacaggtgaagcaatgaaccctgatgtcaaaatcacagaatggtcagctaagtattttaatggctcaaacattcaaggacgtggtgcatggtatgttctcaaggattggtcaacaaatcaatactttaatgtttcaagtggtagtgaatttttacctaagcaactgttaggcgaaaaaacaagtacagggtttaccaacgtggacaatggcaagactgagttttattctacgagtggctaccaagcaaagaatacatttattcaagataatgacaattggtattattttgataatgatggctatatggttgttggcggtcaagaaattaatggtaaaaaatattatttcctaccaaatggtgtagagttacaagatgcttatttgtctgatgggactagtgagtattactacagtagtgatggtcgtcaaatttctaatcaatattatcaaggatcagacaacaactggcgttatttctttgcagatggtcatatggctgtagggttagcaacaattactacagaaaatggtacaacaaatcaacaatatttcgatgcaaatggtatgcaacttaagggcgtagctataaaggatactgatggcaatgtgcactattttgatggtaagacaggaaacatggttataaattcctggggcaaaataagcgatggttcatggttatacttaaatgatagcggtgtagcggtcacaggaccgcaaaatattaacggtcaaaatctttacttcaacgaagacggtattcaagtaaagggtgaagccattactgataatagtggaaacatacattattatgatcgcagcacaggaaatatggttgtgaactcatggggtgaaacgaataatggttcatggctatacttgaacgacaagggtgatgccgttacaggagaacaagttattgacggtcaaaaactatatttcagtagtaatggaatccaacttaaaaatacattcaagaagctatccgatggttcatggctatatttgaacgataaaggtcttccagtgacaggagcacaggtcattgatggacaaaacttgtatttcgaccaagatgggaagcaagtcaaaggtgacgttgctacagatggacaaggtaacactcattattatgacggcaacacaggaaatatggttactaattcatgggcagagttagcggacggttcatggatgtatctagataatgatggcaatcctttaacaggaccgcaaaagattgatggccagtcactctactttaatgatgctggtaagcaaatcaaaaacgcattggttaaactagatgatgggtcaacaatttacctcgatgataaaggtgtttcatcaaccggtattcaaagaattgatgataagatatattattttgatcctgatggtaaacaagtagtatgtcgttttgaagaattaccagatggttcatggatgtatctagatgatgacggtgttgctgctacgggcgctcaaaaaattaatggccaggaattatatttcgacaataacgggaaacaagtcaaaaatgacaaagtaattaatgacgatggaacaataaactattacacaggtatgagcggtgaaaaactaaaaaatgattttggtgaattaccagacggttcatggatgtacttggataatcaaggtaatgctgtaataggtgcccaaaaaattaatggccagaatctttacttcaagacagacggacgacaggttaagggtgaagcaaatgttgattcatcgggtgaaatgcacttctatgatcctgattctggcgagctaattacaaatagatttgaacaagttgctagtggtgtatgggcttactttgatgccaacggtgttgctgtaactggtgagcaacgcattggtaagcaaaatttattttttgatccaactggttatcaagttaaaggcgacaaacgaacaattgacggcgttctctatacctttgataaagaaagtggtgagagaaagggtttagattctatatcggtattacccaccaatggacaatacacaaccgataaggcccaaaattggtattaccaagtcgatggtgaaaatgtaaaagggctatatacaaataatgatggtcaattacgttacttcgatttgacaactggcgtgcagactaaaggtaattttgtgacaattggcaatgatacctactatttcaccaaggaacaaggggatggacagatagtttctgaggttgtgtcaggacactatggtactgtccagttgagtgacaattcgtctgcatgggtttatcgcggtgcaaatgatcaaattttgaaaggcctacagaatataaacggtcgtctgcaatattttgatctaaccaccggtgcgcaattaaaaggcggtgctgcaaactatgatggcaacctttattattttgaatcatcagatggtaacctagtcagtaaaattcagcaatcttattctactgggaattatgtgaccgatggtgataaagtaacatatgttgatgagcaaaacaaccaagtcacgggattagcgttgattgatgatcaactacaatacttcaatccaagtgacggtagtcaagtcaagaatgagcaggttatcgttgatggcgtcacatactactttgataaaaatggtaatggacaatacttgtttacaaatactgcaacgatgtctactaatgaatttgccaaacatagtgctgcttatagcaatgatagttctagcttcaagaatacgatagatggtttcttgacggccgatacctggtatcgccctaaagatatcttggaaaacggacaaacgtgggtagtttcttcaacaaatgacgtgcgaccactgataacagtttggtggccaaataaagatgttcaagttaattatttaaattttatgaagaaaaatggtttgctagatacaagtagtcaatttaatctacaatttgatcaatatgacttgaatgtcgccgcgcaaaaagttcaagtggctattgaaaaacgcatttcgaaagaaaagagtacagattggttgaaagatcttttgtttgaagctcatgaagatacgccttcatttgtgaaacaacaatttatttggaataaagattctgaatatcaaggtcaaggggatgcgtggttccaaggtggttatctgaaatatgataatagtgaattaaccccaacaacgaactcagattatcgtgaatccggtaatacattagacttcttgcttgctaatgatgtcgacaattctaacccagcggttcaagctgaaaatttgaattggttacattatttaatgaactttggcacgattacagctaatgatgatgatgccaactttgacagtattcgtattgatgccgttgactttattgataatgatgccattcagagaacctacgattacatgcgtgatgcttataaagttgatgcaagtgaagacaacgctaataagcatatttcactagttgaagctggattagatgctggtacctctacaattaagaataatgctttagttgaatctaactttagagaggcagctacactatcgctagcaaatcaatcagggaaaaatagttccttgactaatatgttgcaagacattgatggtggccagattatagctgatcacgccaacaatgcaacagaaaatgaagcaacgccaaattattcaattattcatgctcatgataaggggattcaagaaaaggttggtgcagcaattaccgacgttactggtgcagactggacgaatttcaccgatgaccaattaaaagaaggattagcagcttattatcaagatcaacgttcaacgaataaaaagtataacatctataacttacctagtatctatgctttgatgttgaccaataaggacacagttcctcgtgtttattacggtgatatgtatcaagatgatggccagtatatggaaaagcaaagtatttattatgatgccattgtttccttgatgaacactagaaagagttatgtgagcggtggacaaaccatggatgtagatgaacatggtttgttgaagagcgttcgttttggtaaagacgcaatgacagctagtgaacttggtacgaatgaaacacgcactgaaggtgttggtgtgctggtcggtaatgattcttcactaaaactaaatgattcagatacagttactttagagatgggggcggctcataaaaaccaagagtaccgagctgcattgttgacaactagtgatggtattgttacgtatgatgctgataatgatgcaccaacgatctggacagatgaccggggtacattaacgttctcaaataaggagattgctggtcaagattatactagtgtgcaaggattcgctaatccacaagtatcaggttacttagcagtttgggtgcccgtaggagctagtgacgatcaagatgcccgaacagcagcatcaacagataaaaatactgatgacaaagtactgcattctaatgctgcattagattcgaacttgatttacgaaggtttttcgaactttcaacctaaagcaaccaccaatgatgaactgactaacgtagtaattgctaaaaatgctaatttatttgaaaagtggggaatcacaagttttgagatggcaccacaatatcgttcaagtggggaccacacgttcttagattcaacgattgataatggttatgtatttactgaccgatacgatttgggatttgaaacaccaactaagtacggtactgataaggatttgcgtactgcaattaaagcattgcaccaatcaaatatgcaggttatggctgatgtagttgataaccaagtttataatttatctggacaagaggtcgtatcagcttcacgtgctggtgtttacggcaatgatgtgtcaactggatttgggacacaactctatgcggttaatagtgttggtggtggtaaatatcaagcccaatacggtggtgaatatttgaatgaattgaagcaacaatacccagatttgttcgaagctaagacgtatgactattgggttaaaaattattcaaatgacggatcggatccgtattacacactgtcgcaaaacacacgaaaagatatgccaagtagtgaggtcattaaacaatggtcagctaaatatatgaatggtactaatgtattaggaaacggtatgggatatgttttgaaagattggaatacaggtgagtacttcaaaattggagaaaagaatgctgattttataacaaattaa

SEQ ID NO: 16 - DNA, 8535 bp, Leuconostoc carnosum
atgagagacaagaatgtaatatgcgatcgaaaaaaattgtataaatccggaaaattgttagtgacagcaggaattttctctacggttgtgtttggtatggccgtatctgacgttagtgctaatgacactgacaacactgtgttaacttcgaacagtggatttttagataaagtagtagatacgacaagtacggataaggcagccacaccagataaagtagtagatacgacaagtacggataaggcagtcacaccagataaagtagcagatacgacaagtacggataaggcagtcacaccagataaagtagcagatacgacaagtacggataaggcagccacaccggataaagtagtagatacgacaagtacggataaggcagccacaccggataaagtagtagatacgacaagtacggataaggcagccacaccggataaagtagtagatacgacaagtacggataaggcagccacaccagataaagtagtagatacgacgagtacggataaggcagccacaccggataaagtagcagatacaacgagtacggataaggcagccacaccagataaagtagtagatacgacgagtacagataaggcagccacaccagataaagtagtagatacgacgagtacagataaggcagccacaccagataaagtagtagatacgacaagtacagataaggcagccacaccggataaagtggtagatacgacaagtacggataaggcagcagatagaaccattagtatttctggtaaaacagttaaaaatattgaggaaattggtgggaaaacttattttgtaggggatgatggcaaagtcaaaaaaaacttcacggttattgttgatgggcaagtaatgtattttgacaaagagtctggagcattgacttcgaaccataagcaatataaagaaggtctttcagatataacaaatgaacataatgctgcctattcattagaaaacgacaactttacacaaattgatagttacttaactgccaatagttggtaccgtccaaaagatatattaaaaagtggcacaacatggacagcctcaaccgataaagactctcgcccattacttatgtcatggtggccagatcaacaaacagaactatcttatttaaagtatatgcaatcagcaggtttcttagcagaggatgttaatttatcagaaaataatagcattgatgatctaacagctgcagcaatggatgttcagaaaaatgttgaagcaaagattagcctatcaggtaatacagattggttgaaagaagatatgaatcagtttgttgattcacagtcaaattggaatatcagcagtgagtcaaaaggcactgatcatcttcagggcggcgctttattgtatggtaacagtgatatgacaccagatgctaattctgattatcggttactgaatcgcacaccaaaaaaccaaaccggacaaatcagtgctacgaatgatcagggtggttatgagatgttattggctaatgatgtcgataattctaatccaattgttcaagccgaacaattaaattggttacactacatgatgaacattggtagtattacaaaaaatgattcaacggctaattttgatggttatagagttgatgcggtagataacgtgaacgctgatttgttacaaattgctggtgactacttcaaggccgcttatgggacggacaaaagtgatgcaaatgctaataatcatatttctattcttgaagattgggataatagtgatcctgactacgtcaaaaagcacgggaatgaacaattaactatggattttccgatgcatttggcattaaaatatgctttaaatatgcctattgatatgcgtagtgggcttgaaccggcaattaagacaagtctggtgaaccgatcacaagatgcaacagaaaatgaggcacagccaaactactcgtttatacgtgcccatgatagtgaagtacagactgttattgctcaaattattaaagataaaattaatccaaagtcagatggtttgacagttacacctgatgaaattgcgaaagcttttgaaatctataatgcagatgaactaaaagctgataaggcatacacagcttttaatatcccgtcatcttatgcacttttgttgactaataaagatacggtgcctcgtgtttactatggcgatttatttacagatgatggacaatatatgtctgatcattcaccatattatgatgctattacgactttattagcgtcacgtattaaatatgcggctggtggtcaaagcatgggtatgacgtatttacacgataatcaagaagttttgacatctgtacgttatggtaaaggggctctgacagcagatgatttgggtaatgttgacacacgtacacaaggtattggacttgttatcagtaataaaacggatttgagtttaaagagtgatgagagcgttgtgctgaatatgggtgtcgcacataaaaatcaagcatatcgcccggcaatgttgactactaagtcaggattaaaaatttacgatactgatgatggtgcaccaattgtttatacaaataatttaggacagctaatttttaacgcagatacagtctatggtgtgagtgatccacaagtttcagggtaccttgctgcgtgggttcctgttggcgcaactgaagatcaagatgctagaactaaaggcagtcatgatggaacaactgatgggaatgtctatcattccaacgctgcattagattctcaggtcatatatgaaggtttctctaatttccaggcaatgccaacgaccactgatgaatatactaacgtaaagattgcacaaaatgcacagtggtttaaaaaattaggactgacaagttttgaactggcaccgcaatatcgttctagcacagatagtagctttttagactctgttattcaaaatggatacgcttttactgatcgatatgatgtgggttataatacaccaacaaaatatggtacagtcgatcaattattagatgcattgagagcattacattcacaagatatccaagcaattaatgattgggtacctgatcaaatttataacttacccggggagcaaattgtaacagcgagtcgtaccaatggatccggaaaatacgatgatgattcagtgattagtaatactttatatgattcacgtactatcggtggtggagaatatcaagcgatgtatggcggggctttcttagatcaattgaagcaagcatatcctggtttgtttgaaacaaaacagctttctactggtgttgcaatggatcctgatgtaaaaataaaagaatggtctgctaagtattttaatggttctaacattcaagggcgtggtgcttggtatgtactaaaagactgggcaactaataagtacttcagtgtctcgagtaataatacatttttacctaagcaattattgggtgaaaaagctagtacaggatttattacgaacgatggaaaaacagaattttattcaacaagtggctaccaggcaaagaatacatttattgaagacaacggtaactggtattacttcgataatgatggttatagcgtagttggaaagcaagtgattgataataaacactactatttcttgcctaatggtgtcgaattgcaagatgcctatttatcagatggggataagcaatattattataaaaaaactggtcgacaaatagtaaatcagtattatagagatgagcaaggtgattggaggtatttctttgcagatgggcatatggctcttgggttaactgacattgtttcaaatgatggaactcatgcgacacagtattttgataacaatggtgttcaagtgaaaggaacatcagaacgagataaagatggtaatattcactattttgatggtacatctggtaatttagttgttagttcatggggacaattgtcggacggatcatggctttacctgaatgataaaggcattgctgttacgggtgctcaacaaattgatggtcaatcactatactttaatgaagatggtaaagaagtaaagggtgatgcggtaacagataatcaagggaatatacgttattttgatggtgaatctggtcacatggtggttaattcatggggtaaattacctgatggttcatggatgtatttgaatgataagggtattgctgttaccgggcaacaaaaaatcaacaatgaagtcttatatttcaatgctgatggtaagcaaatcaaaagtgcatttaaagaactagtggacggatcatggctttacctgaatgataaaggcattgctgttacgggtgctcaacaaattgatggtcaatcactatactttaatgaagatggtaaagaagtaaagggtgatgcggtaacagataatcaagggaatatacgttattttgatggtgaatctggtcacatggtggttaattcatggggtaaattacccgatggttcatggatgtatttgaatgataagggtattgctgttaccgggcaacaaaaaatcaacaatgaaatcttatattttgatgctgatggtaagcagttaaagaatacactgaaaacattatccgatggttcacgtatttatttggatggtaaaggtgtttctgcaacaggtgttcaaaaaattaatggtaaagtgtcatactttgatgttaatggcaaacaagttagcaatcatattcaagaactccctgatggttcatggatgtacctagataatgatggattagctctaattggtaatcaagacgttgatggcaaacaactttactttgatgttgatggtaagcaaataaaaaatgacaaagtcaaaaatagtgatggaacaattaattattacacgggtactgttggtgaaaaactaaagcatgattttggtcagttatccgatggttcgtggatgtatttagatgaaaatggtaatgctgttactggtgaacaaaatattaatgggcaacatttatactttaaagatgatggacagcaagttaaaggagatgtttttgaggatgacttaggccgtatgcgttattatagtgctaactcaggtgagatggttgtcaatcaatttgaacaaatttctgatggtgcctgggcttactttggtgatgatggtgtggcggtaactggtgaacaacatatcaatggacaagatcttttctttgatgcgacaggtcaacaggttaaaggtgaaagtcgaaccattaatggtattccttatacctttgaaaaggagagtggtgagaaacggtctgttaatatagcaccattactagccatgggaaattatgttacaaataatggtacagattggcaatatgaagtgcaaggcaatcctgttaaagggttatatagcacttctgataataagttgcgttattttgatctgacaacaggtgtacagattaaaggcaactttgttactattggacataacacatactatttcaatccagctaatggagacggtgaattattgccagatgtttctgatggccattatggtacgatccaagttaaagatgcgaatacaaatgaaaagacagtttgggtttaccgtaatcaaagtaatactattttgaaaggtattcaaaatattcatggtaatatacaatactttgacttatcaactggggagcaaataaagggtggtattgcaaactatgatggcaatgattattactttgaatcagcaaagggtaacctcacaagtaaaattaagcaagtctatacagatggtcaatatgtaactaaagatggaaaaagcatttatgaagacgcacaacaacaaagtgtcagtgggttagtgtctattaatggtcagttacaatacttcaatccacaagatggcgtacaagttaaaaatcaacaaattattgttgatggcgttacttactactttgatgaaaatggcaatggtcagtatttgtttacgaatacaacggtcatgccaatggatgattttacaaagcacaatacagtttatagtgataacgacaacaactttaaaaataatgttgatgggttcttaactgctgatacatggtatcgtccaaaggaaatcttaaaagcaggaacaacttggacaacaacatcggaaagtgacatgagaccactgatcacgacatggtggccaaataaaaatgtgcaagttaactatctaaactttatgaaacaaaataatctattgcacacaaatgtggagtatagcttgctatctgaccaatatgatttgaatattgcagctcaagcagtacaaacagctattgaaaagcgaattgctcaagaaaatagcactgattggttgcaaaatcttctattcacagctcaagacgatcaaccatcttttgttaagcaacagtttatttggaataaagattctgaataccaaggaaaaggtgatgcttggttccagggtggttacctgaaatacgggaacaataaattgacacctaataccaactcaaattatcgtaaaactgacaacgcgtttgaatttttgttagcaaatgatatcgataattcgaatccggtcgttcaagctgaaaatcttaattggttagaatatctgatgaattttggtactataactggtaaggatgacgatgcaaactttgatagtattcgtgttgatgctgttgattttattagtaatgatacaattcaacgaacatatgattatttacgtgatgcctatcaagtagatcagagtgaagccaaggctaatcaacatatttcattagtagaggctggattagatgcaggaacatcaacagttaaaaatgatgcgcttattgaatctaatttgcgtgaagcggctacgttatctttggccaatgcatctggtaaaaatagtgcgttaaccaatatgttgcaagatgttgatggtggaacattgattgcagatcatacccataattcaaccgaaaatgaagccacaccaaattattcaattattcatgctcatgacaaaggtattcaagagaaagtgggggctgcaatttccgatgctactggggccgactggactaattttacagatacacaattaaaatctggtttggatctttattataaggatcaacgtgctacggataagaaatataatatttataacttgccaagtatttatgcattaatgctcaccaataaagacaccgtaccacgtgtttattatggtgatatgtatcaagataatggtcagtatatggcagagaaaagtatctattataatgctttagaatcattaatgtcagcacgtaaaagctatgtaagtggtggacaaactatggatgttgatagccacggtttgctaaaaagtgttcgttttggtaaaggggctatgactgctgacacggtaggtaatgaagaaacaagaactgaaggtatcggtgtgttagttggtaacgatgcttcattgaaactcaatgattcagatacagtgaccttagatatgggcgcagcacacaaaaatcaaaagtatcgtgcagcaattttgactactaataatggtctatcaacgttcgattctgataaagatgcaccgattgcttggactaatgataaggggatactaacattttcaaataaaaatgttagtggacaagataatactaatgtccatggtgttgctaatccacaggtatctggttatttggcagtatgggttccagttggtgctaaagatgatcaaaatgctgggacaagcgcatctacagtagtcaacacagatggtaaagtattacactctaatgcatcattagattccaacttaatttttgaaggattctctaacttccaacctagagcgacaacaaatgacgaattaaccaatgtcgttatagctaaaaatgccgatttattccagaaatggggtattactagctttgaaatggcaccgcaatatcgctcaagtcaggaccacacatttttagattcaaccattgataacggttatgccttcacagatcgttatgacttaggatttaacacaccaacgaaatatggaacagatagtgatttgcgattggcaatcaaatcattacataaagctggcatgcaagtaatggctgatgttgttgataatcaagtctataacttaccagaccaagaagttgtttctgcttcacgcgcaggtgtatatggtaatgatgtcgcgaccggatttgatacacaattgtatgctgttaattctgttggcggcggtaaatatcaagcacagtatggtggacagtatttgagtgagttaaagaataagtatccagatttgtttgaagctaaagcttatgattattggacaaaaaattatgctaatgatggatcaaacccgtactacacattatcacaacagactcgagatgatataccatcagacgagaaaattaagcaatggtcagcgaaatatatgaacgggaccaatgttttgggacatggtatgggttacgtacttaaggattggaatacgggtcaatattttaagattaataaagatggcgattccaacttaccagtttaa

SEQ ID NO: 17 - DNA, 5016 bp, Fructobacillus tropaeoli
atgagaaagaaattgtataagtcagggaaaatgtgggttgccgcttcagttgccatctccttttccgcgttatctattagcgtggggaataatggtgctaaagcagatgattcacaacaatcatcaactcagattcagtcaacgcaagtaacaactgcgttgccagctggtggacaatattcaactacaaatggtgggcaaagctggaattatttagtcaatggtgttgcaattaaagggatgtaccaagatggccaaggtcagctgcgctattttaatttcattgatggtactcaagttaaaggtgaatttttaagtattaatggtacttattattattttgatcaaaatagtggcgagggacatttggttccaactcaaagtaacggccattatacggaaattggcaatactggtgcttggggctatcagaatagtaatggggaacttgttaagggaattcaaaatatcgatggtcaacttaggtattttgatgagaatactggtaaccaagttaaaggtggctcggctactattggtaataagagttattattttgaaccaagtcaaggaacacttacaacaacaattgatcaagtatccgatgctcaaaatgctaatattcgaggattggcaaccgttaatggtcagttaaattactttgatcctacaactggtgaacaagctaagcataagcaagtggctacaaatggtgcaacgtattatttcaatgatagtggtgttggaacatatttgttcaccaatgtacaaaatacaccggctaatgatgtttcacaacacaatgctgtaaatagtactgatactaaggattatacgaatactgttgatggcttcttaacggctgatacttggtatcgaccaaagtatattttggataatggtgaaaattggcgcgcttcaaacgaaggggagtatcgccctttcattatgaattggtggcctaataaaaacgttgaagttaattatctgaaattaatgcaaaataataatttgctatcaagtacggttcaatatgatcttttcacagatcaggctattttgaatcaagccgcttatcaggctcaaattgcaattgaaaagcgaattaagtcagagggtagcacagattggttaaatacgctgttatttggtggtgatgatagccatccttcatttgttaagcaacaatttatttggaattctgattctgaatctccatggcagggtgacgcttggttccagggtgggtatttgaaatacgggaatagtgttatgacgcctacaagtaattcaaattaccgccaggcaggaaatgcttttgatttcttgttagctaatgatgttgataatcaaaatccaattgtgcaggctgaggatttgaattggctatattatttgatgaattttggttctattacgactaatggtttagataatgattccaattttgatagtattcgattagatgctgttgattttattcataatgacgctattcaaagaacatacgattatttgagacaggcattcaatttaacgaaaaatgaagctactgcaaatcaacatttatcattagtggaagcaggggttgatgctggaacaaccacttataatagcgatggcttaattgaatcaaatattcgtccgttagcaactgattctttaactaacgctccaggtaaaaatgcatcactgtcaaacttaataaaggatgtcgatagtggtgaagtgattgcggatcatgctaatttttctactgatgatggtattccaaattattctattattcatgcacatgataaaggaattcaggaaaacgttggtgcagcgattactgctgcaacaggggctgattggactaattttactaccgaacaattagaacaaggccttgatttatattatcaagatcaacggtcaaccaacaaaaagtataatatttataatttaccaagtatatatgctttaatgctgacaaataagggtactgttccaagagtatattatggagatatgtatcaagataatggtcagtatatgcaacaaaaaagcctatattatgatgccattagttcactaatgactgctagaaagcaatacgtcgctggtggtcaaacaatgagcgttgatgaaaatgggttattaaagagtgtacgttttggaaaaaacgcaatgactgctcaagatacaggtgatgctgaaacaagaacagaaggtgttggtgtcattattggtaatgatccatcagtgaaggttgcggatggtcaaacagttaccttggatatgggtgctgctcataaaaaccaagcttatcgtccattaatcttgacgacaagcgatggcattcaaacttacgatagtgatgaaaatgcaccagttgtatatacagatgacaatggaatcttgactttttcaaatcaagatattaatggtcaagctaacacaaaaattgttggaactttgaatccacaggtttcgggttaccttgctgtttgggttccggttggtgccagtgctgatcaagatgctagaacagcaccatctactcaaagtactaatgatgggaaagtattgcatacgggagctgcgttggattcaaaccttatttttgagggattttctaatttccaaccaatgccaactacacatgatgagatgacaaatgttgtgattagtcaaaatgctagtcaattcgctaaatggggtattactagttttgaaatggcaccgcagtatcgctcatcagaggatcatagtttcttagattcaacaattgataatggatatgctttttcagatcgctatgatttgggatttggaacgcctactaaatatggtactgatgaagatttaaggaacgcaatcaaggctcttcatcaaaatggcatgcaggtgatggctgatgtcgtaatgaatcagttatattccttaaacggaaaggaagttgtttcagctagtcgtgcgggtgtttacggaaatgatgtagatttgccttttggaacacagctatacgtggtcaatactaccggtggtggtgagtatcagaagaaatatggtggtgctttcttaaacattattaaagaaaaatatccaactttatttgattcagagtcttacgattattatttgaaaaattattctgataatggccacggaccagcatatatgacaacagctacagcaactcgagaggcgattccatctgatcagccgcttaaagaatggtcggctaaatatatgaatggtacgaacattttaggacttggtatgggatatgttcttaaagattggaataatggtgcctatttcaaattatcaggaactgatacaacgcttccacaatcattggttgccttgactgggtggaatcaaaacgatgatggcacttggtcatattacagcactgacactgatgatcgagtaacagggaaacaagtgattgatggaagaaccctacttttcgataatcaaggaaaccagattaagggtggttggggtgaaaaccctgatggtacatggtcgtattacaatgctgacactggtgatcgagtaataggtgagcaagtaattgatggaagaactctattttttgataatcagggagttcaagttaaaggcggttggggtgaaaactatgatggtacatggtcatattacaacgctgataccggtgatcgagtaacgggaaagcaagtaattgatggaagaacattattgtttgataatcggggagttcaagtgaaaggcggttggggtgaaaactctgatggtacatggtcatattacaacgctgacaccggtgaccgagtaacaggcaatcaattgattgggggaagaaatttacttttcgataatcaaggaaatcaaatcaagggcggttgggatgaaaaccctgatggaacttggtcatattacaatgccgatactggtgatcgagtaaccggggtgcaagtgattgatggaaagcagttgctattcgatagtaatggtattcaggttaaaaattcatggcagaaaaatgccaatggaacttggtcatattatgatgctaatgacggacatttagtccctgcaaatagctcaaatgatggaacttcatcatctactcaagatagtgggaataagagcaatcaaaatccttcaagtagtagcaatgctgtaaataagactactggttggattaagaatagtgatggaacctggtcttatctatctgcaaaaagtggtcaaaaggtcactggaagtcaaactatcgatggcaagcaattgttgtttgatgaccatggcgtccaaattaaaggtggctggggtaaaaatgctgatggtacatggtcatattatgatgcgaactcaggggaactgacttcaactagtgatatgagtaatgtaaatccacagcaaacaacaactactacgaatgaacagagtacaaccaatcagccaacagatatcacaaaaaatagtgatggtgtttatgtatataagaatgattccaataagaaggcgcaaggctacttgaatgatggatcatcatggaagtggtttaatgatggtcaactttacaccggtttccaaaattacatgggtgcttactattactttattaatggtattcgtcaacaaaaccagtgggaaaatatctggggattgaagtattatgttggtgatgatggtcgaacagttgaaggaattcatgctatcgacggtcatgcttatgactttggtaccgatgggactttcaatgtgaagggatcggctagtggctacttgaatgatggcaagagctggatgtggtacgaaggtggtaacccatatactggtttccgctactacatggatacttactattggttcgaaaatggtgtgcgtcaagataatgcttggcatcaagcttggggtctgacatactacacaggtgcagacggtcgagcagttcagggtgttcaaaacatcaatggtaagctttactacttcggtaatgacggcaccttctttatgcggacaaaccaagaagta

SEQ ID NO: 18 - DNA, 4899 bp, Lactobacillus kunkeei
atgaataataataatagtgaacaaaaacttcgttttaaaatgtataaatcgggaaagcattgggttgttgcaggtttaacaacagctgttgtatcagttgcaatatacagtggctcttcaatcattaatggtggagtaactgtaaaggcagatgtgcaaagcactacacaagcaactacatcagtttctgataattcaaaagattcatcaaatagtattagtaataataattcaaatgatgacaatcaaattgcaacacttcctcaagatggtacatattcaactggagataacggtcaaacttggaagtatgttgaacaaaataaaaacatacagggactttataaagatagtgacaaccaactaagatactttaatgaatatgatggaactcaagcaaagggtgatatcgtaaatgttaataataataactattattttgatagtggtagtggtcaaggacataagatagataactactcaggtggaaattatgttgaatctaacgtcaataatgaaaatggttggatttataaagctactgacaatactgaagtaaaagggattgccactatcgatggtaatgttcaatattttgatcaatcaactggacttcaactaaagggtggagcggttcaagtaggaggagccgactactattttgatccaaacaagggaaacttagttggtaaagttgatcaagttgtaaattcaaacaattatagtgataataaattactagatagtaataaaaatgtagtaaaaggattaacagttaataatggaacattacaatactatgatccttctactggtgatcaagttaaaaataaacaagtgattgctaatggcgtcacatattattttgatgcaagtggtaacggaacatacttgttcacaaatacaggcaatagtgccgttaatgatttctcacaacgtaacgctgcaaatagtgtaaatccaagtgattacaaaaatgtagtagatggatttttcaccgcagatacttggtatcgaccaaaacaaattatcgataacggtacaacatggagaaattccaatagtaatgacttacgtccaatgattaccgcttggtggccaaataaggatgttcaagttaattatttgaaattgatgcaagacaatggacttttagataaaagtgatacttatacattgcaatcagatcaacaagttttaaatcaagccgcccagagcgctcaagtaaatattgaaaagaaaatatcacagacaggaagtacagattggttaaacgatttattgtttgcaagtcatggcaataatccttcatttgtaaaacaacaatatgtatggaattctgactctgaatctccatggcaaggtgatgcttggttccaaggaggatacttaaaatatgggaatagtgttatgacaccaaacactaattctaattacagagattcaaataatttatttgatttcttgctagcaaacgatgtagataattcaaatccagcagttcaagctgaggacttaaattggctatattacttaactaattttgggacaattactgctaatgattcaaatgctaattttgatagtattagaatcgatgctgttgattttattagtaacgatatcatacaaagaagttatgattaccttcgccaaaagtttaatttaacacaaagtgatgctaatgctgattcacatatttcattagttgaaggtggagtagatgcaggaaccacttcttacagtaatgatggattagttgaagcgccatttagactaggtgcctatccattgctacataagcaaggtggagacgtatttaaagatttaataaacgaagaagattctggaatcgatatttcaaatcataacggtgaaactaatacaactaacactattggtggattaactttatctggtggaaaacctaactactcaattgttcatgcacatgataaagatgttcaggaaaaagttgggcaagccattgttgataccacaggtattaaggattggactgattttactccaagtcagttagcacaaggtctagaaacattctataacgatcaaagacaaacagacaagaaatacaatgattataacgttcctagtgcatacgcaattatgttaactaataagggaacggttcctcgtatttactatggtgatatgtaccaagatgatggtcaattcatgcaaaagaagagtctttactatgatgatatagcaaacttgatgactgcaagaaagaaatatgtatctggtggtcaatatatggttgataacgatggaattctaactagtgtacgttttggtaagggcgcaaatacagtcaatgattctggtacatcagatactagaaaccaagggattggattaatagttggatcagatcctaaaaaggtattaaacgatggggataccattgttttacacatgggtgctgcacataaaaatcaaaagtatcgtgcattaatgctaacaactgaaaacggagttcaaaattatagttcagatgataacgctccagttgctgaaactgatgataacggtgatttagttttcagtaacaaagatattaatggacaagataatactgcaattaaacaagtcgctaatccagaagtaaatggttatttagctgcctgggttccatttggcgcttctgatgatcaagatgctagaacatcaccatcaactagccaaaataacgatggtaatgttttacatgaaaatgatgcattggactcaaatcttatttttgaaggattttcaaacttccaacctactccaacaaatcatgatgaatatgcaaatgtagtaattgcaaaaaatgcatcattatttaaagattggggtgtaacaagttttgaaatggcacctcaatatagatcaagccaagatcatactttcgttgactcaactatagataatggttacgctttttctgatagatacgatttaggattcgggacaccaactaaatatggaacagatgaagatctaagaaatgccattaaatcacttcatgcaaatggaatgcaagtaatggccgatgttgtttataatcaactatataacttaccaggagaagaagttgtttcggcaacaagagctggagtaactggaaatgataatgcacttccttttggaacacaactatatgttgttaatacagttggtggtggagactatcaaaagaaatacggaggggcattcttaaaccaattacaagaacaatacccttcattattccaatctcaaaaatacaagtattactacaagaattatgctaataatggtgctggaccaggttatttaactgtaactgatggagaacgttctgcaattccttctgatcaaccaattactgcatggtcagctaagtatatgaatggtaccaatattcttggtcgtggtatgggatatgttctaaaagactggaacactggcgcttacttcaagataagtggtgatgactctactcttcctacgagcttaacttatagaagcggatgggtagaaaatccagacagcacttggtcatactattcaaaggatagcattgccaaattaactggagcacaaattgttaatgatcaaagagtattctttgataacaacggtattcaggttaaaggtggatgggtagaaaatccagatggaacttattcatactatgacaaaaatagcggtgaacttttggtaggttctcaactagtagacggaagacatgtattctttgataatgttggagtgcaagttaaaggtggatgggtagctaacactgatggtagttattcatactacaatgctaatgatggtaccatgttaacgggtgctcaatttatcgatggacaaaatgtatactttgatgctgatggtaaacaggttaagggtaactgggtgcaaaataacgatggttcttgggcatattatgatgctaatttaggtcatcttgtaaaagatgctaagcatgttgattcacaaccaagcactcaacaagttaataataaacaatccgaggaaaaatcaaattcaccattagttgaagctcaaaacaataaagattcagcttcagtagaatctcaaaatcatcaaaattcagtgtcagtagaatctaagaatgaaaacaaaaatcaatcaaacgatgtaagaaatccttccgaaaaaacagacaccaaaacatctaatgaaaaatcaaaagaagtatccaaagaagatgctgcatatgacaatgccaaaaaatcattagtagaagctaaaaagttggtagataagaagccaaataaaactaatattaataaatataaaaaggcattgaagtcttatgaaaatgcacaaaagaagatgaataagtctgtgatttcatcatataaaaaggctgcaaaagaactaaacgctgctaagaaaaacctttctaagaaaaataataaggttaatatgaagaaatatagtattgctttaaacaaatatcgtaatgctaagaaatcttacgtggtaattaagaaaaaagatttagataaatctaaatctgcgttaaatactgctaaaaaagcacttgctaaaaagaagacaaagcaaagtcaaaagaagtataacgatgcattgaaaaaatattacgatgcagaaaaaacttatctaaacttgactggtaattacactaaaaaatattattatgatttcgataaagtagggaaaaaggttaaagttatcaaatcaacttccgtatataattcattgaaaccaaatagtaaaaaagtagtaaagaagattaaaaaaggatcagtaattaaagtgaagaaacttattttgtcaaataagaagtcatactttgatttaggatataaccgttttgtaatcgcaagtaaatcttctataaaaaaagctaagtaa

SEQ ID NO: 19 - DNA, 3957 bp, Lactobacillus kunkeei
atgaaatcaaaagataacaattcaaaaatacatttcaaaatgtataaatctggaaaacaatgggttattgctggattaactacagcggttgctgctgtttctatttatggtggaacaactatatttaatgacagcgtggtagctaaggctgatacagcagttaaatcttcacaaagttccaacgctgatactactcaatcttcatctgctgttgttgattctagctctgcaaattcaagcagtccatcatcgactgaagtatcagtaaacgtaaaaaatacatcaaatgcagatacacaaggtattcaagcattaccagatggtggtaactacacatcagaagataatggtcaaacttggaaatactcatatcaaaacaatgatgttaaaggtctatatcaagaaaacaataacattcgttattttagtgaaaatgatggatcacaagtaaaaggaaacatcttaaatgtaaataacaaaaactattattttgatagtaataatggtgatggccatttaattaaagactattctggtggaaactatgttgaacaaagtcaagataaatggacttataagacatctgataataaccttgttaaaggtatcgcaactattgatggacaaattaaatattacgatcctactacaggtatccaattaaaaggtggagcttttgagattggtggggctgcttattacgttgaccccgctcaaggaaacgttgtcggaagagtaaattcaattattaactctggaaattatgtcaataagaacaacaatactacttttgttgatgataataacaatacagttaagggattgaatgtagtaaggggtaacttacaatactttaactcaacaacaggatatcaagctaagagtgaacaagttgttgctaacggagccacatattactttgataaagatggtaacggaactttcttatttaataacacaggttcattttcagtaactgattttgcaaaacacaacgttgctaacagtaatcaaccatctgattttaccaatactgtagatggtttcttgacagctgaaacatggtatcgtccaaaacaaattttagataatggtactaagtggcgcaactcaaataaagatgatcttagacctcttattacagtttggtggcctaacaaagacgtacaggttaattacttgaaactaatgcaagataatggactattggataatagtgttaaatatactgtattttctgaccaacaaactttaaatgaagcagctcaatcagctcaagttaatatcgaaaagagaatcactcaacaaaaagcatcatcatggttatatgatttattattcaagggagattcatctcatccatcatttatgaaccaacaatatatttggaatatgggttcagaatcacaatggcaaggggatgcttggttccaaggaggatacctaaaatatggtaatagtcctttaaccccaacaaccaactcaaaatatagaaaaacagataatcaatttgatttccttttggccaatgatgttgataattctaatccagcagttcaagctgaagatattaattggttatattacttaactcatttcggaacaattaccggtaaaaatgataaagccaattttgatagcattagattggatgcagtcgattttgtaagtaacgagattattgaacgaagcaatgattatctaagagatttatataagttaaccaagagtgatgcaaatgctgataagcatatatcacttgttgaagccggtgttgacgctggaactagttcaacaaatggtgattctttggttgaagcaccttttagattatcagcctatggattacttcataattctggtaaagttgatgcattgcaagacttagttaaagaagttgattcaggtgttcttatttccgatcacagtaaaaactctaaggatggtggggttcctaattattccatcgtgcatgctcatgataaagatgttcaagaaagagtaggacaagcaattgttgattccactggcattaaagattggacaaactttacacctgctcagttagctaaaggattaagcgtttactatgctgatcaaagaaagacagttaaaaaatataatgattacaatatgccaagtgcttatgcaattatgttgacaaacaagggtacagttccacgtatttattacggtgatatgtatcaagatgatggtcaatttatgcaaaagaagagcttctactatgatgatattgtcaaattgatgactgctagattgaaatacgttgcaggtggtcaaacaatgagcgttgattctaacggatttttgaagagtgttcgttttggtaaaggcgcaaagacagttaattctaagggaacaaaagaaacaagacacgaaggtattggtttaattgttggaaatgatgctaagaaagttctatcaaatggacaaaaagtaacattgaacatgggtgctgctcataagaaccaaaaatatcgtgcattaatgttaacaactaacaagggagttcaaacatttgcttcagataaaaatgctcctgtagttaagacagatggaaatggtgttttaacatttactaacaaggatattaaaggtcaagctaataccagtgttagaggagttttaaatcctaaggtttctggataccttgctgtatgggtaccagtaggcgctaaagataaccaagatgcccgtactcaaccatctaagaaaaatagaaatgatggtaaagtgcttcattcaaatgatgctttagattctaatttaatttacgaaggattctccaatttccaaccacaaccaaagaaacgcagccaatatgcaaatgttgtaattgccaaaaatgcaaagctattcaaaaaatggggaatcactagttttgaaatggctccacaatatcgttcaagtaatgataaaacttttgttgattcaacaatcaacaacggatatgcattctcagatagatatgacttaggtttcggtaagccaaccaagtatggtactgataaggacttaagaaaggctattgaatcactgcatgatcaaggcatgcaagttatggctgatgctgtattaaatcaactatacaacttacctggaaaacaagttgtttcagcacaaagagctggagtaacaggtaacatagctgatttgccatttggaaagcaattatacgttgttaatacaattggtggcggtaagtatcaaaagaaatatggtggaaaattcttaaaggctttaaaagctaaatatccaaacatatttaagggtaagacttataaatataactacaagaattattctccaactggtgaaggatatttaacacttaatacaggtaagacggtttcaattccatccaaccagcctattactgaatggtcagctaaatacatgaatggtactaatatccttggtagaggtatgggttatgtattgaaggattggaatacaggaacatactttaagttgaacggactaaagacagttcttccttctgaactaacagataagagtaactgggttaatgaagtttctacatcttcaaaagatgtatataataagtctgtttcaaatttaaaagacgctaaaaagaaattagctgcaaagaaatcaaaagaaaacacacaactatataacaatgctctaaattcttattacaaagcagaaaaagaatacttgagcagtgctaaactttacaataaaaagtactactatgattttgataaattaccttcaaaagttaaagtagctaaggtcacttactcatataaatcaactgatttcagcaaagataataggattaaaaagcttaaaaaaggaactgttttaaatgttaagggattagttcttaacggaaaagttacaagaattaatattggtaacggtaagtttgtaactgcatctaaagatttcataaaagcaattagatag

SEQ ID NO: 20 - DNA, 3420 bp, Lactobacillus kunkeei
atgaaagcagaacataataatttaaaattacatttcaaaatgtataaatctggaaaacaatgggttattgcgggactaacaactgtggtagcttcaattgctatcttcagtggaaaccaactatttagtgggaatgttgtagcaaaggcagacggggtaacaacaacccaagtttctcaaaatagcaatagtagtaatggaatttctacacttccaaaagatggaaagtatgtatctagtgataatggaaaaacatggaagtatgtttctcaaaacaatgctgcaaaaggattatatagtgatggttcaaacattttctactttaatgaaagtgatggaactcaagtaaaaggtaacattattagtgttggaaaaaacacttattatttcgatagcaaaactggtcaaggaacaaaaatatcagattatactggtggaaagtacactaacccaagtactgataataaagctgcttggacctaccaagataagagcaataacactgtaaagggtgttgcaacaattggagattcagttcaatattacgatgaaaaagatggatttcagctaaaaggtggatctattaacttaggaaacacaaattattatgtagattcaaaccaaggaaatgtaactagtaaagtaaatagagttgtttcttctaatgacgggactttaaaaggattaaacgtcgtaaatggtaatttacagtaccttgattataaaactggaaaacaagtaaagaataaacaagtagcagttaatggtgttacatactactttgatgataatggaaatggttcatatttatttaccaatttaggtaaatctgttcgtactaattttgataaatataatgctgttaatggtgtaaataaatctaatttcacaaacacagttgatggattcttaacagcagattcatggtatcgtcctaaacaagttttggctaacggtaagaaatggcgtaagtctacttctaaagattttagaccattagtaacagtagcatggccaaacaaagatgttcaggttaattatttagctttaatgcaaatgaacggtttgttatctaataaggaaaagtacactgttttctctgatcaacaaacattaaatgctgctgctcaaaaagcccaagttaatattgagaaacgcattagtaaaaagaaaagtactaaatggttagacaagttgttattccaaggtacaactactgaaccatcatttataaagagacaatatgtttggagttctgcatctgaatatcctggacaaggggatgctcaatggttccaaggaggatacttgaagtatggtaataatcgtttaactccaaaaactaattcaaagtatcgtcaaattggtaatgcttttgactttttattagcaaatgatgttgataactctaacccatcagttcaagctgaagatattaattggctacattatttaactcactttggttcaataactgctaaagatcctaaagctaatttcgatagtatcagaattgatgctgtggactttatcagtaatgatatagttcaaagaagtaatgattacctaagggatttatacaaacttacaaagaatgatagcaatgctgataagcatatttcattggttgaaggtagtctagaagcggcaacaagttattcacattcagattctctaattgaatctccttatagaaatgatattgatggactattaggaaactcaggaaattctgcagacttaagtaaattaattaaagagtatgattctggaatcattatttcagatcattcaggaactactaacaatagttctattccaacttattctattgttcatgcccatgataagggagttcaagaaagagttggacaagcaattatggataattctggtataactgattgggcaaactttactcctaagcaattaagagatggattgaagttatactatgatgatcaaagaaaaactgttaagaaatacaatgactataacgttccaagtgcctatgcaataatgctaactaacaacaacactgttcctcgtatctactatggtgatatgtatcaagatgatggacaattcatgcaaaaaaagagtctatattatgatgacatcgttagtttgatgctggctagaaccaaatatgttgccggtggtcaaagtatgagcatggattcaaatggattcctaacaagtgttcgttatggaaaaggtgctaataatgttaattcacaaggtacatctgaaactagaaatgaaggaattggagtaattgttggtaacgacactaataaagttcttaatgatggacaaacagttactttaaatatgggtgcagctcataagaaccaacaatatcgtcctgttttattaacaaccaaagatggaatcaagacatattcttctgataaaaatgcgcctgttgtagaaactgattcaaatggggttcttacatttagcaataaagatgttaatggacaaagtgacacaagtgtaaggggaacattaaatccacaagtttccggatatttagctgtatgggtacctgttggtgctaagaatggacaagatgctagaacaaaaccatcaaagaaagccagaaatgatggtaaagtacttcatttaaatgatgctttagcttctaacttgatttttgaaggattctcaaactttcaacctatgccaaaaaataagagtcaatacactaacgttgtaattgccaaaaatgctaaaacatttaaaaaatggggtattacaagttttgaaatggcacctcaatatcgttctaccaacgataagagttttgtcgattcaactataaaaaacgggtatgcattctcagacagatatgatttaggtttcggtaagccaaccaaatacggtacagataaagatttaagaaaggccattaagtccctacatgctcaaggcatgcaagttatggctgatgttgtatataatcaactatataaccttcctggtaaagaagtagtatctacttctcgagctagtgcttatggtaataatgttgatgttccatttggaaaccaattatatgttgtaaatactattggtggtggaaagtatcaaactaagtttggtggaaaataccttaaagaactaaagaagaaatatcctagtttatttaaggcaaaaacatataaatactattacaaagacaatcaaaaagatggctcagttaaattagctcttacttcaagcaagagatcaagcattccagcaaacaaacctattaaggaatggtctgctaaatatatgaacggtacaaatgtattgggattaggaatgggatatgtcttaaaagattggaataatggtaaatactttaagattaatgggacaaagacttcgttaccaagttctatttattacaaaagtacaaaaaataagtaa

SEQ ID NO: 21 - DNA, 4392 bp, Lactobacillus kunkeei
atgaatatcaatagtaatgaacgtaaggttcgatttaaaatgtataaatctggtaaacaatggattgtagctggattaactacagcagtaatatctattgctgtgtatggtggttcttcaattgccaatggtggaattgaagctaaagctgatgcacaaaacgcagctacttcttcaattgtgaatactaataattctacaaatagtagtaatgctaattcaattgcatctcttcctcaaaatggtacatattcaacaaatgataacggacaaacttggaagtatgtatcacaaaataaggacattcaaggtttatataaggataataatgatcagttaagatattttaacgaatatgatggcactcaagccaagggtgatattgtaaatgttaataatgacaattactattttgataaagacagtggtcagggacataagattgatagctacactgggggaagctactctgaaagtaaggtcaataaccaggatggttggatttataaatcaagtgataacaatgatgttaaaggagtcgctactgtcgacggtaatattcaatattttgatcaaaatacaggtctgcaattaaaaggtggatctgcgcaaattggtggagttgattactattttgacccaaacaagggtaatttagttggaaaagttgatcaagtagtaaactcaaatgattatagcgataataagttactggatagcaacaaaaatgtagttaaaggtttagtagtaaataatggtcagttacaattttttgatacatctaacggtaatcaggctaagaataagcaagtaatagctaatggaattacctactattttgatactaatggaaatggtcaatacttgtttactaatacaggtaagagtgctgttgatgactttacacaaagaaatgctgctaacagtgttaacccaagtgattacaaaaatgttgtagatggattttttacagcagatacttggtaccgtccaaaacaaatattagataatggtactacttggcgtaattcaaatagtaatgaactccgtcctatgattactgcttggtggccaaacaaggatgttcaagttaattatttgaaattaatgcaaaataacggactattagataaaagcaattcgtattcaatacaatctgatcaacagacattaaatcaagcagcacagaaagctcaagtaaatattgaaaagaaaatttcacaaacggggaatactgattggttaaatgatttgttatttaaaggaaacggcgataacccatcatttgtgaagcaacagtatatttggagttcagattcagaatcgccatggcaaggagatgcatggttccaaggtggatatttaaaatatggcaatagtgtcatgacaccaaatactaattctaattatagagattctaataacttgtttgatttcttgttagctaatgatgtagataattcaaaccctgcagttcaagcggaggacttaaattggctatactacttaactaacttcggaactattaccgctaatgattctaatgctaattttgatagtattagaattgatgccgttgattttattagtaacgatattatacaaagaagttatgattacttacgtcaaaagtttaatttaatgcaaagtgatgcaaatgctgattcgcatatttcgttagttgaaggtggagtggatgcaggaactacatcttatagcaatgacggattagttgaggcaccattcagactggatgcttatcctttgctacataagcaagatggagacgtatttaaaaacttaatagatgaagaagattctggaatcgacatttcaaatcataatggagaaaccaatacaaataatactattggtggaataactctatctggtggaaaacctaactattcaattgttcatgcccatgataaggatgttcaagaaaaagtaggtcaagctataatcgatacaactggaattaaggattggactgactttacaccaagtcaattagcacaaggattagaaactttctataacgatcaaagacaaacagtaaaaaaatacaatgattataatgtgcctagtgcatatgcaatcatgctaactaacaagggaacagttcctcgtatttattatggtgatatgtaccaagatgacggtcaatttatgcaaaagaagagtctttattatgatgatatagcaaacttgatgactgcgagaaagaaatatgtatctggtggtcaatctatggttgataataatggaattctaacaagcgtacgttttggtaaaggtgccaatacagttagtgattcaggaacagaagatacaaggaatcaaggtattggattaatagttggatctgaccccaaaaaggttttaaatgatggggataccgttgttttacacatgggtgcagcccataagaaccaaaaatatcgtgccttgatgctaactactgaaaatggaattcaaaattataattcagatgataatgcaccagttgctgaaacagatgataatggtgatttagttttcagtaacaaagatattaatggtcaagctaacactgcaattaaacaagttgccaatccagaggtgaatggttatctagcagcatgggttccggttggggcttccgatgaccaagattcaagaacagcaccatccactagtcaaaataatgatggtaatgttttgcacgaaaacgacgcactagattcaaatcttatttttgaaggattttctaacttccaaccaactccaacaaatcatgatgaatatgcaaacgttgtaattgctaagaatgcgtcactatttaaggattggggtgtaacaagtttcgaaatggcaccacaatacagatctagtcaagatcatacattcgttgattctacaatcgataacggttacgccttttcagatagatatgacttgggatttggtacaccaactaaatatggaacagatgaagacttaagaaatgcaataaaatctcttcatgataatggtatgcaagtaatggctgatgtagtatacaaccaattatataatttgccaggacaagaagttgtatctgcaaccagagcaggtgttactggtaatacaaatgcattaccttttggtactcaattgtatgtagttaatacaatcggtggtggagattatcaaaagaaatatggtggagcattcttaaatgaactgcaagaacaatatccatcattattcaaatctcaaaagtacaagtattactacaaaaattatgctaataatggtgctggaccaggttatttaacagttaatgatgcagaacgttcggatattccatataatcaaccaatcactgaatggtcagctaagtatatgaatggaactaatattcttggacgtggtatgggttatgtattaaaggactggaatacaggtgattatttcaagttaagcgggagcgattcaacactaccaagtagtttaacttacaagagcggttgggttgaaaatcctgatagtacttggtcatactatgaaaagaataatattgacaaattaactggatctcaagttattaatgaggaaagagttttctttgataacaacggtattcaagttaaaggaggatgggtaaaaaattcaaatggtacctattcttactatgacaagaatagtggaaacatcctaactggtgatcaattaatcgacggtgaacatttcttctttgataacaatggtgttcaagtaaaaggaaaatggataaagaatagtgatgggtctaagtcatattacgattctcacttaggaaaacttataaagacggataaaaaagtatcttctaatgctcgaaaaaagaaatctaaggaagaattattgtatgagaatgccttaaaagttttaagaaaagataagaaacgtctcgataaaaataagacaaaggcaaatatcagaaaatataataaatctctaaaaaaatatcgtaaagcaaagaagaaacttttagcgattactaagaatagagttgctaatgctagaaaagcgattaaaattgctaaaaaagttctttctaagagaaaaaatattaataatgaaaaaagatattataaagctctaaaagaatattatgtagcggaaaaatcatatttgaaaattactggaaattacaataagaagtattattacgaatttgataaacttactccaaaagtcaaagtggttaagaacatttattcctataagagtagacattttactaaaaagaatagagttaaaaagattaaaaaaggtactcttgttagagttaaaagtatagttcgaagtggtaaagtcgctcgaattaatatcggaaatggtcattttataacttcatctaaagattttattaagatgtttaaataa

SEQ ID NO: 22 - DNA, 8526 bp, Leuconostoc mesenteroides
atgagagacaaaagaataatatgcgatcgtaaaaaattgtataaatctgggaaactgttagtgacagccggtattttttctgctgtgatatttggcgtttccacaactaacgtaagcgctgatagcactaacaacactggtgttacggtgtcacaagcaccagataaagtagcggacacaacagctacaacagataaagtagcagacacgacggctacaacggataaagcagcggacacaacagctacaacagataaagtggccgacacagcagctgcaacggacaaagtagcggacacaacagctacaacggacaaagtagcggacacaacagctacaacagataaagtggccgacacagcagctgcaacggacaaagtagcggacacaacagctacaacagataaagtagcggacacaacagctacaacggacaaagtagcggacacaacagctacaacagataaagtagcggacacagcagctgcaacggataaagcagcggacacgacggctacaacagataaagcagcggacacgacggctacaacagataaagtggccgacacagcagctacaacagataaagcagcggacacgacggctacaacagataaagtggccgacacagcagctacaacagataaagcagccgatacagcggctacaacggataaagtaaccgacacaacagttgcaacgaataaagcagtggacacaacagctacaacagataaagtggacgacacaacagccacaacgtcagaaaaatcaaaaagtattaaacaaattgatggtaaaacttatttcattggtgatgatggtcagcctaagaaaaattttacagccattgttgacggtcaagtattatatttcgacaaagatactggtgctttgacatcaaatagtagtcaatataccgatggtttagtcaatataggaaatgagcataatgcggcttattcattgtcttcggatagttttacacaagttgatggctatctaacggctaacagttggtaccgacctaaagatatattaaaaaatggtacaacttggacggctgcaacagcaaacgattttcgaccattgttaatgtcttggtggccagataaagatacccaagtttcatacttaaaatatatgcaatctgcgggattattatcagatgacgttgcattatcaaacaatgatagtatgaacagtttgacggatacggctatgactgttcaaaaaaacattgaagaaaaaattggcctattgggcagtactgactggcttaaggccgatatgaaccaaatggttgattcacaatcgaattggaacattagtagtgagtctaaaggaacagatcatttgcaaggtggtgcgctcctatacgttaatagtgatttaacaccaaatgccaattctgattatcgtttattaaatcgaacgccaactaaccaaaaaggtcaaattacaacaaatggtaatcaaggtggctatgagatgctgttggccaacgatgttgataattctaacccaattgttcaagctgaacaattgaattggttatactacatgatgaatatcggtagcatcgcccaaaatgatccaacagcaaattttgacggttacagagttgatgctgttgataacgtgaatgctgacttgttgcaaattgctggagattattttaaagcagcatatggaacaaatcaaagtgacgctaatgcaaacaatcacatttccatcttagaagactgggacaataatgatccagcgtatgtaaaagcacaggggaacaaccaattaaccatggattttccaatgcatttggcattgaagtattcattgaatatgccaagtagtgctcgtagcggtttggaaccagcaatttcaacaagcctagtaaatcgtgcagcagacgccacagaaaatgaagcccaaccgaactattcatttattcgtgcacatgatagtgaagtacaaacggttattgctcaaattattaaagataaaattaatcctagttccgatggattgactgtctcaacagatgaaattgccaaagcattcgaaatatataatgctgacgaattaaaggctgataaagagtataccgcatataatataccctcatcatatgcattgatgttaactaacaaagatacaattcctcgtgtgtattatggtgatttgtttacggatgatggacaatatatgtctgcaaaatcaccatattatgatgcacttacttcattgcttcaatcgcgagtaaaatatgtttcaggtggtcaatctatgaatatgacttaccttcataataatcaaggccttttgacgtcagtccgctatggaaaagacgccatgacagctaacgacactggtacaagtgaaacgcgcacacaaggtattggattaattgtcggcaacaaaactgatttaaacctgaataatgatgagcaaattgtgcttaacatgggcgccgcacacaaaaatcaagcttaccgtgcattaatgttaagtactaaagatggcttgaaaatttataatagtgatgacgaggcaccggtatcgtatacagatgatcaaggccgtttgatttttaaatctgatgtggtttatggtgtgagtgatgctcaggtttctggttatttagcagcttgggtgccagtcggtgcaaacgatagccaagatgctagaacagaaagtagtacaacagcgtcaacagatggtaatacctatcattcaaatagtgccttagattctcaagttatatatgaaggtttttcaaacttccaagccatgccaacacaggccgatgagtataccaatatcaagattgccgaaaatgcacaattattcaagagccttgggataacaagctttgaattggcacctcaataccgttcaagtacggataacagtttcttagattcagttattcaaaatggctatgccttcacggatcgctacgacattggttataatacgcctacaaagtacggtacagttgaccaactattagatgctttaagagcattgcatgcccaaggcattcaggctatcaatgattgggtcccagaccaaatttataatttgcctggcgaagaaatagtgacagccagtcgaacaaacggttcgggaaaggtgaatgaaagttcagttattaataatacgctatatgattctcgtactgttggtggcggagagtatcaagcaatatatggaggtgctttcttagataagttaaaacaagattatcctgagttatttgaaacaaaacaaatttcaacaggtgaagcaatgaaccctgatgtcaaaatcacagaatggtcagctaagtattttaatggctcaaacattcaaggacgtggtgcatggtatgttctcaaggattggtcaacaaatcaatactttaatgtttcaagtggtagtgaatttttacctaagcaactgttaggcgaaaaaacaagtacagggtttaccaacgtggacaatggcaagactgagttttattctacgagtggctaccaagcaaagaatacatttattcaagataatgacaattggtattattttgataatgatggctatatggttgttggcggtcaagaaattaatggtaaaaaatattatttcctaccaaatggtgtagagttacaagatgcttatttgtctgatgggactagtgagtattactacagtagtgatggtcgtcaaatttctaatcaatattatcaaggatcagacaacaactggcgttatttctttgcagatggtcatatggctgtagggttagcaacaattactacagaaaatggtacaacaaatcaacaatatttcgatgcaaatggtatgcaacttaagggcgtagctataaaggatactgatggcaatgtgcactattttgatggtaagacaggaaacatggttataaattcctggggcaaaataagcgatggttcatggttatacttaaatgatagcggtgtagcggtcacaggaccgcaaaatattaacggtcaaaatctttacttcaacgaagacggtattcaagtaaagggtgaagccattactgataatagtggaaacatacattattatgatcgcagcacaggaaatatggttgtgaactcatggggtgaaacgaataatggttcatggctatacttgaacgacaagggtgatgccgttacaggagaacaagttattgacggtcaaaaactatatttcagtagtaatggaatccaacttaaaaatacattcaagaagctatccgatggttcatggctatatttgaacgataaaggtcttccagtgacaggagcacaggtcattgatggacaaaacttgtatttcgaccaagatgggaagcaagtcaaaggtgacgttgctacagatggacaaggtaacactcattattatgacggcaacacaggaaatatggttactaattcatgggcagagttagcggacggttcatggatgtatctagataatgatggcaatcctttaacaggaccgcaaaagattgatggccagtcactctactttaatgatgctggtaagcaaatcaaaaacgcattggttaaactagatgatgggtcaacaatttacctcgatgataaaggtgtttcatcaaccggtattcaaagaattgatgataagatatattattttgatcctgatggtaaacaagtagtatgtcgttttgaagaattaccagatggttcatggatgtatctagatgatgacggtgttgctgctacgggcgctcaaaaaattaatggccaggaattatatttcgacaataacgggaaacaagtcaaaaatgacaaagtaattaatgacgatggaacaataaactattacacaggtatgagcggtgaaaaactaaaaaatgattttggtgaattaccagacggttcatggatgtacttggataatcaaggtaatgctgtaataggtgcccaaaaaattaatggccagaatctttacttcaagacagacggacgacaggttaagggtgaagcaaatgttgattcatcgggtgaaatgcacttctatgatcctgattctggcgagctaattacaaatagatttgaacaagttgctagtggtgtatgggcttactttgatgccaacggtgttgctgtaactggtgagcaacgcattggtaagcaaaatttattttttgatccaactggttatcaagttaaaggcgacaaacgaacaattgacggcgttctctatacctttgataaagaaagtggtgagagaaagggtttagattctatatcggtattacccaccaatggacaatacacaaccgataaggcccaaaattggtattaccaagtcgatggtgaaaatgtaaaagggctatatacaaataatgatggtcaattacgttacttcgatttgacaactggcgtgcagactaaaggtaattttgtgacaattggcaatgatacctactatttcaccaaggaacaaggggatggacagatagtttctgaggttgtgtcaggacactatggtactgtccagttgagtgacaattcgtctgcatgggtttatcgcggtgcaaatgatcaaattttgaaaggcctacagaatataaacggtcgtctgcaatattttgatctaaccaccggtgcgcaattaaaaggcggtgctgcaaactatgatggcaacctttattattttgaatcatcagatggtaacctagtcagtaaaattcagcaatcttattctactgggaattatgtgaccgatggtgataaagtaacatatgttgatgagcaaaacaaccaagtcacgggattagcgttgattgatgatcaactacaatacttcaatccaagtgacggtagtcaagtcaagaatgagcaggttatcgttgatggcgtcacatactactttgataaaaatggtaatggacaatacttgtttacaaatactgcaacgatgtctactaatgaatttgccaaacatagtgctgcttatagcaatgatagttctagcttcaagaatacgatagatggtttcttgacggccgatacctggtatcgccctaaagatatcttggaaaacggacaaacgtgggtagtttcttcaacaaatgacgtgcgaccactgataacagtttggtggccaaataaagatgttcaagttaattatttaaattttatgaagaaaaatggtttgctagatacaagtagtcaatttaatctacaatttgatcaatatgacttgaatgtcgccgcgcaaaaagttcaagtggctattgaaaaacgcatttcgaaagaaaagagtacagattggttgaaagatcttttgtttgaagctcatgaagatacgccttcatttgtgaaacaacaatttatttggaataaagattctgaatatcaaggtcaaggggatgcgtggttccaaggtggttatctgaaatatgataatagtgaattaaccccaacaacgaactcagattatcgtgaatccggtaatacattagacttcttgcttgctaatgatgtcgacaattctaacccagcggttcaagctgaaaatttgaattggttacattatttaatgaactttggcacgattacagctaatgatgatgatgccaactttgacagtattcgtattgatgccgttgactttattgataatgatgccattcagagaacctacgattacatgcgtgatgcttataaagttgatgcaagtgaagacaacgctaataagcatatttcactagttgaagctggattagatgctggtacctctacaattaagaataatgctttagttgaatctaactttagagaggcagctacactatcgctagcaaatcaatcagggaaaaatagttccttgactaatatgttgcaagacattgatggtggccagattatagctgatcacgccaacaatgcaacagaaaatgaagcaacgccaaattattcaattattcatgctcatgataaggggattcaagaaaaggttggtgcagcaattaccgacgttactggtgcagactggacgaatttcaccgatgaccaattaaaagaaggattagcagcttattatcaagatcaacgttcaacgaataaaaagtataacatctataacttacctagtatctatgctttgatgttgaccaataaggacacagttcctcgtgtttattacggtgatatgtatcaagatgatggccagtatatggaaaagcaaagtatttattatgatgccattgtttccttgatgaacactagaaagagttatgtgagcggtggacaaaccatggatgtagatgaacatggtttgttgaagagcgttcgttttggtaaagacgcaatgacagctagtgaacttggtacgaatgaaacacgcactgaaggtgttggtgtgctggtcggtaatgattcttcactaaaactaaatgattcagatacagttactttagagatgggggcggctcataaaaaccaagagtaccgagctgcattgttgacaactagtgatggtattgttacgtatgatgctgataatgatgcaccaacgatctggacagatgaccggggtacattaacgttctcaaataaggagattgctggtcaagattatactagtgtgcaaggattcgctaatccacaagtatcaggttacttagcagtttgggtgcccgtaggagctagtgacgatcaagatgcccgaacagcagcatcaacagataaaaatactgatgacaaagtactgcattctaatgctgcattagattcgaacttgatttacgaaggtttttcgaactttcaacctaaagcaaccaccaatgatgaactgactaacgtagtaattgctaaaaatgctaatttatttgaaaagtggggaatcacaagttttgagatggcaccacaatatcgttcaagtggggaccacacgttcttagattcaacgattgataatggttatgtatttactgaccgatacgatttgggatttgaaacaccaactaagtacggtactgataaggatttgcgtactgcaattaaagcattgcaccaatcaaatatgcaggttatggctgatgtagttgataaccaagtttataatttatctggacaagaggtcgtatcagcttcacgtgctggtgtttacggcaatgatgtgtcaactggatttgggacacaactctatgcggttaatagtgttggtggtggtaaatatcaagcccaatacggtggtgaatatttgaatgaattgaagcaacaatacccagatttgttcgaagctaagacgtatgactattgggttaaaaattattcaaatgacggatcggatccgtattacacactgtcgcaaaacacacgaaaagatatgccaagtagtgaggtcattaaacaatggtcagctaaatatatgaatggtactaatgtattaggaaacggtatgggatatgttttgaaagattggaatacaggtgagtacttcaaaattggagaaaagaatgctgattttataacaaattaa

SEQ ID NO: 23 - DNA, 7740 bp, Lactobacillus kunkeei
atgaataattatcaagatagaaaattgcattataaaatgtataaaagtggaaaaaactgggttgttgcaggtattgtttcagcaacaatgtctattgtattattccaaaatattaatgatgttacagcaaaagctagtcaaaatcagattacatattcaggtagctatgcttcgacagattccggtagtgctaaaagtgcatattcagcgtcatcttacataaacggatcaagttctttgtctgtacctagcactgataattcaaacaaatcaagcttagcgtcttcaacaaactctagtgttgtgacttcttcattaagttcaaatgttatgaatcaatcatctaattcacatgcgtcatcaataagttcagacgtttcaaatcaatcacaaagttcaaaatcagcatcaacgagttcaaattcgtcagaaaaatctgattcagcatcacagtctaataattctgtgcaatcatatgaatcggtttctttaagtgtatctttagcatccaatgcttcacaaaacttaaaatcgcatacaaagaacattgatggaaagacatatttttatgatttaaataataatgaagttaagtctgctttaattgacgataacaacacatactattattttggacccaatggatatctgactacatttgatgattcaaagttttcggatggctcaatcaactcatcagatcagttatctatttataccccagatggtaaatcaattacaaatgttgatggctttttaacagctgactcatggtatcgtcctaagcaaattcaagtaagcgatactcaatggagaaattctactaatgcagattttcgaccactattgagtgtgtggtggcctaacaagacagttgaaattaattacttaaattatatgagcaaaaatggtctagttaatggtcattttgataataatagtagtgcaaacgatatcaaccaagcagctgcaactgtaagattaagcattgaaaacaaaattaaagcagataatggtgatttaagtgcgattagatctttatttactactttcataaattctcaggatgaatggaatatcgacagtgaagactataattctggagatggtttacaaggtgggtcacttctttttggaaacaatagtgaaactaaagatgccaactcaaactacagattacttaatagaaatccgactcaacaagatggaaaaattgattatacacatacacaagatccaggctttgaatttttgttggctaacgacgttgataattctaatcctgtcgtacaagctgaaacactcaattggttgcattacctaatgaattttgggtcaattgttaacaaagatagttcagcaaattttgatggcgtgcgtgttgatgctgttgataatatggacgccgatgtgctaaatatcattagccaatattttagagatgcatacaaaattaacgccaatgacgttaattctaataatcatctttctattctagaagactggagtggaaatgacccatattaccaaaaagatcatggaacaaatcaaatgactcttgatagtgactatttaagctcattacgatcgattttaatgtacaatccttctgttagatctgatatgtcaactattattaatgctggtattgtggatagagctgatgacaatacaactaacaaagctattccaaattatgaaattgtaagggctcatgatgcaggtgttcaagacatcatttcacaaattattattgacaacattgatccccatgcttcagcttctaatccaacgtgggaacaaatgagagaagctttcaagatatacgatgctgatgaaaatagcactgtaaaaaaatacacacaatataacattcccgcatcatatgcattgacccttacaaataaagatacaaccccaagagtttactatggtgacctatacactgacgacggtcaatttatggaacaaaagactccatattatgatgctattgctgaaatgcttaaatcaagagttaagtatgtagctggtggacaacatatggaagcggttaaggttaataatggtgaagatacgattcttacttctgttagatatgggaaggatgcattaaatgcagatgacttaggtgatagtctaactagaacatctggaatagctgttgttgaaagtaataatcctactttgtcactttcggataaagacaaagttgttattcatatgggggcagcccataagaatcaagaatatcgtcaattattaacggcttcaaattcaggaattgattcttttgacagtgatagttcaaaaggttatgttgtcgttcgtacagatgataatggtgacttaacattagatggaaatatcattaagggatatgctaacccgcaagtatctggatacttatcaatgtgggtaccactaggggcttctgataatcaagacattagaactgctccttcttcagaatcaagtactgatggtcaatccattcattctaatgaagcatctgactcgaacgttatattagaagcattttctaactttcaaaattttccacaaacaactgatcaatatgaaaatgttgttattcaaaaaaatgcagaagattttaaaaatttaggttttacttatttagaattaccaccacaatataagtcaacaaaagatggttcgtttattgattcggttgtacaaaatggttattcatttaatgatagatatgacctaggatttgatacgccaactaagtatggtacggctgaacaattgattgatgcaattaaatctctacatgcacaaggaataaaagtacttgctgatatcgttccagatcagatatattcattgccaaaccaacaaattgtaaacgcaactagaacaaatccttatggagatgcaaactttaattcaaatcttattaatgttttgtatgatgcgtttagtaagggttctggaactgattatcaatataagtatggtggtgagttcttagaacaactaaaaaaattatatcctgacttatttaccacaaaacaaatttcaacaggacaaccaatcgatgcttctaaaaagttaaagatttggactgctgaatatttaaatggttcaaatatccaaggtcgaggttcggggtatgtattaagtagtacaccaaattctaattactacactgttgtagatgatggaaacacaaacataaagagttctaatctacccaaaggattattaggtgataatgttgaatatggtttaaaacttattgatggcaagatgaagtacgtttccaccggtggatttattgctaaaaatacttttattcaagatgataatcacaattggtactatgttgataataacggtgattttgttacttctccacaagttatcaatggaaataagtatttcttcctatcaaacggtgttaatttaagagacttcatttcagttaatagtgatggaacgatgaattattatcaaagtaatggaattttagcaaataaccccgggtattattacagtaataatataaatcaaatggtacatgttaataataacggtgttttagatactgggattgttaatgttaatggttatgttcaatattttgatgataatggttaccaagttaagggagacatagttaattttaatggtcgaaaaatgtattttgacgatggatctggtaatttagtttacaatcgatttgtttcttacaatggaaattggtactatgcaggttccaacgggctattggtaaacggattacaaaatataaataaccaaagtctttacttcgatgataatggaaaacaagttaaaggtggaatgatttcattagataatcataaaatgtattttgatgctaatagtggaaacctttataaaaatagttttgtattgttagatggagatgtctattatgcaaataatgatggatatattgtaaatggatatcaaaacataggcggaagaaatctatattttgattcagacggaaaacaagtaaaagaccaatttgttaatattaacgggaataaagtatattttaatggtactgatggttctgaagtaaaagacgattttattattcatgatgacaaagaatattatgcggacaatcaaggacatcttttgacgggatataattttgttaatgggcaaaatatgtatttcaatgaggatggatcgcaagtaaaaaattcgattgttagtttagatggtaaattaatgtattttgacgaaaattcaggtaaccaggttaagaatggctttattttacacaatgggaatgtttactattctaacaaagacggcattttggttactggatatcagaatatagacgggcaagatttgttttttaatgcagatggtactcaaattaaaggtggtactgctgaaatagatggtgttaattattattttgaaaatggagaaggacatttagttggcaaagttgaccaagtaattaactcaaatagatttagtgacaataagcttttggatgctaataataatgttgttaaaggattaatttttaataatggtcaattgcaatacttcgattcattaactggagatcaagctaaaaataaacaaattattgctgatggcaatacttattattttgataattctggtaatggaacttatttatttaccaatattggtgaaagtgaaacaaatgatttttcacaaaggaatgcagctaatagtgttaacctaagtgattacaaaaatgttgtagatggattctttacagcagatacttggtaccgtccaaaacaaatattagataatggtactacttggcgtaattcaaatagtaatgatttccgaccaatgattacagtatggtggccaaataaaaacgttcaagttaattatttaaagttaatgcaaaataataatctcttagataagagcaccaattatacattacagtccaatcaacaaatgttaaatcaagctgctcaaaatgcgcaggttaacattgaaaagaaaattgcacaaacgggaaatactgattggttaaatgatctgttatttaaaggaaatggagatacaccatcatttgtaaagcaacaatatatttggaatattttatctgaatcaccaggacaagatgatgctttgttacaaaatggatattttaaatatgttaacagcgagctaacaccaaataccaattcttcatatagaatatcaaataatttatgtgatttcttacttgctaatgatgtggataattccaatccagctgttcaggctgaagacttaaactggttatattatttaactaattttggaactattaccgccaatgatccaaatgcaaactttgacagtattagaattgatgcgtatgcctttataaataatgatattgtccaaagaagtaatgactacatgaaacaaaaatataaattaactgaaagttctaataacgcaaatagccatttgtcaattgtggaggcaggtgtcgatgctggaacgacatcaactaataatgatgagttagtggaatcaccttttagaacaatatcgtatggattaatacacaaagatagaaatcctcaagatatgaataactttataaaagaagtggatacaggtgtcgttattgccgatcatgaaaataattcacaagaaattggacagcctaactattctatcgttcatgcgcatgataaggatatacaagacaaagttggcgaagcgattgttgatgcaaccggaatcaaggactggacgaattttactccttctgaattatctgcaggtttgaaattatattatgatgatcaacgaagttctgaaaaaaaatataatgattataatatacctagcgcttacgcaattatgttgacaaataaaggtacagtcccacgaatatattatggtgatatgtatcaggatgatggacaatttatgcaaaaacaaagcgtttattatgacgatattgtttcactattgacagctagaaaaaaatacgtttctggtggtcaatcaatgtctgtagatcataacaatttcttagaaagtgtacgttttggtaagggagctggtagtgaaagcgattctggtaatgcagaaacgcgtaatgaaggaatcggcttgattgttggaaatgaccagaataagaaattaaatgatggagacactgttgttttgcatatgggtgctgctcatagaaatcaaaagtatcgtgcattaatgttaacgacaaatgatggtataaaaaattacgattctgatgaaaatgctcctattgccgaaacagatagtaatggagatcttgtttttagtaataaggatattaacggacaagccaacacaagtgttagaggtgttttaaacccagaagttgccggatatgttgcagcatgggttcctttaggagcatctgatgatcaggattcgagaacattatctagtaataaatcttataatgatggaaaagtacttcattcaggagatgatttagattctaatgttatttttgaagccttttcaaattttcaaccagaaccaacaaatgaaaatgaatatgagaatgtagtaatcccccaaaaagcttcattatttaaagactggggtattactagttttgaacttcctccacaatacaggtctagtaatgaccatacttttgttgatgcaaccattaataatggttatgcgttctctgatagatatgacctgggatttggtcaacccactaaatatggaactgatgtagatttaagaaacacaattaaatcattgcatgataacggaatgcaggtcatggcagatgtagtttataatcaactatataatttgccggggcaagaagttgtttctgctgtaagagcaggatttactggtaacacagtttcattgccatttggaaatcaattatatgttgtgaatactgttggtggtggtgactatcaaaagaaatatggtggagcatttttgcagaagctataccaagaatatccaagcttgtttgattcagaaaaatatcaatataatagtaagaattatgttactgatttacttgttatgacagatggagaacgttcggcgattccttctgatcaaccaatcacagaatggtctgccaagtacatgaatggaactaacattcttggacgtggtatgggatatgtattaaaagattggaacacaggaacttactttaaactgaatggaaacaattctgtgcttccggatgttttaacttatagaaatagttttgatgataatacaggaactcaatcaagctcaagtgcgcaaagcagtgcatcaaaccatgaaacacaaattagctcaagtgcccaaagcagtgcatcaaaccatgaagcacaaagtagctcaagtgcgcaaagcagtgtatcaagtcatgaagtacaaagtagctcaagtgcgcaaagcagtgcttcaagtcatgaagtacaaagtagctcaagtgcgcaaagcagtgcttcaagccatgaagtacaaagtagctcaagtgcgcaaagcagtgcatcaagttatgaagcacaaagtagctcaagtgcgcaaagcagtgcttcaagccatgaagtacaaagtagctcaagtgcgcaaagcagtgtatcaagtcatgaaacacaaagtagctcaagtgcgcaaagcagtgcttcaagccatgaagtacaaagtagctcaagtgcgcaaagcagtgcatcaagtaatgaagcacaaagtagctcaagtgcccaa

SEQ ID NO: 24 - DNA, 4392 bp, Lactobacillus kunkeei
atgaatatcaatagtaatgaacgtaaggttcgatttaaaatgtataaatctggtaaacaatggattgtagctggattaactacagcagtaatatctattgctgtgtatggtggttcttcaattgccaatggtggaattgaagctaaagctgatgcacaaaacgcagctacttcttcaattgtgaatactaataattctacaaatagtagtaatgctaattcaattgcatctcttcctcaaaatggtacatattcaacaaatgataacggacaaacttggaagtatgtatcacaaaataaggacattcaaggtttatataaggataataatgatcagttaagatattttaacgaatatgatggcactcaagccaagggtgatattgtaaatgttaataatgacaattactattttgataaagacagtggtcagggacataagattgatagctacactgggggaagctactctgaaagtaaggtcaataaccaggatggttggatttataaatcaagtgataacaatgatgttaaaggagtcgctactgtcgacggtaatattcaatattttgatcaaaatacaggtctgcaattaaaaggtggatctgcgcaaattggtggagttgattactattttgacccaaacaagggtaatttagttggaaaagttgatcaagtagtaaactcaaatgattatagcgataataagttactggatagcaacaaaaatgtagttaaaggtttagtagtaaataatggtcagttacaattttttgatacatctaacggtaatcaggctaagaataagcaagtaatagctaatggaattacctactattttgatactaatggaaatggtcaatacttgtttactaatacaggtaagagtgctgttgatgactttacacaaagaaatgctgctaacagtgttaacccaagtgattacaaaaatgttgtagatggattttttacagcagatacttggtaccgtccaaaacaaatattagataatggtactacttggcgtaattcaaatagtaatgaactccgtcctatgattactgcttggtggccaaacaaggatgttcaagttaattatttgaaattaatgcaaaataacggactattagataaaagcaattcgtattcaatacaatctgatcaacagacattaaatcaagcagcacagaaagctcaagtaaatattgaaaagaaaatttcacaaacggggaatactgattggttaaatgatttgttatttaaaggaaacggcgataacccatcatttgtgaagcaacagtatatttggagttcagattcagaatcgccatggcaaggagatgcatggttccaaggtggatatttaaaatatggcaatagtgtcatgacaccaaatactaattctaattatagagattctaataacttgtttgatttcttgttagctaatgatgtagataattcaaaccctgcagttcaagcggaggacttaaattggctatactacttaactaacttcggaactattaccgctaatgattctaatgctaattttgatagtattagaattgatgccgttgattttattagtaacgatattatacaaagaagttatgattacttacgtcaaaagtttaatttaatgcaaagtgatgcaaatgctgattcgcatatttcgttagttgaaggtggagtggatgcaggaactacatcttatagcaatgacggattagttgaggcaccattcagactggatgcttatcctttgctacataagcaagatggagacgtatttaaaaacttaatagatgaagaagattctggaatcgacatttcaaatcataatggagaaaccaatacaaataatactattggtggaataactctatctggtggaaaacctaactattcaattgttcatgcccatgataaggatgttcaagaaaaagtaggtcaagctataatcgatacaactggaattaaggattggactgactttacaccaagtcaattagcacaaggattagaaactttctataacgatcaaagacaaacagtaaaaaaatacaatgattataatgtgcctagtgcatatgcaatcatgctaactaacaagggaacagttcctcgtatttattatggtgatatgtaccaagatgacggtcaatttatgcaaaagaagagtctttattatgatgatatagcaaacttgatgactgcgagaaagaaatatgtatctggtggtcaatctatggttgataataatggaattctaacaagcgtacgttttggtaaaggtgccaatacagttagtgattcaggaacagaagatacaaggaatcaaggtattggattaatagttggatctgcccccaaaaaggttttaaatgatggggataccgttgttttacacatgggtgcagcccataagaaccaaaaatatcgtgccttgatgctaactactgaaaatggaattcaaaattataattcagatgataatgcaccagttgctgaaacagatgataatggtgatttagttttcagtaacaaagatattaatggtcaagctaacactgcaattaaacaagttgccaatccagaggtgaatggttatctagcggcatgggttccggttggggcttccgatgaccaagattcaagaacagcaccatccactagtcaaaataatgatggtaatgttttgcacgaaaacgacgcactagattcaaatcttatttttgaaggattttctaacttccaaccaactccaacaaatcatgatgaatatgcaaacgttgtaattgctaagaatgcgtcactatttaaggattggggtgtaacaagtttcgaaatggcaccacaatacagatctagtcaagatcatacattcgttgattctacaatcgataacggttacgccttttcagatagatatgacttgggatttggtacaccaactaaatatggaacagatgaagacttaagaaatgcaataaaatctcttcatgataatggtatgcaagtaatggctgatgtagtatacaaccaattatataatttgccaggacaagaagttgtatctgcaaccagagcaggtgttactggtaatacaaatgcattaccttttggtactcaattgtatgtagttaatacaatcggtggtggagattatcaaaagaaatatggtggagcattcttaaatgaactgcaagaacaatatccatcattattcaaatctcaaaagtacaagtattactacaaaaattatgctaataatggtgctggaccaggttatttaacagttaatgatgcagaacgttcggatattccatataatcaaccaatcactgaatggtcagctaagtatatgaatggaactaatattcttggacgtggtatgggttatgtattaaaggactggaatacaggtgattatttcaagttaagcgggagcgattcaacactaccaagtagtttaacttacaagagcggttgggttgaaaatcctgatagtacttggtcatactatgaaaagaataatattgacaaattaactggatctcaagttattaatgaggaaagagttttctttgataacaacggtattcaagttaaaggaggatgggtaaaaaattcaaatggtacctattcttactatgacaagaatagtggaaacatcctaactggtgatcaattaatcgacggtgaacatttcttctttgataacaatggtgttcaagtaaaaggaaaatggataaagaatagtgatgggtctaagtcatattacgattctcacttaggaaaacttataaagacggataaaaaagtatcttctaatgctcgaaaaaagaaatctaaggaagaattattgtatgagaatgccttaaaagttttaagaaaagataagaaacgtctcgataaaaataagacaaaggcaaatatcagaaaatataataaatctctaaaaaaatatcgtaaagcaaagaagaaacttttagcgattactaagaatagagttgctaatgctagaaaagcgattaaaattgctaaaaaagttctttctaagagaaaaaatattaataatgaaaaaagatattataaagctctaaaagaatattatgtagcggaaaaatcatatttgaaaattactggaaattacaataagaagtattattacgaatttgataaacttactccaaaagtcaaagtggttaagaacatttattcctataagagtagacattttactaaaaagaatagagttaaaaagattaaaaaaggtactcttgttagagttaaaagtatagttcgaagtggtaaagtcgctcgaattaatatcggaaatggtcattttataacttcatctaaagattttattaagatgtttaaataa

SEQ ID NO: 25 - DNA, 8475 bp, Leuconostoc carnosum
gtgacagcaggaattttctctacggttgtgtttggtatggccgtatctgacgttagtgctaatgacactgacaacactgtgttaacttcgaacagtggatttttagataaagtagtagatacgacaagtacggataaggcagccacaccagataaagtagtagatacgacaagtacggataaggcagtcacaccagataaagtagcagatacgacaagtacggataaggcagtcacaccagataaagtagcagatacgacaagtacggataaggcagccacaccggataaagtagtagatacgacaagtacggataaggcagccacaccggataaagtagtagatacgacaagtacggataaggcagccacaccggataaagtagtagatacgacaagtacggataaggcagccacaccagataaagtagtagatacgacgagtacggataaggcagccacaccggataaagtagcagatacaacgagtacggataaggcagccacaccagataaagtagtagatacgacgagtacagataaggcagccacaccagataaagtagtagatacgacgagtacagataaggcagccacaccagataaagtagtagatacgacaagtacagataaggcagccacaccggataaagtggtagatacgacaagtacggataaggcagcagatagaaccattagtatttctggtaaaacagttaaaaatattgaggaaattggtgggaaaacttattttgtaggggatgatggcaaagtcaaaaaaaacttcacggttattgttgatgggcaagtaatgtattttgacaaagagtctggagcattgacttcgaaccataagcaatataaagaaggtctttcagatataacaaatgaacataatgctgcctattcattagaaaacgacaactttacacaaattgatagttacttaactgccaatagttggtaccgtccaaaagatatattaaaaagtggcacaacatggacagcctcaaccgataaagactctcgcccattacttatgtcatggtggccagatcaacaaacagaactatcttatttaaagtatatgcaatcagcaggtttcttagcagaggatgttaatttatcagaaaataatagcattgatgatctaacagctgcagcaatggatgttcagaaaaatgttgaagcaaagattagcctatcaggtaatacagattggttgaaagaagatatgaatcagtttgttgattcacagtcaaattggaatatcagcagtgagtcaaaaggcactgatcatcttcagggcggcgctttattgtatggtaacagtgatatgacaccagatgctaattctgattatcggttactgaatcgcacaccaaaaaaccaaaccggacaaatcagtgctacgaatgatcagggtggttatgagatgttattggctaatgatgtcgataattctaatccaattgttcaagccgaacaattaaattggttacactacatgatgaacattggtagtattacaaaaaatgattcaacggctaattttgatggttatagagttgatgcggtagataacgtgaacgctgatttgttacaaattgctggtgactacttcaaggccgcttatgggacggacaaaagtgatgcaaatgctaataatcatatttctattcttgaagattgggataatagtgatcctgactacgtcaaaaagcacgggaatgaacaattaactatggattttccgatgcatttggcattaaaatatgctttaaatatgcctattgatatgcgtagtgggcttgaaccggcaattaagacaagtctggtgaaccgatcacaagatgcaacagaaaatgaggcacagccaaactactcgtttatacgtgcccatgatagtgaagtacagactgttattgctcaaattattaaagataaaattaatccaaagtcagatggtttgacagttacacctgatgaaattgcgaaagcttttgaaatctataatgcagatgaactaaaagctgataaggcatacacagcttttaatatcccgtcatcttatgcacttttgttgactaataaagatacggtgcctcgtgtttactatggcgatttatttacagatgatggacaatatatgtctgatcattcaccatattatgatgctattacgactttattagcgtcacgtattaaatatgcggctggtggtcaaagcatgggtatgacgtatttacacgataatcaagaagttttgacatctgtacgttatggtaaaggggctctgacagcagatgatttgggtaatgttgacacacgtacacaaggtattggacttgttatcagtaataaaacggatttgagtttaaagagtgatgagagcgttgtgctgaatatgggtgtcgcacataaaaatcaagcatatcgcccggcaatgttgactactaagtcaggattaaaaatttacgatactgatgatggtgcaccaattgtttatacaaataatttaggacagctaatttttaacgcagatacagtctatggtgtgagtgatccacaagtttcagggtaccttgctgcgtgggttcctgttggcgcaactgaagatcaagatgctagaactaaaggcagtcatgatggaacaactgatgggaatgtctatcattccaacgctgcattagattctcaggtcatatatgaaggtttctctaatttccaggcaatgccaacgaccactgatgaatatactaacgtaaagattgcacaaaatgcacagtggtttaaaaaattaggactgacaagttttgaactggcaccgcaatatcgttctagcacagatagtagctttttagactctgttattcaaaatggatacgcttttactgatcgatatgatgtgggttataatacaccaacaaaatatggtacagtcgatcaattattagatgcattgagagcattacattcacaagatatccaagcaattaatgattgggtacctgatcaaatttataacttacccggggagcaaattgtaacagcgagtcgtaccaatggatccggaaaatacgatgatgattcagtgattagtaatactttatatgattcacgtactatcggtggtggagaatatcaagcgatgtatggcggggctttcttagatcaattgaagcaagcatatcctggtttgtttgaaacaaaacagctttctactggtgttgcaatggatcctgatgtaaaaataaaagaatggtctgctaagtattttaatggttctaacattcaagggcgtggtgcttggtatgtactaaaagactgggcaactaataagtacttcagtgtctcgagtaataatacatttttacctaagcaattattgggtgaaaaagctagtacaggatttattacgaacgatggaaaaacagaattttattcaacaagtggctaccaggcaaagaatacatttattgaagacaacggtaactggtattacttcgataatgatggttatagcgtagttggaaagcaagtgattgataataaacactactatttcttgcctaatggtgtcgaattgcaagatgcctatttatcagatggggataagcaatattattataaaaaaactggtcgacaaatagtaaatcagtattatagagatgagcaaggtgattggaggtatttctttgcagatgggcatatggctcttgggttaactgacattgtttcaaatgatggaactcatgcgacacagtattttgataacaatggtgttcaagtgaaaggaacatcagaacgagataaagatggtaatattcactattttgatggtacatctggtaatttagttgttagttcatggggacaattgtcggacggatcatggctttacctgaatgataaaggcattgctgttacgggtgctcaacaaattgatggtcaatcactatactttaatgaagatggtaaagaagtaaagggtgatgcggtaacagataatcaagggaatatacgttattttgatggtgaatctggtcacatggtggttaattcatggggtaaattacctgatggttcatggatgtatttgaatgataagggtattgctgttaccgggcaacaaaaaatcaacaatgaagtcttatatttcaatgctgatggtaagcaaatcaaaagtgcatttaaagaactagtggacggatcatggctttacctgaatgataaaggcattgctgttacgggtgctcaacaaattgatggtcaatcactatactttaatgaagatggtaaagaagtaaagggtgatgcggtaacagataatcaagggaatatacgttattttgatggtgaatctggtcacatggtggttaattcatggggtaaattacccgatggttcatggatgtatttgaatgataagggtattgctgttaccgggcaacaaaaaatcaacaatgaaatcttatattttgatgctgatggtaagcagttaaagaatacactgaaaacattatccgatggttcacgtatttatttggatggtaaaggtgtttctgcaacaggtgttcaaaaaattaatggtaaagtgtcatactttgatgttaatggcaaacaagttagcaatcatattcaagaactccctgatggttcatggatgtacctagataatgatggattagctctaattggtaatcaagacgttgatggcaaacaactttactttgatgttgatggtaagcaaataaaaaatgacaaagtcaaaaatagtgatggaacaattaattattacacgggtactgttggtgaaaaactaaagcatgattttggtcagttatccgatggttcgtggatgtatttagatgaaaatggtaatgctgttactggtgaacaaaatattaatgggcaacatttatactttaaagatgatggacagcaagttaaaggagatgtttttgaggatgacttaggccgtatgcgttattatagtgctaactcaggtgagatggttgtcaatcaatttgaacaaatttctgatggtgcctgggcttactttggtgatgatggtgtggcggtaactggtgaacaacatatcaatggacaagatcttttctttgatgcgacaggtcaacaggttaaaggtgaaagtcgaaccattaatggtattccttatacctttgaaaaggagagtggtgagaaacggtctgttaatatagcaccattactagccatgggaaattatgttacaaataatggtacagattggcaatatgaagtgcaaggcaatcctgttaaagggttatatagcacttctgataataagttgcgttattttgatctgacaacaggtgtacagattaaaggcaactttgttactattggacataacacatactatttcaatccagctaatggagacggtgaattattgccagatgtttctgatggccattatggtacgatccaagttaaagatgcgaatacaaatgaaaagacagtttgggtttaccgtaatcaaagtaatactattttgaaaggtattcaaaatattcatggtaatatacaatactttgacttatcaactggggagcaaataaagggtggtattgcaaactatgatggcaatgattattactttgaatcagcaaagggtaacctcacaagtaaaattaagcaagtctatacagatggtcaatatgtaactaaagatggaaaaagcatttatgaagacgcacaacaacaaagtgtcagtgggttagtgtctattaatggtcagttacaatacttcaatccacaagatggcgtacaagttaaaaatcaacaaattattgttgatggcgttacttactactttgatgaaaatggcaatggtcagtatttgtttacgaatacaacggtcatgccaatggatgattttacaaagcacaatacagtttatagtgataacgacaacaactttaaaaataatgttgatgggttcttaactgctgatacatggtatcgtccaaaggaaatcttaaaagcaggaacaacttggacaacaacatcggaaagtgacatgagaccactgatcacgacatggtggccaaataaaaatgtgcaagttaactatctaaactttatgaaacaaaataatctattgcacacaaatgtggagtatagcttgctatctgaccaatatgatttgaatattgcagctcaagcagtacaaacagctattgaaaagcgaattgctcaagaaaatagcactgattggttgcaaaatcttctattcacagctcaagacgatcaaccatcttttgttaagcaacagtttatttggaataaagattctgaataccaaggaaaaggtgatgcttggttccagggtggttacctgaaatacgggaacaataaattgacacctaataccaactcaaattatcgtaaaactgacaacgcgtttgaatttttgttagcaaatgatatcgataattcgaatccggtcgttcaagctgaaaatcttaattggttagaatatctgatgaattttggtactataactggtaaggatgacgatgcaaactttgatagtattcgtgttgatgctgttgattttattagtaatgatacaattcaacgaacatatgattatttacgtgatgcctatcaagtagatcagagtgaagccaaggctaatcaacatatttcattagtagaggctggattagatgcaggaacatcaacagttaaaaatgatgcgcttattgaatctaatttgcgtgaagcggctacgttatctttggccaatgcatctggtaaaaatagtgcgttaaccaatatgttgcaagatgttgatggtggaacattgattgcagatcatacccataattcaaccgaaaatgaagccacaccaaattattcaattattcatgctcatgacaaaggtattcaagagaaagtgggggctgcaatttccgatgctactggggccgactggactaattttacagatacacaattaaaatctggtttggatctttattataaggatcaacgtgctacggataagaaatataatatttataacttgccaagtatttatgcattaatgctcaccaataaagacaccgtaccacgtgtttattatggtgatatgtatcaagataatggtcagtatatggcagagaaaagtatctattataatgctttagaatcattaatgtcagcacgtaaaagctatgtaagtggtggacaaactatggatgttgatagccacggtttgctaaaaagtgttcgttttggtaaaggggctatgactgctgacacggtaggtaatgaagaaacaagaactgaaggtatcggtgtgttagttggtaacgatgcttcattgaaactcaatgattcagatacagtgaccttagatatgggcgcagcacacaaaaatcaaaagtatcgtgcagcaattttgactactaataatggtctatcaacgttcgattctgataaagatgcaccgattgcttggactaatgataaggggatactaacattttcaaataaaaatgttagtggacaagataatactaatgtccatggtgttgctaatccacaggtatctggttatttggcagtatgggttccagttggtgctaaagatgatcaaaatgctgggacaagcgcatctacagtagtcaacacagatggtaaagtattacactctaatgcatcattagattccaacttaatttttgaaggattctctaacttccaacctagagcgacaacaaatgacgaattaaccaatgtcgttatagctaaaaatgccgatttattccagaaatggggtattactagctttgaaatggcaccgcaatatcgctcaagtcaggaccacacatttttagattcaaccattgataacggttatgccttcacagatcgttatgacttaggatttaacacaccaacgaaatatggaacagatagtgatttgcgattggcaatcaaatcattacataaagctggcatgcaagtaatggctgatgttgttgataatcaagtctataacttaccagaccaagaagttgtttctgcttcacgcgcaggtgtatatggtaatgatgtcgcgaccggatttgatacacaattgtatgctgttaattctgttggcggcggtaaatatcaagcacagtatggtggacagtatttgagtgagttaaagaataagtatccagatttgtttgaagctaaagcttatgattattggacaaaaaattatgctaatgatggatcaaacccgtactacacattatcacaacagactcgagatgatataccatcagacgagaaaattaagcaatggtcagcgaaatatatgaacgggaccaatgttttgggacatggtatgggttacgtacttaaggattggaatacgggtcaatattttaagattaataaagatggcgattccaacttaccagtttaa

SEQ ID NO: 26 - DNA, 8436 bp, Leuconostoc mesenteroides
atgagagacaaaagaataatatgcgatcgtaaaaaattgtataaatctgggaaactgttagtgacagccggtattttttctgctgtgatatttggcgtttccacaactaacgtaagcgctgatagcactaacaacactggtgttacggtgtcacaagcaacagataaagtagcagacacgacggctacaacggacaaagtagcggacacaacagctacaacagataaagtggccgacacagcagctacaacggacaaagtagcggacacaacagctacaacagataaagtggccgacacagcagctacaacggacaaagtagcggacacaacagctacaacagataaagtggccgacacgacggctacaacggacaaagtagcggacacaacagctacaacagataaagtggccgacacagcagctgcaacagataaagcagccgatacagcggctacaacggataaagtggccgacacagcagctgcaacggataaagtagcggacacagtagctgcaacggacaaagtagcggacacaacagctacaacagataaagcagccgatacagcggctacaacggataaagtaaccgacacaacagctgcaacggataaagcagcggacacgacggctacaacagataaagtggccgacacaacagccacaacatcagaaaaatcaaaaagtattaaacaaattgatggtaaaacttatttcattggtaatgatggtcagcctaagaaaaattttacagccattgttgacggtcaagtattatatttcgacaaagatactggtgctttgacatcaaatagtagtcaatataccgatggtttagccaatataggaaatgagcataatgcggcttattcattgtcttcggatagttttacacaagttgatggctatctaacggctaacagttggtaccgacctaaagatatattaaaaaatggtacaacttggacggctgcaacagcaaacgattttcgaccattgttaatgtcttggtggccagataaagatacccaagtttcatacttaaaatatatgcaatctgcgggattattatcagatgacgttgcattatcaaacaatgatagtatgaacagtttgacggatacggctatgactgttcaaaaaaaaattgaagaaaaaattggcttattgggcagtactgactggcttaaggccgatatgaaccaaatggttgattcacaatcgaattggaacattagtagtgagtctaaaggaacagatcatttgcaaggtggtgcgctcctatacgttaatagtgatttaacaccaaatgccaattctgattatcgtttattaaatcgaacgccaactaaccaaaaaggtcaaattacaacaaatggtaatcaaggtggctatgagatgctgttggccaacgatgttgataattctaacccaattgttcaagctgaacaattaaattggttatactacatgatgaatatcggtagcatcgcccaaaatgatccaacagcaaattttgacggttacagagttgatgctgttgataacgtgaatgctgacttgttgcaaattgctggagattattttaaagcagcatatggaacaaatcaaagtgacgctaatgcaaacaatcacatttccatcttagaagactgggacaataatgatccagcgtatgtaaaagcacaggggaacaaccaattaaccatggattttccaatgcatttggcattgaagtattcattgaatatgccaagtagtgctcgtagcggtttggaaccagcaatttcaacaagcctagtaaatcgtgcagcagacgccacagaaaatgaagcccaaccgaactattcatttattcgtgcacatgatagtgaagtacaaacggttattgctcaaattattaaagataaaattaatcctagttccgatggattgactgtctcaacagatgaaattgccaaagcattcgaaatatataatgctgacgaattaaaggctgataaagagtataccgcatataatataccctcatcatatgcattgatgttaactaacaaagatacaattcctcgtgtgtattatggtgatttgtttacggatgatggacaatatatgtctgcaaaatcaccatattatgatgcacttacttcattgcttcaatcgcgagtaaaatatgtttcaggtggtcaatctatgaatatgacttaccttcataataatcaaggccttttgacgtcagtccgctatggaaaagacgccatgacagctaacgacactggtacaagtgaaacgcgcacacaaggtattggattaattgtcggcaacaaaactgatttaaacctgaataatgatgagcaaattgtacttaacatgggggccgcacacaaaaatcaagcttaccgtgcattaatgttaagtactaaagatggcttgaaaatttataataatgatgacgaggcaccggtatcgtatacagatgaccaaggccgtttgatttttaaatctgatgtggtttatggtgtgagtgatgctcaggtttctggttatttagcagcttgggtgccagtcggtgcaaacgatagccaagatgctagaacagaaagtagtacaacagcgtcaacagatggtaatacctatcattcaaatagtgccttagattctcaacttatatatgaaggcttttcaaacttccaagccatgccaacacaggccgatgagtataccaatatcaagattgccgaaaatgcacaattattcaagagccttgggataacaagctttgaattggcacctcaataccgttcaagtacggataacagtttcttagattcagttattcaaaatggctatgccttcacggatcgctacgacattggttataatacgcctacaaagtacggtacagttgaccaactattagatgctttaagagcattgcatgctcaaggcattcaggctatcaatgattgggtcccagaccaaatttataatttgcctggggaagaaatagtgacagccagtcgaacaaacggttcgggaaaggtgaatgaaagttcagttattaataatacgctatatgattctcgtactgttggtggcggagagtatcaagcaatatatggaggtgctttcttagataagttaaaacaagattatcctgagttatttgaaacaaaacaaatttcaacaggtgaagcaatgaaccctgatgtcaaaatcacagaatggtcagctaagtattttaatggctcaaacattcaaggacgtggtgcatggtatgttctcaaggattggtcaacaaatcaatactttaatgtttcaagtggtagtgaatttttacctaagcaactgttaggcgaaaaaacaagtacagggtttaccaacgtggacaatggcaagactgagttttattctacgagtggctaccaagcaaagaatacatttattcaagataatgacaattggtattattttgataatgatggctatatggttgttggcggtcaagaaattaatggtaaaaaatattatttcctaccaaatggtgtagagttacaagatgcttatttgtctgatgggactagtgagtattactacagtagtgatggtcgtcaaatttctaatcaatattatcaaggatcagacaacaactggcgttatttctttgcagatggtcatatggctgtagggttagcaacaattactacagaaaatggtacaacaaatcaacaatatttcgatgcaaatggtgtgcaacttaagggcgtagctataaaggatactgatggcaatgtgcactattttgatggcaagacaggaaacatggttataaattcctggggtaaaataagcgatggttcatggttatacttaaatgatagcggtgtagcggtcacaggaccgcaaaatattaacggccaaaatctttacttcaacgaagacggtattcaagtaaagggtgaagccattactgataatagtggaaacatacattattatgatcgcagcacaggaaatatggttgtgaactcatggggtgaaacgaataatggttcatggctatacttgaacgacaagggtgatgccgttacaggagaacaagttattgacggtcaaaaactatatttcagtagtaatggaatccaacttaaaaatacattcaagaagctatccgatggttcatggctatatttgaacgataaaggtcttccagtgacaggagcacaggtcattgatggacaaaacttgtatttcgaccaagatgggaagcaagtcaagggtgacgttgctacagatggacaaggtaacactcattattatgatggcaacacaggaaatatggttactaattcatgggcagagttaccggacggttcatggatgtatctagacaatgatggcaatcctttaacaggacagcaaaagattgatggccagtcactctactttaatgatgctggtaagcaaatcaaaaacgcattggttaaactagatgatgggtcaacaatttacctcgatgataaaggtgtttcatcaactggtattcaaagaattgatgataagatatattattttgatcctgatggtaaacaagtagtatgtcgttttgaagaattaccagatggttcatggatgtatctagatgatgacggtgttgctgctacgggcgctcaaaaaattaatggccaggaattatatttcgacaatagcgggaaacaagtcaagaacgacaaagtaattaatgacgatggaacaataaactattacacaggtatgagcggtgaaaaactaaaaaatgattttggtgaattaccagacggttcatggatgtacttggataatcaaggtaatgctgtaataggtgcccaaaaaattaatggccagaatctttacttcaagacagacggacgacaggttaagggtgaagcaaatgttgattcatcaggtgaaatgcacttctatgatcctgattctggcgagctaattacaaatagatttgaacaagttgctagtggtgtatgggcttactttgatgccaaaggtgttgctgtaactggtgagcaacgcattggtaagcaaaatttattttttgatccaactggttatcaagttaaaggcgacaaacgaacaattgacggcgttctctatacctttgataaagaaagtggtgagagaaagggtttagattctatatcggtattacccaccaatggacaatacacaaccgataaggcccaaaattggtattaccaagtcgatggtgaaaatgtaaaagggctatatacaaataatgatggtcaattacgttacttcgatttgacaactggcgtgcagactaaaggtaattttgtgacaattggcaatgatacctactatttcaccaaggaacaaggggatggacagatagtttctgaggttgtgtcaggacactatggtactgtccagttgagtgacaattcgtctgcatgggtttatcgcggtgcaaatgatcaaattttgaaaggcctacagaatataaacggtcgtctgcaatattttgatctaaccaccggtgcgcaattaaaaggcggtgctgcaaactatgatggcaacctttattattttgaatcatcagatggtaacctagtcagtaaaattcagcaatcttattctactgggaattatgtgaccgatggtgataaagtaacatatgctgatgagcaaaacaaccaagtcacgggattagcgttgattgatgatcaactacaatacttcgatccaagtgacggtcgtcaagtcaagaatgagcaggttatcgttgatggcgtcacatactactttgataaaaatggtaatggacaatacttgtttacaaatactgcaacgatgtcaactaatgaatttgccaaacatagtgctgcttatagcaatgatagttctagcttcaagaatacgatagatggtttcttgacggccgatacctggtatcgccctaaagatatcttggaaaacggacaaacgtgggtagtttcttcaacaaatgacgtgcgaccactgataacagtttggtggctaaataaagatgttcaagttaattattcaaattttatgaagcaaaatggtttgctagatacaagtagtcaatttaatctacaatctgatcaatatgacttgaatgtcgccgcgcaaaaagttcaagtggctattgaaaaacgcatttcgaaagaaaagagtacagattggttgaaagatcttttgtttgaagctcatgaagatacgccttcatttgtgaaacaacaatttatttggaataaagattctgaatatcaaggtcaaggggatgcgtggttccaaggtggttatctgaaatatggtaacaatgaattaaccccaacaacgaactcagattatcgtgaatccggtaatacattagacttcttgcttgctaatgatgtcgacaattctaacccagcggttcaagctgaaaatttgaattggttacattatttaatgaactttggcacgattacagctaatgatgatgatgctaattttgacagtattcgtattgatgccgttgactttattgataatgatgccattcagagaacctacgattacatgcgtgatgcttataaagttgatgcaagtgaagacaacgctaataagcatatttcactagtggaagctggattagatgctggtacctctacaattaagagtgatgctttagttgaatctaactttagagaggcagctacactatcgctagcaaatcaatcaggggaaaatagttccttgactaatatgttgcaagacattgatggtggccagattatagctgatcacgccaacaatgcaacagaaaatgaatcaacgccaaattattcaattattcatgctcatgataaggggattcaagaaaaggttggtgcagcaattaccgacgttactggtgcagactggacgaatttcaccgatgaccaattaaaagaaggattagcagcttattatcaagatcaacgttcaacgaataaaaagtataacatctataacttacctagtatctatgctttaatgttgaccaataaggacacagttcctcgtgtttattacggtgatatgtatcaagatgatggccagtatatggaaaagcaaagtatttattatgatgccattgtttccttgatgaacactagaaagagttatgtgagtggtgggcaaactatggatgtagatgaacatggtttgttgaagagtgttcgttttggtaaagacgcaatgacagctagtgaccttggtacgaatgaaacacgcactgaaggtgttggtgtgctggtcggcaatgattcttcactaaaactaaatgattcagatacagttactttagagatgggggcggctcataaaaaccaaaagtaccgagctgcattgttgacaactagtgatggtattgttacgtatgatgctgataatgatgcaccaacaatctggacagatgaccgtggtacattgacgttctcaaataaggagattgctggtcaagattatactagtgtgcaaggattcgctaattcacaagtatcaggttacttagcagtttgggtgcccgtaggagctagtgacgatcaagatgtccgaacagcagcattaacagatgcaaatcttgatgacaaagtactgcattctaatgctgcattagattcgaacttgatttacgaaggcttttctaactttcaacctaaagcaaccaccaatgatgaattgactaacgtagtaattgctaaaaatgctaatttatttgaaaagtggggaatcacaagttttgagatggcaccacaatatcgttcaagtggggaccacacgttcttagattcaacgattgataatggttatgcatttactgaccgatacgatttgggatttgaaacaccaactaagtacggtactgataaggatttgcgtactgcaattaaagcattgcaccaatcaaatatgcaggttatggctgatgtagttgataaccaagtttataatttatctggacaggaggtcgtatcagcttcacgtgccggtgtttacggcaatgatgtgtcaactggatttgggacacaactctatgcggttaatagtgttggtggtggtaaatatcaagcccaatacggtggtgaatatttgaatgaattgaagcaacaatacccagatttgttcgaagctaagacgtatgactattgggttaaaaattattcaaatgacggatcggatccgtattacacactgtcgcaaaacacacgaaaagatatgccaagtagtgaggtcattaaacaatggtcagctaaatatatgaatggtactaatgtattaggaaacggtatgggatatgttttgaaagattggaatacaggtgagtatttcaaaattggagaaaagaatgctgattttataacaaattaa

SEQ ID NO: 27 - protein, 1107 aa, Leuconostoc mesenteroides
VKGDKRTIDGVLYTFDKESGERKGLDSISVLPTNGQYTTDKAQNWYYQVDGENVKGLYTNNDGQLRYFDLTTGVQTKGNFVTIGNDTYYFTKEQGDGQIVSEVVSGHYGTVQLSDNSSAWVYRGANDQILKGLQNINGRLQYFDLTTGAQLKGGAANYDGNLYYFESSDGNLVSKIQQSYSTGNYVTDGDKVTYADEQNNQVTGLALIDDQLQYFDPSDGRQVKNEQVIVDGVTYYFDKNGNGQYLFTNTATMSTNEFAKHSAAYSNDSSSFKNTIDGFLTADTWYRPKDILENGQTWVVSSTNDVRPLITVWWLNKDVQVNYSNFMKQNGLLDTSSQFNLQSDQYDLNVAAQKVQVAIEKRISKEKSTDWLKDLLFEAHEDTPSFVKQQFIWNKDSEYQGQGDAWFQGGYLKYGNNELTPTTNSDYRESGNTLDFLLANDVDNSNPAVQAENLNWLHYLMNFGTITANDDDANFDSIRIDAVDFIDNDAIQRTYDYMRDAYKVDASEDNANKHISLVEAGLDAGTSTIKSDALVESNFREAATLSLANQSGENSSLTNMLQDIDGGQIIADHANNATENESTPNYSIIHAHDKGIQEKVGAAITDVTGADWTNFTDDQLKEGLAAYYQDQRSTNKKYNIYNLPSIYALMLTNKDTVPRVYYGDMYQDDGQYMEKQSIYYDAIVSLMNTRKSYVSGGQTMDVDEHGLLKSVRFGKDAMTASDLGTNETRTEGVGVLVGNDSSLKLNDSDTVTLEMGAAHKNQKYRAALLTTSDGIVTYDADNDAPTIWTDDRGTLTFSNKEIAGQDYTSVQGFANSQVSGYLAVWVPVGASDDQDVRTAALTDANLDDKVLHSNAALDSNLIYEGFSNFQPKATTNDELTNVVIAKNANLFEKWGITSFEMAPQYRSSGDHTFLDSTIDNGYAFTDRYDLGFETPTKYGTDKDLRTAIKALHQSNMQVMADVVDNQVYNLSGQEVVSASRAGVYGNDVSTGFGTQLYAVNSVGGGKYQAQYGGEYLNELKQQYPDLFEAKTYDYWVKNYSNDGSDPYYTLSQNTRKDMPSSEVIKQWSAKYMNGTNVLGNGMGYVLKDWNTGEYFKIGEKNADFITN

SEQ ID NO: 28 - protein, 856 aa, Leuconostoc mesenteroides
TMSTNEFAKHSAAYSNDSSSFKNTIDGFLTADTWYRPKDILENGQTWVVSSTNDVRPLITVWWLNKDVQVNYSNFMKQNGLLDTSSQFNLQSDQYDLNVAAQKVQVAIEKRISKEKSTDWLKDLLFEAHEDTPSFVKQQFIWNKDSEYQGQGDAWFQGGYLKYGNNELTPTTNSDYRESGNTLDFLLANDVDNSNPAVQAENLNWLHYLMNFGTITANDDDANFDSIRIDAVDFIDNDAIQRTYDYMRDAYKVDASEDNANKHISLVEAGLDAGTSTIKSDALVESNFREAATLSLANQSGENSSLTNMLQDIDGGQIIADHANNATENESTPNYSIIHAHDKGIQEKVGAAITDVTGADWTNFTDDQLKEGLAAYYQDQRSTNKKYNIYNLPSIYALMLTNKDTVPRVYYGDMYQDDGQYMEKQSIYYDAIVSLMNTRKSYVSGGQTMDVDEHGLLKSVRFGKDAMTASDLGTNETRTEGVGVLVGNDSSLKLNDSDTVTLEMGAAHKNQKYRAALLTTSDGIVTYDADNDAPTIWTDDRGTLTFSNKEIAGQDYTSVQGFANSQVSGYLAVWVPVGASDDQDVRTAALTDANLDDKVLHSNAALDSNLIYEGFSNFQPKATTNDELTNVVIAKNANLFEKWGITSFEMAPQYRSSGDHTFLDSTIDNGYAFTDRYDLGFETPTKYGTDKDLRTAIKALHQSNMQVMADVVDNQVYNLSGQEVVSASRAGVYGNDVSTGFGTQLYAVNSVGGGKYQAQYGGEYLNELKQQYPDLFEAKTYDYWVKNYSNDGSDPYYTLSQNTRKDMPSSEVIKQWSAKYMNGTNVLGNGMGYVLKDWNTGEYFKIGEKNADFITN

SEQ ID NO: 29 - DNA, 4848 bp, Artificial sequence
  Codon-optimized sequence encoding mature GTF8117 with added methionine
gtggacgagacaagcagctcaaacgaaacacaaacggaacaaacgcttaacacggatgagtcaacagacacaacgacggacgtctcaaatgaggccaaagcaacggaggcacaactgacaacgcaagatgcagacatggcgagctcagaagaaaaaacaacgaatgtcgagaaagaggttacaacggctgaaacaaataaagacacgacggtcaaaaatgtggagtcaagcgaacagaatacaacgacagtggcagacaagaatgccgtggattcaacagctcaagttaacacagcggagaaggagaacaagtacacgcaggagaatgtgaacggcaattggtatctgaaagatgagcagggcaactatcttacgggattccaagagattaaagaccaaaacaaaacagtgtattataaccctgatagcaagcagatggtctacggacagcaaaacatcaacggaaactggtaccttttcgatacattcaatggagcgatgcaaacaggacttcaatatatcagagatcaaaaaaagcttgcttattacaatgaacagggacaaatgcaatatggcacagtcgagatcgatggacaaaagtaccaagcggatacgtttaatggcgcgatcaaaggcaaaggccagacaaaaatcgctgacaattggtatcttttcaataatgccggacaggtcgtggatggctggcagtggattaacgaccagggaaagacagtttattactcaacaaaaacggcccaaatggtccatggccagcagaatattaatggacattggtacctgttcgataagacaacaggcgctatgcaaagaggcttccaaaaccttaaagcctacggagacgacaagacggtgtactataatcaagacggctggatgctgtatggccaacagaagattgataacaagtggtacaatttcgacacgttcaatggagctatgaagacaggattcgtgaaaattccggagcagaacaagacagtctactacgcaccgaacggccaaatgcagtatggctggcagtgggtcgataacgcgacgagatatttcgacacgtttaatggcgcaatggcaacgggacagaagctgattacaggacactggtatctgtttgacaacaatggcgcaatgcagagaggcttccagaatctgaagaattatggagacaataaaacggtttactacaaccaagatggatggatgctttatggctggcaatgggtcaacaacgctacaagatactttgacacatttaacggagccatgacgacgggccagaaaaagattaatgaccattggtacctttttgataaggacggcgccatgcagagaggaatccaatacatccctgaggaaaataagcttgtgtactacaatcaggacggatggatgctgtacggcaagcaaaatatcaatggcgtcgatcataactttaatacgttcaatggagcacttgaggctaagggccaagtgaaagtgggcaataattggtatctgttcaacaatagcggaacgattcagacaggctttcaggacctgaaggcttacggccaggataaagtcgtttactatgatcctaagacggcagccatggtttatggatatcagaacatcgacggcaactggtaccttttcagcagagcaaatggcagcatgcaaagaggccttcaaaacgtcaacggcgttgacctgcttttcgatgaaaagacgggcgcactgctgacaggagttcaaaatatcaagggaaataactactttgtggataagagaagcggaaacatcaagaagaaccttgtggtccttggagccgataataagtggatgtacttcgatgcgaaaacgggaaaaggcacgaacacgcttgaggatcagtacaaaaaaggagttgttagcggcaacgtggaatttattacgaataacgcagcgtatagctttgatggcaatagcttcgaaaacattaacggcttcctgacggccgattcatggtacagaccgaaatcaattcttaaagatggctcaacatggacagcaacaacagagacagaccttagaccgctgctgatgacatggtggccgaacgaacaaatcaaggccaactacctgaactacatgaaggacaagggattcatcaataactcaggcacgtataatgctgagtcagacccgaactatatggacttcgctgcccaggaggcgcagagaaatattgagagaaaaatcacgaaggaaaacgatacgacgtggcttagagatcttatcacagacttcattaaaacacaggatatctggaacgagcaatcagagggagttagcacggagggcctgcaaaaatttcagggcggctttcttaagtatgtgaatagcgagctgacgccttacgcaaactcagaatggagaaaactgggctaccaaccgacgatgcttacacaaaataacgttggcgcggagttccttcttgccaatgatatcgacaactcaaatccggtcgtgcaagctgaacaacttaactggctgcactttctgatgaactttggcacgatcacagctaacgatccgagcgcgaacttcgacggaatcagaatcgatgcagtcgataatgtggacgcatcactgctgtcaatcgctggcgattatttcaaggcagcgtacaaggtgggccaaaacgatgccacagccaacaagcacatctcaatcctggaagactggaacgataaggaccctgagtacgttaatagcatcggaaacccgcaactgacaatggatgactacatcgtgcaacaactgaaattttcactgggacaggcacctgataaggtcgacagaatgcaaagatttaaggagtggtacctggttgacagatcaaaggataatacggaaaacacagcgatcccgaactatagcttcgtgagagcacatgacgcctcagttcaagaggacatcctgcagctgatccaggacacgacaggaaaaccgtggggcgtctatacgaacgaagagctgcaacaaggcctgaaggactatatggcggaccagaagcttacgaacaagaaatacaatagatacaacatcccgagcagctatgctatcctgctgacaaacaaagacacaatccctagagtgtattatggcgacctgtatagcgacgccggaaagtacatggccgagaagtcaatttactttgatgccattgacaacctgcttaaaacgagaacgaaatatgtggcaggcggccaaacactggacgttgacggacatgatatcctgacaagcgtcagattcggaaagggagccctgaatgtcacagataaaggcacgagcgagacaagaacgcaaggcatgggactgatcatcagcaataacaactcactgaagctgaacgacggagaaaaggttgtgcttcatatgggcgccgcacacaagaatcaagcctatagagcagtcatgcttagcagcgcaaatggcctgattaactatacatcagacgcgaacgcacctgtggtttatacaaataacgatggcgatctgatctttacgaataaagatgtcgtcacaaatggaaaggtgcaggccaatacagcaattaagggcgttatgaacccttacgtcagcggctatcttgcaatgtgggtgccggttggcgcatcagcgacacaggatgcaagaacagccgctagcacgaagacaacgacagatggctcagttttccacagcaacgctgcacttgatagcaacctgatttatgaaggattctcaaacttccaagcttttccggagaatgcctcagaaaatgccaatgcgatcatcgcccaaaatgtcgatctgttcaactcatggggagtcacgtcatttcaactggctcctcaatatgtctcaagccacgacggcagcttcctggacagcatcatcgacaacggctatgcattcacggacagatacgaccttgcgatgagcaaaaacaacaaatatggctcataccaggatctggttaatgtcctgaaggcactgcatgcgggaggaatccaagttatcgcagattgggttccggaccaaatctattcactgccgggcaaagaggtcgttagcgttgttagaagcgacgagttcggcaacaaagtggatggcacgcaaatcgataacacgctgtacgtggtcaatacgatcggcggaggccagtatcaaaaggaatacggcggaagataccttgaagaacttaaacaaaagtatccggagctttttaagacgaaacagccttcaacaggcgttacaatcgatccgtcagagaagattacggagtggagcgccaagtatctgaacggcacaaacattcttcatagaggcgcagaatttgtcctgagagatggcgctacatactttagagtcgcagaaacaagcgaagtgttccttcctagccagcttagaggcaaaatcacaaaaaacggattttggaaaaacgacgcgggaaaagtcaactactataactcagagggagaaatcatgaaaaatgctttcgtcaaagacggaaagaataactggtactacttcgacaatgacggcaatatggtcacgaacacggcactgacgattgattcagatgcccaggtggctgattactatttcctgaataacggcattagccttagagacggctttgtgcaacttgcaaacggagacatctactactacgatgtgaatggcagaaaacttaagaacggcaaagttacagtcaataacgttgaatacacaacggacaaaaatggcaaggtggtcggagagaacgtgctgaaaaaactggatgagattattacaacgggaaagacgacacttatttga

SEQ ID NO: 30 - protein, 1615 aa, Artificial sequence
  Mature GTF8117 with added methionine
MDETSSSNETQTEQTLNTDESTDTTTDVSNEAKATEAQLTTQDADMASSEEKTTNVEKEVTTAETNKDTTVKNVESSEQNTTTVADKNAVDSTAQVNTAEKENKYTQENVNGNWYLKDEQGNYLTGFQEIKDQNKTVYYNPDSKQMVYGQQNINGNWYLFDTFNGAMQTGLQYIRDQKKLAYYNEQGQMQYGTVEIDGQKYQADTFNGAIKGKGQTKIADNWYLFNNAGQVVDGWQWINDQGKTVYYSTKTAQMVHGQQNINGHWYLFDKTTGAMQRGFQNLKAYGDDKTVYYNQDGWMLYGQQKIDNKWYNFDTFNGAMKTGFVKIPEQNKTVYYAPNGQMQYGWQWVDNATRYFDTFNGAMATGQKLITGHWYLFDNNGAMQRGFQNLKNYGDNKTVYYNQDGWMLYGWQWVNNATRYFDTFNGAMTTGQKKINDHWYLFDKDGAMQRGIQYIPEENKLVYYNQDGWMLYGKQNINGVDHNFNTFNGALEAKGQVKVGNNWYLFNNSGTIQTGFQDLKAYGQDKVVYYDPKTAAMVYGYQNIDGNWYLFSRANGSMQRGLQNVNGVDLLFDEKTGALLTGVQNIKGNNYFVDKRSGNIKKNLVVLGADNKWMYFDAKTGKGTNTLEDQYKKGVVSGNVEFITNNAAYSFDGNSFENINGFLTADSWYRPKSILKDGSTWTATTETDLRPLLMTWWPNEQIKANYLNYMKDKGFINNSGTYNAESDPNYMDFAAQEAQRNIERKITKENDTTWLRDLITDFIKTQDIWNEQSEGVSTEGLQKFQGGFLKYVNSELTPYANSEWRKLGYQPTMLTQNNVGAEFLLANDIDNSNPVVQAEQLNWLHFLMNFGTITANDPSANFDGIRIDAVDNVDASLLSIAGDYFKAAYKVGQNDATANKHISILEDWNDKDPEYVNSIGNPQLTMDDYIVQQLKFSLGQAPDKVDRMQRFKEWYLVDRSKDNTENTAIPNYSFVRAHDASVQEDILQLIQDTTGKPWGVYTNEELQQGLKDYMADQKLTNKKYNRYNIPSSYAILLTNKDTIPRVYYGDLYSDAGKYMAEKSIYFDAIDNLLKTRTKYVAGGQTLDVDGHDILTSVRFGKGALNVTDKGTSETRTQGMGLIISNNNSLKLNDGEKVVLHMGAAHKNQAYRAVMLSSANGLINYTSDANAPVVYTNNDGDLIFTNKDVVTNGKVQANTAIKGVMNPYVSGYLAMWVPVGASATQDARTAASTKTTTDGSVFHSNAALDSNLIYEGFSNFQAFPENASENANAIIAQNVDLFNSWGVTSFQLAPQYVSSHDGSFLDSIIDNGYAFTDRYDLAMSKNNKYGSYQDLVNVLKALHAGGIQVIADWVPDQIYSLPGKEVVSVVRSDEFGNKVDGTQIDNTLYVVNTIGGGQYQKEYGGRYLEELKQKYPELFKTKQPSTGVTIDPSEKITEWSAKYLNGTNILHRGAEFVLRDGATYFRVAETSEVFLPSQLRGKITKNGFWKNDAGKVNYYNSEGEIMKNAFVKDGKNNWYYFDNDGNMVTNTALTIDSDAQVADYYFLNNGISLRDGFVQLANGDIYYYDVNGRKLKNGKVTVNNVEYTTDKNGKVVGENVLKKLDEIITTGKTTLI

SEQ ID NO: 31 - DNA, 4674 bp, Streptococcus salivarius
gaagaaacaaataactctaatggatcaccttcaacaactacggtcggggaaaatacaaatcctgtggttgaaaaagaggtaggcacaacaactgaggtagcaaatacttcaaatgccacaacaacagagcgagcagaagttactgctgacaaaccagctgaaacgacggttcaaccaaattcaggaacaactacaagtgatagagctgtagcagtagaggttgaagccaaacctgaaacgactgctaagccagaagttgctactaaaccagaaacagctacaacatcagaagtcgctgcaaatgctggagtagctgctccaacgactgagaagtctaaagagctttctgaagccgaaattaaggctgcagtctcactcgataatattaaaaaagaaaaagatggtaaatattactatcttttagaagatggatcacacaagaaaaactttgccattactgtaaatggtcaggtcctttattttgatgaaaatggtgccctttcaagcacatcaacgtattcatttacacaagaaacaacaaatctagtcactgattttacaaaaaataatgctgcctacgattcaactaaagcgagctttgaacttgttgatggttatttgacagcagacagttggtaccgtccaaaagaaatccttgaagctggtacaacttggaaagcgtcaactgaaaaagattttcgtccacttttgatgtcttggtggcctgataaggatactcaagtagcttacttgaattacatgactaaggctcttagcaacggtgaagaaacaaaagatgtctttacgattgaaaattctcaagcgagcttgaatgccgcagctcaaatcctccaacgtaagattgaagttaagattgctgctaataagtcaacagactggttgcgtcagtcaatcgaggcttttgttaaagaccaagataaatggaacattaattctgaatcgccaggtaaggaacacttccaaaaaggtgcgcttctttttgtgaacagcgattcaactaaatgggctaactctgattatcgtaaacttaatcaaacggcgacaagttatattaaaaatcataagattgttaatggtagcgatggtggttatgaattcttgctctcaaatgacattgacaactctaatccagtcgttcaagcagaaatgcttaaccaattgtattactttatgaactggggacaaatcgtctttggtgataaggacaaggatgctcactttgatggtatacgtgttgatgctgtggataatgttagcgttgacatgcttcaattagtgtcttcatacatgaaggctgcatacaaggttaatgagtcggaagctcgtgcccttgcgaatatctctattcttgaagcatggtcacacaatgacccatattatgtgaatgagcacaacacagcagctctttctatggataatggtctccgtttgtcaattgttcacggattaactcgtccagtaactaataaaggtacaggtgcacgtaatgcatcaatgaaggaccttattaacggaggttatttcggtctctcaaaccgtgcagaagtcacttcatatgatcaacttggttttgcaacctacctctttgttcgtgcacatgactcagaagttcaaacggttatcgcagacattatcagtaaaaaaattgatcctacaacagatggtttcactttcacattagatcaattgaaacaagcattcgatatttataatgctgatatgttgaaagttgataaggaatatacgcattcaaatattcctgctgcctatgctttgatgcttcaaacaatgggtgcggcaacacgtgtttattatggagatttgtatactgataatggtcaatacatggctaagaaatcaccatactttgatcaaatcacaactcttcttaaagcgcgtcctaagtatgtagctggtggtcaaacatcttatatccacaaccttgctggtgatggggtatcatctgctaaagacaataaagaagttcttgtctctgtccgttatggtcaagatttgatgtctaagacagatacagaaggtggaaaatacggtcgcaattcaggtatgttgacccttattgctaataacccggatttgaaattagcagatggtgaaactattactgtaaatatgggtgcagctcacaagaaccaagcctaccgtccactcttgcttggtacggataaaggtatcgtgtcatcattgaatgattcagatactaaggttgttaaatatacagatgcacaaggaaatcttgtcttcacagctgatgaaatcaaaggctttaagactgttgatatgagtggttacctttcagtttgggtaccagtaggtgcgactgacgatcaaaacgttcttgctaaaccatcaacaaaagcctacaaagaaggggataaggtttatagttcttctgcagcacttgaagcacaagtgatttacgaaggcttctcaaacttccaagactttgttaaagaagatagtcaatacactaataaattgattgcagctaatgcagacctcttcaagtcatggggcattacgtcatttgaaattgcacctcaatatgtctcatctaaggatggaactttccttgattctattattgagaatggttatgccttcacagaccgttatgactttgccatgagcaaaaacaataaatacggttcaaaagaagatcttcgtgatgctctcaaggctcttcacaaacaaggtattcaagtcattgctgactgggttccagaccaattgtacacccttccaggtaaagaagtagtgactgctacgcgtactgatacacatggtaaggtccttgatgatactagcttggttaataaactttatgtgacaaataccaagtcatcaggtaatgatttccaagcccagtacggtggtgccttcctcgacaaacttcaaaaactttatccagaaatcttcaaagaagttatggaagcgtctggtaagacaattgatccatctgtgaagattaaacagtgggaagctaaatactttaacggtacaaacatccaaaaacgtggttctgactatgttctcagcgatggtaaattgtacttcaccgttaacgataaaggtaccttcctcccagcagccttgactggtgatacaaaagctaagactggttttgcctatgatggtacaggtgtaacttattacacaacatcaggtactcaagctaagagtcagtttgtaacttataacggtaagcaatactactttaacgataagggttaccttgtaactggtgaacaaactatcgatggttctaactatttcttcttgccaaatggtgtcatgtttactgatggtgtcagaaaaaatgccaaaggtcaatcattggtttatggtaagtcaggtaaattgacgactcaaactggttggaaagaagttaccgttaaagatgatagtggtaaggaagagaaattctaccaatacttcttcaagggtggtatcatggctactggtttgactgaagtagaaggtaaggaaaaatacttctatgataatggttaccaagctaaaggtgtcttcgttcctacaaaagacggccatttaatgttcttctgtggtgattcaggcgaacgtaagtactcaggcttctttgaacaagatggtaactggtactacgccaatgataaaggctatgttgctactgggtttactaaggtaggtaaacaaaacctttacttcaatgaaaaaggtgttcaagttaagaatcgcttcttccaagttggtgatgctacatactatgcaaataacgaaggtgacgttcttcgtggtgctcaaaccatcaatggagacgaactctactttgatgaatcaggtaaacaagttaaaggtgagttcgtgaacaatcctgatggtacgacttcatactacgatgcaatcacaggtgtgaaacttgttgatacatcactggtagttgatggtcaaacctttaatgtcgatgctaagggtgttgtgactaaggcacatacaccaggcttctatactactggggacaacaactggttctatgcagactcatatggacgtaatgtcacaggtgctcaggtcatcaatggtcaacacctctactttgatgctaatggtcgccaagttaagggtggcttcgtaacgaacactgacggtagtcgttcattctaccactggaataccggtgataaattggtatcaaccttcttcactaccggtcatgatagatggtattatgctgatgataggggtaatgtcgttacaggagctcaagttatcaacggtcaaaaactcttctttgatactgatggtaagcaggttaaaggtgctttcgcaacaaatgcgaatggtagtcgctcatactaccactggaatactggtaataagttagtatcaaccttcttcacaagtggagataacaactggtattatgcagatgccaagggtgaagttgttgttggcgaacagacgatcaacggtcaacacctttactttgaccaaactggtaagcaagtgaagggggcaactgctacgaatcctgatggctcaatctcttactatgatgttcatacaggggaaaaggctattaatcgttgggttaaaattccttcagggcaatgggtatacttcaacgctcaaggaaaaggctacgtgtcataa

SEQ ID NO: 32 - protein, 1557 aa, Streptococcus salivarius
EETNNSNGSPSTTTVGENTNPVVEKEVGTTTEVANTSNATTTERAEVTADKPAETTVQPNSGTTTSDRAVAVEVEAKPETTAKPEVATKPETATTSEVAANAGVAAPTTEKSKELSEAEIKAAVSLDNIKKEKDGKYYYLLEDGSHKKNFAITVNGQVLYFDENGALSSTSTYSFTQETTNLVTDFTKNNAAYDSTKASFELVDGYLTADSWYRPKEILEAGTTWKASTEKDFRPLLMSWWPDKDTQVAYLNYMTKALSNGEETKDVFTIENSQASLNAAAQILQRKIEVKIAANKSTDWLRQSIEAFVKDQDKWNINSESPGKEHFQKGALLFVNSDSTKWANSDYRKLNQTATSYIKNHKIVNGSDGGYEFLLSNDIDNSNPVVQAEMLNQLYYFMNWGQIVFGDKDKDAHFDGIRVDAVDNVSVDMLQLVSSYMKAAYKVNESEARALANISILEAWSHNDPYYVNEHNTAALSMDNGLRLSIVHGLTRPVTNKGTGARNASMKDLINGGYFGLSNRAEVTSYDQLGFATYLFVRAHDSEVQTVIADIISKKIDPTTDGFTFTLDQLKQAFDIYNADMLKVDKEYTHSNIPAAYALMLQTMGAATRVYYGDLYTDNGQYMAKKSPYFDQITTLLKARPKYVAGGQTSYIHNLAGDGVSSAKDNKEVLVSVRYGQDLMSKTDTEGGKYGRNSGMLTLIANNPDLKLADGETITVNMGAAHKNQAYRPLLLGTDKGIVSSLNDSDTKVVKYTDAQGNLVFTADEIKGFKTVDMSGYLSVWVPVGATDDQNVLAKPSTKAYKEGDKVYSSSAALEAQVIYEGFSNFQDFVKEDSQYTNKLIAANADLFKSWGITSFEIAPQYVSSKDGTFLDSIIENGYAFTDRYDFAMSKNNKYGSKEDLRDALKALHKQGIQVIADWVPDQLYTLPGKEVVTATRTDTHGKVLDDTSLVNKLYVTNTKSSGNDFQAQYGGAFLDKLQKLYPEIFKEVMEASGKTIDPSVKIKQWEAKYFNGTNIQKRGSDYVLSDGKLYFTVNDKGTFLPAALTGDTKAKTGFAYDGTGVTYYTTSGTQAKSQFVTYNGKQYYFNDKGYLVTGEQTIDGSNYFFLPNGVMFTDGVRKNAKGQSLVYGKSGKLTTQTGWKEVTVKDDSGKEEKFYQYFFKGGIMATGLTEVEGKEKYFYDNGYQAKGVFVPTKDGHLMFFCGDSGERKYSGFFEQDGNWYYANDKGYVATGFTKVGKQNLYFNEKGVQVKNRFFQVGDATYYANNEGDVLRGAQTINGDELYFDESGKQVKGEFVNNPDGTTSYYDAITGVKLVDTSLVVDGQTFNVDAKGVVTKAHTPGFYTTGDNNWFYADSYGRNVTGAQVINGQHLYFDANGRQVKGGFVTNTDGSRSFYHWNTGDKLVSTFFTTGHDRWYYADDRGNVVTGAQVINGQKLFFDTDGKQVKGAFATNANGSRSYYHWNTGNKLVSTFFTSGDNNWYYADAKGEVVVGEQTINGQHLYFDQTGKQVKGATATNPDGSISYYDVHTGEKAINRWVKIPSGQWVYFNAQGKGYVS

SEQ ID NO: 33 - protein, 1338 aa, Streptococcus criceti
MEKNLRYKLHKVKKQWVAIGVTTFAVGFLAGGQVVAADATDGNGGNTQVAHLIPKEPTDYKFDTPSGILTGLNFANAQTSPAGDNAGANQPAGGIEPQTAENAATDGQAVPQTSDQPGHLENVDGKTYYVDANGQRLKNYSTVIDGKTYYFDAQTGQAQAETPQINQNDNQVAPDTYAANNQAFTNDVSSFETVDNYVTADSWYRPRKILKNGESWQASAESDMRPILMTWWPDAATKAAYANYWVKEGLISGSYSPNSANLETAVQTIQAAIEKKIASEGSTAWLRDKMSQFVKSQNQWSLASENPTVYPNQDHLQGGALLFSNNEATAHANSDWRLLNRNPTFQTGKQKYFTTNYAGYELLLANDVDNSNPIVQAEQLNHFHYLMNWGEIVMGDKNANFDGVRVDAVDNVNADLLQIQRDYYKAKYGVDQNEKNAIDHLSILEAWSGNDNDYVKDQNNFSLSIDNSQRSYMLAAFAYPASQRGNDYISLLPKVGLKDRRYAKNGNPVPNYVFIRAHDSEVQTRIAKIIRERLGKTNADGLTNITLDDLNKAFDIYNQDMKAVDKQYYPNNLPMAYAWMLQNKDTVTRVYYGDMYTDDGQYMETKTPFHDAIETLLKARIKYVAGGQTAGYVQGWGSGILTSVRYGKGADTAIDAGTAETRTSGMAVLINNKPNFQSYNGLTLDMGAAHKNQAYRPLLLSTKDGIATYLNDSDVSSNQYKYTDGQGRLNFSASELRSVANVQVSGMIQVWVPVGAADNQDVRVAPNTNRNNSSNIYTQSDALDSQVIYEGFSNFQAFAKTPEQYTNAVIAKNADLFKSWGITQFEMAPQYVSSEDGTFLDSVVLNGYAFSDRYDLAMSKNNKYGSKEDLANAIKGLHNAGIKVLSDWVPDQMYNLPGKEVVTATRVDQYGRPKAGATINRTPYVVNTKTYGDYQEQYGGKFLDELQKLYPSLFTTKQISTGKPIDPSVKITNWSAKYFNGSNILGRGAKYVLSDNNKYLNLGAGQFFLPTNLNNTYGQPQAPANGFISKNGGIHYIDNNGQEVKNQFKEIAGSWYYFDANGKMATGQTKIGNTTYLFMPNGKQLKEGVWYDGKKAYYYDDNGRTWTNKGFVEFKVNGQDKWRYFNGDGSIAVGLVSLDNRTLYFDAYGYQVKGQTLTINGKTYSFDANEGDLITGNTPSPEPNNQGAWEALGDNQWGYRKDGKLLTGSQTIAGQKVFFQPNGVQVKGGTAKDEAGVLRFYDRDQGHLAGKGWYSTADNNWVYVDDAGRVVTGLQKIGSQTLYFDDNGIQAKGKAIWDKDGNLRYFAAGSGDMITNRWYNIGDNQWYWFNNQGIASRW

SEQ ID NO: 34 - DNA, 4914 bp, Artificial sequence
  Codon-optimized sequence encoding mature GTF9905
gatgattcacaacaaagctctacacaaatccaaagcacacaagtgacgacagcgttaccggcgggcggccaatattctacgacgaacggaggacaatcttggaattacctggtgaacggggtcgcgattaaaggcatgtatcaagatggccaaggccaacttcggtattttaattttatcgatggaacacaagttaaaggtgaatttttgagcattaatggcacgtattattattttgatcaaaatagtggagaaggacatctggttcctacacaatctaatggccattatacagaaatcggcaatacgggagcgtggggctatcaaaattctaacggagaactggtgaaaggcatccaaaatatcgatggccaacttcgctattttgatgaaaatacaggaaatcaagtgaaaggcggctcagcgacgattggcaacaaaagctattattttgaaccgagccaaggaacactgacaacgacgatcgatcaagtttctgatgcgcaaaatgcgaatatccggggccttgcgacagtgaatgggcaacttaattattttgatcctacaacgggagaacaagcgaaacataaacaagttgcgacgaatggcgcgacgtattattttaatgatagcggcgtcggcacatatctgtttacgaatgtccaaaatacacctgcgaatgatgtgagccaacataatgcagtcaattctacggatacgaaagattatacgaatacagtcgatggctttcttacagcggatacgtggtatagacctaaatatatcttagataacggcgaaaattggagggcgtctaatgagggcgaatatcgcccgtttatcatgaattggtggcctaacaaaaatgtcgaagttaattatctgaaacttatgcaaaacaacaatctgctgagctctacagttcaatatgatttgtttacggatcaagcgatcctgaatcaagcagcatatcaagcgcaaattgcaattgaaaaacgcattaaatctgaaggctctacggattggctgaatacactgctgtttggcggcgatgattctcatccgagctttgttaaacaacagtttatctggaactcagattcagaaagcccttggcaaggggatgcgtggtttcaggggggctatcttaaatatggcaattctgtcatgacaccgacgtctaatagcaattatagacaagcaggcaatgcgtttgattttctgcttgcgaatgatgtcgataatcaaaatccgatcgtccaagcagaagatcttaattggttgtattatcttatgaattttggctctatcacgacgaatggtctggataatgattctaattttgattctattcggttagatgcagtcgattttatccataatgatgcgatccaacgtacatatgattatcttcgccaagcgtttaatctgacgaaaaacgaggcgacagcgaatcaacatctgagcctggttgaagcaggcgtcgatgcaggaacaacgacgtataattcagatggacttatcgaaagcaatattcgcccgcttgcgacggatagcctgacgaatgcaccgggcaaaaatgcgagcctttctaatctgattaaagatgtcgatagcggagaagtcattgcagatcatgcgaattttagcacggatgatggcatccctaattatagcatcatccatgcacatgataaaggcatccaagaaaatgtcggcgcggcgatcacagcagcgacgggcgcggattggacgaattttacgacagaacaacttgaacaaggcttagatctgtattatcaagatcaacgctctacgaataagaaatataatatctataacttgccgagcatctatgcacttatgttgacgaataagggaacggtgcctagagtgtattatggagatatgtatcaagataatggccaatatatgcaacaaaaatctctgtattatgatgcgattagctcacttatgacagcgcgtaaacaatatgtcgcgggaggccaaacgatgtctgtcgatgaaaacggactgcttaaatcagttcgctttggcaaaaatgcaatgacagcacaagatacaggggacgcagaaacacgcacagaaggggtgggagtcatcattggcaatgatccttcagtgaaagtcgcggatggccaaacggtgacgttagatatgggcgcagcacataaaaatcaagcgtatagaccgttgatcctgacgacgtcagatggcatccaaacgtatgatagcgatgaaaatgcaccggttgtgtatacggatgataatggcattcttacattttctaatcaagatatcaatggccaagcgaatacgaaaattgtcggcacgctgaatcctcaagtctcaggctatcttgcagtgtgggttccggtcggcgcatctgcggatcaagatgcacgcacagcgccgagcacgcaaagcacgaatgatggcaaagtgcttcatacaggcgcagcactggattctaatcttatctttgaaggcttttctaattttcaacctatgccgacaacgcatgatgaaatgacaaatgttgtcatctcacaaaatgcgtctcaatttgcgaaatggggcatcacgagctttgaaatggcgcctcaatatcgtagctcagaagatcatagctttttagattctacgatcgataatggctatgcgttttcagatcgctatgatctgggctttggaacacctacgaaatatggaacggatgaagatcttcgtaatgcgattaaagcgctgcatcaaaatggcatgcaagtcatggcggatgttgtcatgaatcaactgtatagcctgaatggcaaagaagtggtgagcgcgtctcgtgcgggagtgtatggcaatgatgtcgatcttccgtttggaacgcaactgtatgtcgttaatacgacgggcggcggagaatatcagaaaaaatatggaggcgcgtttctgaatatcattaaagaaaaatatcctacgctgtttgattcagaaagctatgattattatcttaaaaattattcagataatggccatggacctgcgtatatgacgacggcgacagcgacacgggaagcgatcccgtcagatcaaccgcttaaagaatggtctgcgaaatatatgaacggcacgaatatcctgggactgggcatgggctatgtgcttaaagattggaataacggcgcgtattttaaactttcaggaacggatacgacactgccgcaaagccttgttgcacttacaggctggaatcaaaatgatgatggaacgtggtcatattatagcacggatacagatgatcgtgtcacgggcaaacaagtcatcgatggccgcacgttactgtttgataatcaaggcaatcaaattaaaggcggctggggagaaaatccggatggaacgtggtcatattataatgcggatacgggggatcgggtcatcggagaacaagtcatcgatggccgtacattgttctttgataatcaaggcgtccaagttaaaggcggatggggagaaaattatgatggaacgtggtcttattataatgcagatacaggcgatagagtgacaggcaaacaagtcatcgatggccgtacgctgttgtttgataatagaggcgtccaagttaaagggggctggggagaaaattcagatggaacgtggtcatattataatgcagatactggcgatagagtcacgggcaatcaactgatcggcggccgtaacttgctgtttgataatcaaggcaatcaaattaaaggcggctgggatgaaaatccggatggcacgtggtcatattataatgcagatacgggagatcgtgtgacgggagtccaagtcattgatggcaaacaactgctgtttgatagcaatggcattcaagttaaaaatagctggcagaagaacgcgaatggcacatggtcatattatgatgcgaatgatggccaccttgttcctgcgaatagctctaatgatggcacgagctcttctacacaagattcaggcaacaaaagcaatcaaaatccgtctagctctagcaatgcagttaacaaaacaacgggctggattaaaaattcagatggaacgtggtcatatctgagcgcgaaaagcggccaaaaagttacaggaagccaaacgatcgatggcaaacaactgttgtttgatgatcatggagtccaaattaagggtggctggggcaaaaatgcggatggaacgtggtcatattatgatgcgaatagcggagaacttacgtctacgtcagatatgtctaatgtgaatcctcaacaaacgacaacgacgacgaatgagcaatctacgacgaatcaacctacggatatcacgaaaaattcagatggagtgtatgtgtataagaatgattctaacaagaaagcacaaggctatcttaatgatggaagctcttggaaatggtttaatgatggccaactgtatacgggctttcaaaattatatgggcgcgtattattattttatcaatggcatccgccaacaaaatcaatgggaaaatatctggggacttaaatattatgtgggagatgatggccgtacggtcgaaggcatccatgcgatcgatggacatgcgtatgattttggcacggatggaacgtttaatgttaaaggctcagcgtcaggctatttgaatgatggcaaatcttggatgtggtatgaaggcggcaatccgtatacaggctttcggtattatatggatacgtattattggtttgaaaatggtgttagacaagataatgcgtggcatcaagcgtggggacttacatattatacgggcgcagatggacgcgcggtccagggtgtccaaaatatcaatggcaaactgtattattttggcaatgatggaacatttttcatgcgtacgaatcaagaagtgtga